European Patent Application EP 4 198 050 A1, published June 21, 2023. Title: FUSION PROTEIN COMPRISING IL-12 AND ANTI-CD20 ANTIBODY AND USE THEREOF. Applicant: Kanaph Therapeutics INC. The sequence listing filed with the application follows.

SEQUENCE LISTING (285 sequences)

SEQ ID NO: 1 - protein, 451 aa, Artificial Sequence
  anti-hu CD20 HC hu IgG1 Fc knob
QVQLQQPGAELVKPGASVKMSCKASGYTFTSYNMHWVKQTPGRGLEWIGAIYPGNGDTSYNQKFKGKATLTADKSSSTAYMQLSSLTSEDSAVYYCARSTYYGGDWYFNVWGAGTTVTVSAASTKGPSVFPLAPSSKSTSGGTAALGCLVKDYFPEPVTVSWNSGALTSGVHTFPAVLQSSGLYSLSSVVTVPSSSLGTQTYICNVNHKPSNTKVDKKVEPKSCDKTHTCPPCPAPELLGGPSVFLFPPKPKDTLMISRTPEVTCVVVDVSHEDPEVKFNWYVDGVEVHNAKTKPREEQYNSTYRVVSVLTVLHQDWLNGKEYKCKVSNKALPAPIEKTISKAKGQPREPQVYTLPPSRDELTKNQVSLWCLVKGFYPSDIAVEWESNGQPENNYKTTPPVLDSDGSFFLYSKLTVDKSRWQQGNVFSCSVMHEALHNHYTQKSLSLSPGK

SEQ ID NO: 2 - protein, 213 aa, Artificial Sequence
  anti-hu CD20 LC
QIVLSQSPAILSASPGEKVTMTCRASSSVSYIHWFQQKPGSSPKPWIYATSNLASGVPVRFSGSGSGTSYSLTISRVEAEDAATYYCQQWTSNPPTFGGGTKLEIKRTVAAPSVFIFPPSDEQLKSGTASVVCLLNNFYPREAKVQWKVDNALQSGNSQESVTEQDSKDSTYSLSSTLTLSKADYEKHKVYACEVTHQGLSSPVTKSFNRGEC

SEQ ID NO: 3 - protein, 755 aa, Artificial Sequence
  hu scIL-12-hu IgG1 Fc hole
IWELKKDVYVVELDWYPDAPGEMVVLTCDTPEEDGITWTLDQSSEVLGSGKTLTIQVKEFGDAGQYTCHKGGEVLSHSLLLLHKKEDGIWSTDILKDQKEPKNKTFLRCEAKNYSGRFTCWWLTTISTDLTFSVKSSRGSSDPQGVTCGAATLSAERVRGDNKEYEYSVECQEDSACPAAEESLPIEVMVDAVHKLKYENYTSSFFIRDIIKPDPPKNLQLKPLKNSRQVEVSWEYPDTWSTPHSYFSLTFCVQVQGKSKREKKDRVFTDKTSATVICRKNASISVRAQDRYYSSSWSEWASVPCSGGGGSGGGGSGGGGSRNLPVATPDPGMFPCLHHSQNLLRAVSNMLQKARQTLEFYPCTSEEIDHEDITKDKTSTVEACLPLELTKNESCLNSRETSFITNGSCLASRKTSFMMALCLSSIYEDLKMYQVEFKTMNAKLLMDPKRQIFLDQNMLAVIDELMQALNFNSETVPQKSSLEEPDFYKTKIKLCILLHAFRIRAVTIDRVMSYLNASGGGGSGGGGSDKTHTCPPCPAPELLGGPSVFLFPPKPKDTLMISRTPEVTCVVVDVSHEDPEVKFNWYVDGVEVHNAKTKPREEQYNSTYRVVSVLTVLHQDWLNGKEYKCKVSNKALPAPIEKTISKAKGQPREPQVYTLPPSRDELTKNQVSLSCAVKGFYPSDIAVEWESNGQPENNYKTTPPVLDSDGSFFLVSKLTVDKSRWQQGNVFSCSVMHEALHNHYTQKSLSLSPGK

SEQ ID NO: 4 - protein, 755 aa, Artificial Sequence
  hu scIL-12 mut1-hu IgG1 Fc hole
IWELKKDVYVVELDWYPDAPGEMVVLTCDTPEEDGITWTLDQSSEVLGSGKTLTIQVKEFGDAGQYTCHKGGEVLSHSLLLLHKKEDGIWSTDILKDQKEPKNKTFLRCEAKNYSGRFTCWWLTTISTDLTFSVKSSRGSSDPQGVTCGAATLSAERVRGDNKEYEYSVECQEDSACPAAEESLPIEVMVDAVHKLKYENYTSSFFIRDIIKPDPPKNLQLKPLKNSRQVEVSWEYPDTWSTPHSYFSLTFCVQVQGASKREAKDRVFTDKTSATVICRKNASISVRAQDRYYSSSWSEWASVPCSGGGGSGGGGSGGGGSRNLPVATPDPGMFPCLHHSQNLLRAVSNMLQKARQTLEFYPCTSEEIDHEDITKDKTSTVEACLPLELTKNESCLNSRETSFITNGSCLASRKTSFMMALCLSSIYEDLKMYQVEFKTMNAKLLMDPKRQIFLDQNMLAVIDELMQALNFNSETVPQKSSLEEPDFYKTKIKLCILLHAFRIRAVTIDRVMSYLNASGGGGSGGGGSDKTHTCPPCPAPELLGGPSVFLFPPKPKDTLMISRTPEVTCVVVDVSHEDPEVKFNWYVDGVEVHNAKTKPREEQYNSTYRVVSVLTVLHQDWLNGKEYKCKVSNKALPAPIEKTISKAKGQPREPQVYTLPPSRDELTKNQVSLSCAVKGFYPSDIAVEWESNGQPENNYKTTPPVLDSDGSFFLVSKLTVDKSRWQQGNVFSCSVMHEALHNHYTQKSLSLSPGK

SEQ ID NO: 5 - protein, 755 aa, Artificial Sequence
  hu scIL-12 mut2-hu IgG1 Fc hole
IWELKKDVYVVELDWYPDAPGEMVVLTCDTPEEDGITWTLDQSSEVLGSGKTLTIQVKEFGDAGQYTCHKGGEVLSHSLLLLHKKEDGIWSTDILKDQKEPKNKTFLRCEAKNYSGRFTCWWLTTISTDLTFSVKSSRGSSDPQGVTCGAATLSAERVRGDNKEYEYSVECQEDSACPAAEESLPIEVMVDAVHKLKYENYTSSFFIRDIIKPDPPKNLQLKPLKNSRQVEVSWEYPDTWSTPHSYFSLTFCVQVQGASAREAADRVFTDKTSATVICRKNASISVRAQDRYYSSSWSEWASVPCSGGGGSGGGGSGGGGSRNLPVATPDPGMFPCLHHSQNLLRAVSNMLQKARQTLEFYPCTSEEIDHEDITKDKTSTVEACLPLELTKNESCLNSRETSFITNGSCLASRKTSFMMALCLSSIYEDLKMYQVEFKTMNAKLLMDPKRQIFLDQNMLAVIDELMQALNFNSETVPQKSSLEEPDFYKTKIKLCILLHAFRIRAVTIDRVMSYLNASGGGGSGGGGSDKTHTCPPCPAPELLGGPSVFLFPPKPKDTLMISRTPEVTCVVVDVSHEDPEVKFNWYVDGVEVHNAKTKPREEQYNSTYRVVSVLTVLHQDWLNGKEYKCKVSNKALPAPIEKTISKAKGQPREPQVYTLPPSRDELTKNQVSLSCAVKGFYPSDIAVEWESNGQPENNYKTTPPVLDSDGSFFLVSKLTVDKSRWQQGNVFSCSVMHEALHNHYTQKSLSLSPGK

SEQ ID NO: 6 - protein, 587 aa, Artificial Sequence
  (anti-hu CD20 VH)2-hu IgG1 Fc knob
QVQLQQPGAELVKPGASVKMSCKASGYTFTSYNMHWVKQTPGRGLEWIGAIYPGNGDTSYNQKFKGKATLTADKSSSTAYMQLSSLTSEDSAVYYCARSTYYGGDWYFNVWGAGTTVTVSAGGGGSGGGGSGGGGSQVQLQQPGAELVKPGASVKMSCKASGYTFTSYNMHWVKQTPGRGLEWIGAIYPGNGDTSYNQKFKGKATLTADKSSSTAYMQLSSLTSEDSAVYYCARSTYYGGDWYFNVWGAGTTVTVSAASTKGPSVFPLAPSSKSTSGGTAALGCLVKDYFPEPVTVSWNSGALTSGVHTFPAVLQSSGLYSLSSVVTVPSSSLGTQTYICNVNHKPSNTKVDKKVEPKSCDKTHTCPPCPAPELLGGPSVFLFPPKPKDTLMISRTPEVTCVVVDVSHEDPEVKFNWYVDGVEVHNAKTKPREEQYNSTYRVVSVLTVLHQDWLNGKEYKCKVSNKALPAPIEKTISKAKGQPREPQVYTLPPSRDELTKNQVSLWCLVKGFYPSDIAVEWESNGQPENNYKTTPPVLDSDGSFFLYSKLTVDKSRWQQGNVFSCSVMHEALHNHYTQKSLSLSPGK

SEQ ID NO: 7 - protein, 334 aa, Artificial Sequence
  (anti-hu CD20 VL)2
QIVLSQSPAILSASPGEKVTMTCRASSSVSYIHWFQQKPGSSPKPWIYATSNLASGVPVRFSGSGSGTSYSLTISRVEAEDAATYYCQQWTSNPPTFGGGTKLEIKGGGGSGGGGSGGGGSQIVLSQSPAILSASPGEKVTMTCRASSSVSYIHWFQQKPGSSPKPWIYATSNLASGVPVRFSGSGSGTSYSLTISRVEAEDAATYYCQQWTSNPPTFGGGTKLEIKRTVAAPSVFIFPPSDEQLKSGTASVVCLLNNFYPREAKVQWKVDNALQSGNSQESVTEQDSKDSTYSLSSTLTLSKADYEKHKVYACEVTHQGLSSPVTKSFNRGEC

SEQ ID NO: 8 - protein, 713 aa, Artificial Sequence
  anti-hu CD20 HC hu IgG1 Fc knob-anti-hu CD20 scFv
QVQLQQPGAELVKPGASVKMSCKASGYTFTSYNMHWVKQTPGRGLEWIGAIYPGNGDTSYNQKFKGKATLTADKSSSTAYMQLSSLTSEDSAVYYCARSTYYGGDWYFNVWGAGTTVTVSAASTKGPSVFPLAPSSKSTSGGTAALGCLVKDYFPEPVTVSWNSGALTSGVHTFPAVLQSSGLYSLSSVVTVPSSSLGTQTYICNVNHKPSNTKVDKKVEPKSCDKTHTCPPCPAPELLGGPSVFLFPPKPKDTLMISRTPEVTCVVVDVSHEDPEVKFNWYVDGVEVHNAKTKPREEQYNSTYRVVSVLTVLHQDWLNGKEYKCKVSNKALPAPIEKTISKAKGQPREPQVYTLPPSRDELTKNQVSLWCLVKGFYPSDIAVEWESNGQPENNYKTTPPVLDSDGSFFLYSKLTVDKSRWQQGNVFSCSVMHEALHNHYTQKSLSLSPGKGGGGSGGGGSGGGGSQVQLQQPGAELVKPGASVKMSCKASGYTFTSYNMHWVKQTPGRGLEWIGAIYPGNGDTSYNQKFKGKATLTADKSSSTAYMQLSSLTSEDSAVYYCARSTYYGGDWYFNVWGAGTTVTVSAGGGGSGGGGSGGGGSGGGGSQIVLSQSPAILSASPGEKVTMTCRASSSVSYIHWFQQKPGSSPKPWIYATSNLASGVPVRFSGSGSGTSYSLTISRVEAEDAATYYCQQWTSNPPTFGGGTKLEIK

SEQ ID NO: 9 - protein, 475 aa, Artificial Sequence
  anti-hu CD20 LC-anti-hu CD20 scFv
QIVLSQSPAILSASPGEKVTMTCRASSSVSYIHWFQQKPGSSPKPWIYATSNLASGVPVRFSGSGSGTSYSLTISRVEAEDAATYYCQQWTSNPPTFGGGTKLEIKRTVAAPSVFIFPPSDEQLKSGTASVVCLLNNFYPREAKVQWKVDNALQSGNSQESVTEQDSKDSTYSLSSTLTLSKADYEKHKVYACEVTHQGLSSPVTKSFNRGECGGGGSGGGGSGGGGSQVQLQQPGAELVKPGASVKMSCKASGYTFTSYNMHWVKQTPGRGLEWIGAIYPGNGDTSYNQKFKGKATLTADKSSSTAYMQLSSLTSEDSAVYYCARSTYYGGDWYFNVWGAGTTVTVSAGGGGSGGGGSGGGGSGGGGSQIVLSQSPAILSASPGEKVTMTCRASSSVSYIHWFQQKPGSSPKPWIYATSNLASGVPVRFSGSGSGTSYSLTISRVEAEDAATYYCQQWTSNPPTFGGGTKLEIK

SEQ ID NO: 10 - protein, 984 aa, Artificial Sequence
  anti-hu CD20 HC hu IgG1 Fc hole-hu scIL-12
QVQLQQPGAELVKPGASVKMSCKASGYTFTSYNMHWVKQTPGRGLEWIGAIYPGNGDTSYNQKFKGKATLTADKSSSTAYMQLSSLTSEDSAVYYCARSTYYGGDWYFNVWGAGTTVTVSAASTKGPSVFPLAPSSKSTSGGTAALGCLVKDYFPEPVTVSWNSGALTSGVHTFPAVLQSSGLYSLSSVVTVPSSSLGTQTYICNVNHKPSNTKVDKKVEPKSCDKTHTCPPCPAPELLGGPSVFLFPPKPKDTLMISRTPEVTCVVVDVSHEDPEVKFNWYVDGVEVHNAKTKPREEQYNSTYRVVSVLTVLHQDWLNGKEYKCKVSNKALPAPIEKTISKAKGQPREPQVYTLPPSRDELTKNQVSLSCAVKGFYPSDIAVEWESNGQPENNYKTTPPVLDSDGSFFLVSKLTVDKSRWQQGNVFSCSVMHEALHNHYTQKSLSLSPGKGGGGSGGGGSGGGGSIWELKKDVYVVELDWYPDAPGEMVVLTCDTPEEDGITWTLDQSSEVLGSGKTLTIQVKEFGDAGQYTCHKGGEVLSHSLLLLHKKEDGIWSTDILKDQKEPKNKTFLRCEAKNYSGRFTCWWLTTISTDLTFSVKSSRGSSDPQGVTCGAATLSAERVRGDNKEYEYSVECQEDSACPAAEESLPIEVMVDAVHKLKYENYTSSFFIRDIIKPDPPKNLQLKPLKNSRQVEVSWEYPDTWSTPHSYFSLTFCVQVQGKSKREKKDRVFTDKTSATVICRKNASISVRAQDRYYSSSWSEWASVPCSGGGGSGGGGSGGGGSRNLPVATPDPGMFPCLHHSQNLLRAVSNMLQKARQTLEFYPCTSEEIDHEDITKDKTSTVEACLPLELTKNESCLNSRETSFITNGSCLASRKTSFMMALCLSSIYEDLKMYQVEFKTMNAKLLMDPKRQIFLDQNMLAVIDELMQALNFNSETVPQKSSLEEPDFYKTKIKLCILLHAFRIRAVTIDRVMSYLNAS

SEQ ID NO: 11 - protein, 984 aa, Artificial Sequence
  anti-hu CD20 HC hu IgG1 Fc hole-hu scIL-12 mut2
QVQLQQPGAELVKPGASVKMSCKASGYTFTSYNMHWVKQTPGRGLEWIGAIYPGNGDTSYNQKFKGKATLTADKSSSTAYMQLSSLTSEDSAVYYCARSTYYGGDWYFNVWGAGTTVTVSAASTKGPSVFPLAPSSKSTSGGTAALGCLVKDYFPEPVTVSWNSGALTSGVHTFPAVLQSSGLYSLSSVVTVPSSSLGTQTYICNVNHKPSNTKVDKKVEPKSCDKTHTCPPCPAPELLGGPSVFLFPPKPKDTLMISRTPEVTCVVVDVSHEDPEVKFNWYVDGVEVHNAKTKPREEQYNSTYRVVSVLTVLHQDWLNGKEYKCKVSNKALPAPIEKTISKAKGQPREPQVYTLPPSRDELTKNQVSLSCAVKGFYPSDIAVEWESNGQPENNYKTTPPVLDSDGSFFLVSKLTVDKSRWQQGNVFSCSVMHEALHNHYTQKSLSLSPGKGGGGSGGGGSGGGGSIWELKKDVYVVELDWYPDAPGEMVVLTCDTPEEDGITWTLDQSSEVLGSGKTLTIQVKEFGDAGQYTCHKGGEVLSHSLLLLHKKEDGIWSTDILKDQKEPKNKTFLRCEAKNYSGRFTCWWLTTISTDLTFSVKSSRGSSDPQGVTCGAATLSAERVRGDNKEYEYSVECQEDSACPAAEESLPIEVMVDAVHKLKYENYTSSFFIRDIIKPDPPKNLQLKPLKNSRQVEVSWEYPDTWSTPHSYFSLTFCVQVQGASAREAADRVFTDKTSATVICRKNASISVRAQDRYYSSSWSEWASVPCSGGGGSGGGGSGGGGSRNLPVATPDPGMFPCLHHSQNLLRAVSNMLQKARQTLEFYPCTSEEIDHEDITKDKTSTVEACLPLELTKNESCLNSRETSFITNGSCLASRKTSFMMALCLSSIYEDLKMYQVEFKTMNAKLLMDPKRQIFLDQNMLAVIDELMQALNFNSETVPQKSSLEEPDFYKTKIKLCILLHAFRIRAVTIDRVMSYLNAS

SEQ ID NO: 12 - protein, 451 aa, Artificial Sequence
  anti-hu CD20 HC hu IgG1 Fc knob DANG
QVQLQQPGAELVKPGASVKMSCKASGYTFTSYNMHWVKQTPGRGLEWIGAIYPGNGDTSYNQKFKGKATLTADKSSSTAYMQLSSLTSEDSAVYYCARSTYYGGDWYFNVWGAGTTVTVSAASTKGPSVFPLAPSSKSTSGGTAALGCLVKDYFPEPVTVSWNSGALTSGVHTFPAVLQSSGLYSLSSVVTVPSSSLGTQTYICNVNHKPSNTKVDKKVEPKSCDKTHTCPPCPAPELLGGPSVFLFPPKPKDTLMISRTPEVTCVVVAVSHEDPEVKFNWYVDGVEVHNAKTKPREEQYGSTYRVVSVLTVLHQDWLNGKEYKCKVSNKALPAPIEKTISKAKGQPREPQVYTLPPSRDELTKNQVSLWCLVKGFYPSDIAVEWESNGQPENNYKTTPPVLDSDGSFFLYSKLTVDKSRWQQGNVFSCSVMHEALHNHYTQKSLSLSPGK

SEQ ID NO: 13 - protein, 755 aa, Artificial Sequence
  hu scIL-12-hu IgG1 Fc hole DANG
IWELKKDVYVVELDWYPDAPGEMVVLTCDTPEEDGITWTLDQSSEVLGSGKTLTIQVKEFGDAGQYTCHKGGEVLSHSLLLLHKKEDGIWSTDILKDQKEPKNKTFLRCEAKNYSGRFTCWWLTTISTDLTFSVKSSRGSSDPQGVTCGAATLSAERVRGDNKEYEYSVECQEDSACPAAEESLPIEVMVDAVHKLKYENYTSSFFIRDIIKPDPPKNLQLKPLKNSRQVEVSWEYPDTWSTPHSYFSLTFCVQVQGKSKREKKDRVFTDKTSATVICRKNASISVRAQDRYYSSSWSEWASVPCSGGGGSGGGGSGGGGSRNLPVATPDPGMFPCLHHSQNLLRAVSNMLQKARQTLEFYPCTSEEIDHEDITKDKTSTVEACLPLELTKNESCLNSRETSFITNGSCLASRKTSFMMALCLSSIYEDLKMYQVEFKTMNAKLLMDPKRQIFLDQNMLAVIDELMQALNFNSETVPQKSSLEEPDFYKTKIKLCILLHAFRIRAVTIDRVMSYLNASGGGGSGGGGSDKTHTCPPCPAPELLGGPSVFLFPPKPKDTLMISRTPEVTCVVVAVSHEDPEVKFNWYVDGVEVHNAKTKPREEQYGSTYRVVSVLTVLHQDWLNGKEYKCKVSNKALPAPIEKTISKAKGQPREPQVYTLPPSRDELTKNQVSLSCAVKGFYPSDIAVEWESNGQPENNYKTTPPVLDSDGSFFLVSKLTVDKSRWQQGNVFSCSVMHEALHNHYTQKSLSLSPGK

SEQ ID NO: 14 - protein, 755 aa, Artificial Sequence
  hu scIL-12 mut1-hu IgG1 Fc hole DANG
IWELKKDVYVVELDWYPDAPGEMVVLTCDTPEEDGITWTLDQSSEVLGSGKTLTIQVKEFGDAGQYTCHKGGEVLSHSLLLLHKKEDGIWSTDILKDQKEPKNKTFLRCEAKNYSGRFTCWWLTTISTDLTFSVKSSRGSSDPQGVTCGAATLSAERVRGDNKEYEYSVECQEDSACPAAEESLPIEVMVDAVHKLKYENYTSSFFIRDIIKPDPPKNLQLKPLKNSRQVEVSWEYPDTWSTPHSYFSLTFCVQVQGASKREAKDRVFTDKTSATVICRKNASISVRAQDRYYSSSWSEWASVPCSGGGGSGGGGSGGGGSRNLPVATPDPGMFPCLHHSQNLLRAVSNMLQKARQTLEFYPCTSEEIDHEDITKDKTSTVEACLPLELTKNESCLNSRETSFITNGSCLASRKTSFMMALCLSSIYEDLKMYQVEFKTMNAKLLMDPKRQIFLDQNMLAVIDELMQALNFNSETVPQKSSLEEPDFYKTKIKLCILLHAFRIRAVTIDRVMSYLNASGGGGSGGGGSDKTHTCPPCPAPELLGGPSVFLFPPKPKDTLMISRTPEVTCVVVAVSHEDPEVKFNWYVDGVEVHNAKTKPREEQYGSTYRVVSVLTVLHQDWLNGKEYKCKVSNKALPAPIEKTISKAKGQPREPQVYTLPPSRDELTKNQVSLSCAVKGFYPSDIAVEWESNGQPENNYKTTPPVLDSDGSFFLVSKLTVDKSRWQQGNVFSCSVMHEALHNHYTQKSLSLSPGK

SEQ ID NO: 15 - protein, 755 aa, Artificial Sequence
  hu scIL-12 mut2-hu IgG1 Fc
IWELKKDVYVVELDWYPDAPGEMVVLTCDTPEEDGITWTLDQSSEVLGSGKTLTIQVKEFGDAGQYTCHKGGEVLSHSLLLLHKKEDGIWSTDILKDQKEPKNKTFLRCEAKNYSGRFTCWWLTTISTDLTFSVKSSRGSSDPQGVTCGAATLSAERVRGDNKEYEYSVECQEDSACPAAEESLPIEVMVDAVHKLKYENYTSSFFIRDIIKPDPPKNLQLKPLKNSRQVEVSWEYPDTWSTPHSYFSLTFCVQVQGASAREAADRVFTDKTSATVICRKNASISVRAQDRYYSSSWSEWASVPCSGGGGSGGGGSGGGGSRNLPVATPDPGMFPCLHHSQNLLRAVSNMLQKARQTLEFYPCTSEEIDHEDITKDKTSTVEACLPLELTKNESCLNSRETSFITNGSCLASRKTSFMMALCLSSIYEDLKMYQVEFKTMNAKLLMDPKRQIFLDQNMLAVIDELMQALNFNSETVPQKSSLEEPDFYKTKIKLCILLHAFRIRAVTIDRVMSYLNASGGGGSGGGGSDKTHTCPPCPAPELLGGPSVFLFPPKPKDTLMISRTPEVTCVVVDVSHEDPEVKFNWYVDGVEVHNAKTKPREEQYNSTYRVVSVLTVLHQDWLNGKEYKCKVSNKALPAPIEKTISKAKGQPREPQVYTLPPSRDELTKNQVSLTCLVKGFYPSDIAVEWESNGQPENNYKTTPPVLDSDGSFFLYSKLTVDKSRWQQGNVFSCSVMHEALHNHYTQKSLSLSPGK

SEQ ID NO: 16 - protein, 454 aa, Artificial Sequence
  anti-hu FAP HC IgG1 Fc knob
QVQLVQSGAEVKKPGASVKVSCKTSRYTFTEYTIHWVRQAPGQRLEWIGGINPNNGIPNYNQKFKGRVTITVDTSASTAYMELSSLRSEDTAVYYCARRRIAYGYDEGHAMDYWGQGTLVTVSSASTKGPSVFPLAPSSKSTSGGTAALGCLVKDYFPEPVTVSWNSGALTSGVHTFPAVLQSSGLYSLSSVVTVPSSSLGTQTYICNVNHKPSNTKVDKKVEPKSCDKTHTCPPCPAPELLGGPSVFLFPPKPKDTLMISRTPEVTCVVVDVSHEDPEVKFNWYVDGVEVHNAKTKPREEQYNSTYRVVSVLTVLHQDWLNGKEYKCKVSNKALPAPIEKTISKAKGQPREPQVYTLPPSRDELTKNQVSLWCLVKGFYPSDIAVEWESNGQPENNYKTTPPVLDSDGSFFLYSKLTVDKSRWQQGNVFSCSVMHEALHNHYTQKSLSLSPGK

SEQ ID NO: 17 - protein, 220 aa, Artificial Sequence
  anti-hu FAP LC
DIVMTQSPDSLAVSLGERATINCKSSQSLLYSRNQKNYLAWYQQKPGQPPKLLIFWASTRESGVPDRFSGSGFGTDFTLTISSLQAEDVAVYYCQQYFSYPLTFGQGTKVEIKRTVAAPSVFIFPPSDEQLKSGTASVVCLLNNFYPREAKVQWKVDNALQSGNSQESVTEQDSKDSTYSLSSTLTLSKADYEKHKVYACEVTHQGLSSPVTKSFNRGEC

SEQ ID NO: 18 - protein, 454 aa, Artificial Sequence
  anti-hu FAP HC hu IgG1 Fc knob DANG
QVQLVQSGAEVKKPGASVKVSCKTSRYTFTEYTIHWVRQAPGQRLEWIGGINPNNGIPNYNQKFKGRVTITVDTSASTAYMELSSLRSEDTAVYYCARRRIAYGYDEGHAMDYWGQGTLVTVSSASTKGPSVFPLAPSSKSTSGGTAALGCLVKDYFPEPVTVSWNSGALTSGVHTFPAVLQSSGLYSLSSVVTVPSSSLGTQTYICNVNHKPSNTKVDKKVEPKSCDKTHTCPPCPAPELLGGPSVFLFPPKPKDTLMISRTPEVTCVVVAVSHEDPEVKFNWYVDGVEVHNAKTKPREEQYGSTYRVVSVLTVLHQDWLNGKEYKCKVSNKALPAPIEKTISKAKGQPREPQVYTLPPSRDELTKNQVSLWCLVKGFYPSDIAVEWESNGQPENNYKTTPPVLDSDGSFFLYSKLTVDKSRWQQGNVFSCSVMHEALHNHYTQKSLSLSPGK

SEQ ID NO: 19 - protein, 227 aa, Artificial Sequence
  hu IgG1 Fc knob DANG
DKTHTCPPCPAPELLGGPSVFLFPPKPKDTLMISRTPEVTCVVVAVSHEDPEVKFNWYVDGVEVHNAKTKPREEQYGSTYRVVSVLTVLHQDWLNGKEYKCKVSNKALPAPIEKTISKAKGQPREPQVYTLPPSRDELTKNQVSLWCLVKGFYPSDIAVEWESNGQPENNYKTTPPVLDSDGSFFLYSKLTVDKSRWQQGNVFSCSVMHEALHNHYTQKSLSLSPGK

SEQ ID NO: 20 - protein, 227 aa, Artificial Sequence
  hu IgG1 Fc hole DANG
DKTHTCPPCPAPELLGGPSVFLFPPKPKDTLMISRTPEVTCVVVAVSHEDPEVKFNWYVDGVEVHNAKTKPREEQYGSTYRVVSVLTVLHQDWLNGKEYKCKVSNKALPAPIEKTISKAKGQPREPQVYTLPPSRDELTKNQVSLSCAVKGFYPSDIAVEWESNGQPENNYKTTPPVLDSDGSFFLVSKLTVDKSRWQQGNVFSCSVMHEALHNHYTQKSLSLSPGK

SEQ ID NO: 21 - protein, 451 aa, Artificial Sequence
  anti-hu CD20 (Rituximab) HC
QVQLQQPGAELVKPGASVKMSCKASGYTFTSYNMHWVKQTPGRGLEWIGAIYPGNGDTSYNQKFKGKATLTADKSSSTAYMQLSSLTSEDSAVYYCARSTYYGGDWYFNVWGAGTTVTVSAASTKGPSVFPLAPSSKSTSGGTAALGCLVKDYFPEPVTVSWNSGALTSGVHTFPAVLQSSGLYSLSSVVTVPSSSLGTQTYICNVNHKPSNTKVDKKVEPKSCDKTHTCPPCPAPELLGGPSVFLFPPKPKDTLMISRTPEVTCVVVDVSHEDPEVKFNWYVDGVEVHNAKTKPREEQYNSTYRVVSVLTVLHQDWLNGKEYKCKVSNKALPAPIEKTISKAKGQPREPQVYTLPPSRDELTKNQVSLTCLVKGFYPSDIAVEWESNGQPENNYKTTPPVLDSDGSFFLYSKLTVDKSRWQQGNVFSCSVMHEALHNHYTQKSLSLSPGK

SEQ ID NO: 22 - protein, 451 aa, Artificial Sequence
  anti-mu CD20 HC mu IgG2a Fc knob
QVQLQQPGAELVRPGTSVKLSCKASGYTFTSYWMHWIKQRPGQGLEWIGVIDPSDNYTKYNQKFKGKATLTVDTSSSTAYMQLSSLTSEDSAVYFCAREGYYGSSPWFAYWGQGTLVTVSSAKTTAPSVYPLAPVCGDTTGSSVTLGCLVKGYFPEPVTLTWNSGSLSSGVHTFPAVLQSDLYTLSSSVTVTSSTWPSQSITCNVAHPASSTKVDKKIEPRGPTIKPCPPCKCPAPNLLGGPSVFIFPPKIKDVLMISLSPIVTCVVVDVSEDDPDVQISWFVNNVEVHTAQTQTHREDYNSTLRVVSALPIQHQDWMSGKEFKCKVNNKDLPAPIERTISKPKGSVRAPQVYVLPPPEEEMTKKQVTLWCMVTDFMPEDIYVEWTNNGKTELNYKNTEPVLDSDGSYFMYSKLRVEKKNWVERNSYSCSVVHEGLHNHHTTKSFSRTPGK

SEQ ID NO: 23 - protein, 213 aa, Artificial Sequence
  anti-mu CD20 LC
QIVMSQSPAILSASPGEKVTMTCRARSSVSYIHWYQQKPGSSPKPWIYATSNLASGVPGRFSGSGSGTSYSLTITRVEAEDAATYYCQQWSSKPPTFGGGTKLEIKRTDAAPTVSIFPPSSEQLTSGGASVVCFLNNFYPKDINVKWKIDGSERQNGVLNSWTDQDSKDSTYSMSSTLTLTKDEYERHNSYTCEATHKTSTSPIVKSFNRNEC

SEQ ID NO: 24 - protein, 764 aa, Artificial Sequence
  mu scIL-12-mu IgG2a Fc hole
MWELEKDVYVVEVDWTPDAPGETVNLTCDTPEEDDITWTSDQRHGVIGSGKTLTITVKEFLDAGQYTCHKGGETLSHSHLLLHKKENGIWSTEILKNFKNKTFLKCEAPNYSGRFTCSWLVQRNMDLKFNIKSSSSSPDSRAVTCGMASLSAEKVTLDQRDYEKYSVSCQEDVTCPTAEETLPIELALEARQQNKYENYSTSFFIRDIIKPDPPKNLQMKPLKNSQVEVSWEYPDSWSTPHSYFSLKFFVRIQRKKEKMKETEEGCNQKGAFLVEKTSTEVQCKGGNVCVQAQDRYYNSSCSKWACVPCRVRSGGGGSGGGGSGGGGSRVIPVSGPARCLSQSRNLLKTTDDMVKTAREKLKHYSCTAEDIDHEDITRDQTSTLKTCLPLELHKNESCLATRETSSTTRGSCLPPQKTSLMMTLCLGSIYEDLKMYQTEFQAINAALQNHNHQQIILDKGMLVAIDELMQSLNHNGETLRQKPPVGEADPYRVKMKLCILLHAFSTRVVTINRVMGYLSSAGGGGSGGGGSEPRGPTIKPCPPCKCPAPNLLGGPSVFIFPPKIKDVLMISLSPIVTCVVVDVSEDDPDVQISWFVNNVEVHTAQTQTHREDYNSTLRVVSALPIQHQDWMSGKEFKCKVNNKDLPAPIERTISKPKGSVRAPQVYVLPPPEEEMTKKQVTLSCAVTDFMPEDIYVEWTNNGKTELNYKNTEPVLDSDGSYFMVSKLRVEKKNWVERNSYSCSVVHEGLHNHHTTKSFSRTPGK

SEQ ID NO: 25 - protein, 764 aa, Artificial Sequence
  mu scIL-12 mut1-mu IgG2a Fc hole
MWELEKDVYVVEVDWTPDAPGETVNLTCDTPEEDDITWTSDQRHGVIGSGKTLTITVKEFLDAGQYTCHKGGETLSHSHLLLHKKENGIWSTEILKNFKNKTFLKCEAPNYSGRFTCSWLVQRNMDLKFNIKSSSSSPDSRAVTCGMASLSAEKVTLDQRDYEKYSVSCQEDVTCPTAEETLPIELALEARQQNKYENYSTSFFIRDIIKPDPPKNLQMKPLKNSQVEVSWEYPDSWSTPHSYFSLKFFVRIQRAKEKMAETEEGCNQKGAFLVEKTSTEVQCKGGNVCVQAQDRYYNSSCSKWACVPCRVRSGGGGSGGGGSGGGGSRVIPVSGPARCLSQSRNLLKTTDDMVKTAREKLKHYSCTAEDIDHEDITRDQTSTLKTCLPLELHKNESCLATRETSSTTRGSCLPPQKTSLMMTLCLGSIYEDLKMYQTEFQAINAALQNHNHQQIILDKGMLVAIDELMQSLNHNGETLRQKPPVGEADPYRVKMKLCILLHAFSTRVVTINRVMGYLSSAGGGGSGGGGSEPRGPTIKPCPPCKCPAPNLLGGPSVFIFPPKIKDVLMISLSPIVTCVVVDVSEDDPDVQISWFVNNVEVHTAQTQTHREDYNSTLRVVSALPIQHQDWMSGKEFKCKVNNKDLPAPIERTISKPKGSVRAPQVYVLPPPEEEMTKKQVTLSCAVTDFMPEDIYVEWTNNGKTELNYKNTEPVLDSDGSYFMVSKLRVEKKNWVERNSYSCSVVHEGLHNHHTTKSFSRTPGK

SEQ ID NO: 26 - protein, 764 aa, Artificial Sequence
  mu scIL-12 mut2-mu IgG2a Fc hole
MWELEKDVYVVEVDWTPDAPGETVNLTCDTPEEDDITWTSDQRHGVIGSGKTLTITVKEFLDAGQYTCHKGGETLSHSHLLLHKKENGIWSTEILKNFKNKTFLKCEAPNYSGRFTCSWLVQRNMDLKFNIKSSSSSPDSRAVTCGMASLSAEKVTLDQRDYEKYSVSCQEDVTCPTAEETLPIELALEARQQNKYENYSTSFFIRDIIKPDPPKNLQMKPLKNSQVEVSWEYPDSWSTPHSYFSLKFFVRIQAAAEKMAETEEGCNQKGAFLVEKTSTEVQCKGGNVCVQAQDRYYNSSCSKWACVPCRVRSGGGGSGGGGSGGGGSRVIPVSGPARCLSQSRNLLKTTDDMVKTAREKLKHYSCTAEDIDHEDITRDQTSTLKTCLPLELHKNESCLATRETSSTTRGSCLPPQKTSLMMTLCLGSIYEDLKMYQTEFQAINAALQNHNHQQIILDKGMLVAIDELMQSLNHNGETLRQKPPVGEADPYRVKMKLCILLHAFSTRVVTINRVMGYLSSAGGGGSGGGGSEPRGPTIKPCPPCKCPAPNLLGGPSVFIFPPKIKDVLMISLSPIVTCVVVDVSEDDPDVQISWFVNNVEVHTAQTQTHREDYNSTLRVVSALPIQHQDWMSGKEFKCKVNNKDLPAPIERTISKPKGSVRAPQVYVLPPPEEEMTKKQVTLSCAVTDFMPEDIYVEWTNNGKTELNYKNTEPVLDSDGSYFMVSKLRVEKKNWVERNSYSCSVVHEGLHNHHTTKSFSRTPGK

SEQ ID NO: 27 - protein, 587 aa, Artificial Sequence
  (anti-mu CD20 VH)2-mu IgG2a Fc knob
QVQLQQPGAELVRPGTSVKLSCKASGYTFTSYWMHWIKQRPGQGLEWIGVIDPSDNYTKYNQKFKGKATLTVDTSSSTAYMQLSSLTSEDSAVYFCAREGYYGSSPWFAYWGQGTLVTVSSGGGGSGGGGSGGGGSQVQLQQPGAELVRPGTSVKLSCKASGYTFTSYWMHWIKQRPGQGLEWIGVIDPSDNYTKYNQKFKGKATLTVDTSSSTAYMQLSSLTSEDSAVYFCAREGYYGSSPWFAYWGQGTLVTVSSAKTTAPSVYPLAPVCGDTTGSSVTLGCLVKGYFPEPVTLTWNSGSLSSGVHTFPAVLQSDLYTLSSSVTVTSSTWPSQSITCNVAHPASSTKVDKKIEPRGPTIKPCPPCKCPAPNLLGGPSVFIFPPKIKDVLMISLSPIVTCVVVDVSEDDPDVQISWFVNNVEVHTAQTQTHREDYNSTLRVVSALPIQHQDWMSGKEFKCKVNNKDLPAPIERTISKPKGSVRAPQVYVLPPPEEEMTKKQVTLWCMVTDFMPEDIYVEWTNNGKTELNYKNTEPVLDSDGSYFMYSKLRVEKKNWVERNSYSCSVVHEGLHNHHTTKSFSRTPGK

SEQ ID NO: 28 - protein, 334 aa, Artificial Sequence
  (anti-mu CD20 VL)2
QIVMSQSPAILSASPGEKVTMTCRARSSVSYIHWYQQKPGSSPKPWIYATSNLASGVPGRFSGSGSGTSYSLTITRVEAEDAATYYCQQWSSKPPTFGGGTKLEIKGGGGSGGGGSGGGGSQIVMSQSPAILSASPGEKVTMTCRARSSVSYIHWYQQKPGSSPKPWIYATSNLASGVPGRFSGSGSGTSYSLTITRVEAEDAATYYCQQWSSKPPTFGGGTKLEIKRTDAAPTVSIFPPSSEQLTSGGASVVCFLNNFYPKDINVKWKIDGSERQNGVLNSWTDQDSKDSTYSMSSTLTLTKDEYERHNSYTCEATHKTSTSPIVKSFNRNEC

SEQ ID NO: 29 - protein, 713 aa, Artificial Sequence
  anti-mu CD20 HC mu IgG2a Fc knob-anti-mu CD20 scFv
QVQLQQPGAELVRPGTSVKLSCKASGYTFTSYWMHWIKQRPGQGLEWIGVIDPSDNYTKYNQKFKGKATLTVDTSSSTAYMQLSSLTSEDSAVYFCAREGYYGSSPWFAYWGQGTLVTVSSAKTTAPSVYPLAPVCGDTTGSSVTLGCLVKGYFPEPVTLTWNSGSLSSGVHTFPAVLQSDLYTLSSSVTVTSSTWPSQSITCNVAHPASSTKVDKKIEPRGPTIKPCPPCKCPAPNLLGGPSVFIFPPKIKDVLMISLSPIVTCVVVDVSEDDPDVQISWFVNNVEVHTAQTQTHREDYNSTLRVVSALPIQHQDWMSGKEFKCKVNNKDLPAPIERTISKPKGSVRAPQVYVLPPPEEEMTKKQVTLWCMVTDFMPEDIYVEWTNNGKTELNYKNTEPVLDSDGSYFMYSKLRVEKKNWVERNSYSCSVVHEGLHNHHTTKSFSRTPGKGGGGSGGGGSGGGGSQVQLQQPGAELVRPGTSVKLSCKASGYTFTSYWMHWIKQRPGQGLEWIGVIDPSDNYTKYNQKFKGKATLTVDTSSSTAYMQLSSLTSEDSAVYFCAREGYYGSSPWFAYWGQGTLVTVSSGGGGSGGGGSGGGGSGGGGSQIVMSQSPAILSASPGEKVTMTCRARSSVSYIHWYQQKPGSSPKPWIYATSNLASGVPGRFSGSGSGTSYSLTITRVEAEDAATYYCQQWSSKPPTFGGGTKLEIK

SEQ ID NO: 30 - protein, 475 aa, Artificial Sequence
  anti-mu CD20 LC-anti-mu CD20 scFv
QIVMSQSPAILSASPGEKVTMTCRARSSVSYIHWYQQKPGSSPKPWIYATSNLASGVPGRFSGSGSGTSYSLTITRVEAEDAATYYCQQWSSKPPTFGGGTKLEIKRTDAAPTVSIFPPSSEQLTSGGASVVCFLNNFYPKDINVKWKIDGSERQNGVLNSWTDQDSKDSTYSMSSTLTLTKDEYERHNSYTCEATHKTSTSPIVKSFNRNECGGGGSGGGGSGGGGSQVQLQQPGAELVRPGTSVKLSCKASGYTFTSYWMHWIKQRPGQGLEWIGVIDPSDNYTKYNQKFKGKATLTVDTSSSTAYMQLSSLTSEDSAVYFCAREGYYGSSPWFAYWGQGTLVTVSSGGGGSGGGGSGGGGSGGGGSQIVMSQSPAILSASPGEKVTMTCRARSSVSYIHWYQQKPGSSPKPWIYATSNLASGVPGRFSGSGSGTSYSLTITRVEAEDAATYYCQQWSSKPPTFGGGTKLEIK

SEQ ID NO: 31 - protein, 987 aa, Artificial Sequence
  anti-mu CD20 HC mu IgG2a Fc hole-mu scIL-12
QVQLQQPGAELVRPGTSVKLSCKASGYTFTSYWMHWIKQRPGQGLEWIGVIDPSDNYTKYNQKFKGKATLTVDTSSSTAYMQLSSLTSEDSAVYFCAREGYYGSSPWFAYWGQGTLVTVSSAKTTAPSVYPLAPVCGDTTGSSVTLGCLVKGYFPEPVTLTWNSGSLSSGVHTFPAVLQSDLYTLSSSVTVTSSTWPSQSITCNVAHPASSTKVDKKIEPRGPTIKPCPPCKCPAPNLLGGPSVFIFPPKIKDVLMISLSPIVTCVVVDVSEDDPDVQISWFVNNVEVHTAQTQTHREDYNSTLRVVSALPIQHQDWMSGKEFKCKVNNKDLPAPIERTISKPKGSVRAPQVYVLPPPEEEMTKKQVTLSCAVTDFMPEDIYVEWTNNGKTELNYKNTEPVLDSDGSYFMVSKLRVEKKNWVERNSYSCSVVHEGLHNHHTTKSFSRTPGKGGGGSGGGGSGGGGSMWELEKDVYVVEVDWTPDAPGETVNLTCDTPEEDDITWTSDQRHGVIGSGKTLTITVKEFLDAGQYTCHKGGETLSHSHLLLHKKENGIWSTEILKNFKNKTFLKCEAPNYSGRFTCSWLVQRNMDLKFNIKSSSSSPDSRAVTCGMASLSAEKVTLDQRDYEKYSVSCQEDVTCPTAEETLPIELALEARQQNKYENYSTSFFIRDIIKPDPPKNLQMKPLKNSQVEVSWEYPDSWSTPHSYFSLKFFVRIQRKKEKMKETEEGCNQKGAFLVEKTSTEVQCKGGNVCVQAQDRYYNSSCSKWACVPCRVRSGGGGSGGGGSGGGGSRVIPVSGPARCLSQSRNLLKTTDDMVKTAREKLKHYSCTAEDIDHEDITRDQTSTLKTCLPLELHKNESCLATRETSSTTRGSCLPPQKTSLMMTLCLGSIYEDLKMYQTEFQAINAALQNHNHQQIILDKGMLVAIDELMQSLNHNGETLRQKPPVGEADPYRVKMKLCILLHAFSTRVVTINRVMGYLSSA

SEQ ID NO: 32 - protein, 987 aa, Artificial Sequence
  anti-mu CD20 HC mu IgG2a Fc hole-mu scIL-12 mut2
QVQLQQPGAELVRPGTSVKLSCKASGYTFTSYWMHWIKQRPGQGLEWIGVIDPSDNYTKYNQKFKGKATLTVDTSSSTAYMQLSSLTSEDSAVYFCAREGYYGSSPWFAYWGQGTLVTVSSAKTTAPSVYPLAPVCGDTTGSSVTLGCLVKGYFPEPVTLTWNSGSLSSGVHTFPAVLQSDLYTLSSSVTVTSSTWPSQSITCNVAHPASSTKVDKKIEPRGPTIKPCPPCKCPAPNLLGGPSVFIFPPKIKDVLMISLSPIVTCVVVDVSEDDPDVQISWFVNNVEVHTAQTQTHREDYNSTLRVVSALPIQHQDWMSGKEFKCKVNNKDLPAPIERTISKPKGSVRAPQVYVLPPPEEEMTKKQVTLSCAVTDFMPEDIYVEWTNNGKTELNYKNTEPVLDSDGSYFMVSKLRVEKKNWVERNSYSCSVVHEGLHNHHTTKSFSRTPGKGGGGSGGGGSGGGGSMWELEKDVYVVEVDWTPDAPGETVNLTCDTPEEDDITWTSDQRHGVIGSGKTLTITVKEFLDAGQYTCHKGGETLSHSHLLLHKKENGIWSTEILKNFKNKTFLKCEAPNYSGRFTCSWLVQRNMDLKFNIKSSSSSPDSRAVTCGMASLSAEKVTLDQRDYEKYSVSCQEDVTCPTAEETLPIELALEARQQNKYENYSTSFFIRDIIKPDPPKNLQMKPLKNSQVEVSWEYPDSWSTPHSYFSLKFFVRIQAAAEKMAETEEGCNQKGAFLVEKTSTEVQCKGGNVCVQAQDRYYNSSCSKWACVPCRVRSGGGGSGGGGSGGGGSRVIPVSGPARCLSQSRNLLKTTDDMVKTAREKLKHYSCTAEDIDHEDITRDQTSTLKTCLPLELHKNESCLATRETSSTTRGSCLPPQKTSLMMTLCLGSIYEDLKMYQTEFQAINAALQNHNHQQIILDKGMLVAIDELMQSLNHNGETLRQKPPVGEADPYRVKMKLCILLHAFSTRVVTINRVMGYLSSA

SEQ ID NO: 33 - protein, 451 aa, Artificial Sequence
  anti-mu CD20 HC mu IgG2a Fc knob DANG
QVQLQQPGAELVRPGTSVKLSCKASGYTFTSYWMHWIKQRPGQGLEWIGVIDPSDNYTKYNQKFKGKATLTVDTSSSTAYMQLSSLTSEDSAVYFCAREGYYGSSPWFAYWGQGTLVTVSSAKTTAPSVYPLAPVCGDTTGSSVTLGCLVKGYFPEPVTLTWNSGSLSSGVHTFPAVLQSDLYTLSSSVTVTSSTWPSQSITCNVAHPASSTKVDKKIEPRGPTIKPCPPCKCPAPNLLGGPSVFIFPPKIKDVLMISLSPIVTCVVVAVSEDDPDVQISWFVNNVEVHTAQTQTHREDYGSTLRVVSALPIQHQDWMSGKEFKCKVNNKDLPAPIERTISKPKGSVRAPQVYVLPPPEEEMTKKQVTLWCMVTDFMPEDIYVEWTNNGKTELNYKNTEPVLDSDGSYFMYSKLRVEKKNWVERNSYSCSVVHEGLHNHHTTKSFSRTPGK

SEQ ID NO: 34 - protein, 764 aa, Artificial Sequence
  mu scIL-12-mu IgG2a Fc hole DANG
MWELEKDVYVVEVDWTPDAPGETVNLTCDTPEEDDITWTSDQRHGVIGSGKTLTITVKEFLDAGQYTCHKGGETLSHSHLLLHKKENGIWSTEILKNFKNKTFLKCEAPNYSGRFTCSWLVQRNMDLKFNIKSSSSSPDSRAVTCGMASLSAEKVTLDQRDYEKYSVSCQEDVTCPTAEETLPIELALEARQQNKYENYSTSFFIRDIIKPDPPKNLQMKPLKNSQVEVSWEYPDSWSTPHSYFSLKFFVRIQRKKEKMKETEEGCNQKGAFLVEKTSTEVQCKGGNVCVQAQDRYYNSSCSKWACVPCRVRSGGGGSGGGGSGGGGSRVIPVSGPARCLSQSRNLLKTTDDMVKTAREKLKHYSCTAEDIDHEDITRDQTSTLKTCLPLELHKNESCLATRETSSTTRGSCLPPQKTSLMMTLCLGSIYEDLKMYQTEFQAINAALQNHNHQQIILDKGMLVAIDELMQSLNHNGETLRQKPPVGEADPYRVKMKLCILLHAFSTRVVTINRVMGYLSSAGGGGSGGGGSEPRGPTIKPCPPCKCPAPNLLGGPSVFIFPPKIKDVLMISLSPIVTCVVVAVSEDDPDVQISWFVNNVEVHTAQTQTHREDYGSTLRVVSALPIQHQDWMSGKEFKCKVNNKDLPAPIERTISKPKGSVRAPQVYVLPPPEEEMTKKQVTLSCAVTDFMPEDIYVEWTNNGKTELNYKNTEPVLDSDGSYFMVSKLRVEKKNWVERNSYSCSVVHEGLHNHHTTKSFSRTPGK

SEQ ID NO: 35 - protein, 764 aa, Artificial Sequence
  mu scIL-12 mut1-mu IgG2a Fc hole DANG
MWELEKDVYVVEVDWTPDAPGETVNLTCDTPEEDDITWTSDQRHGVIGSGKTLTITVKEFLDAGQYTCHKGGETLSHSHLLLHKKENGIWSTEILKNFKNKTFLKCEAPNYSGRFTCSWLVQRNMDLKFNIKSSSSSPDSRAVTCGMASLSAEKVTLDQRDYEKYSVSCQEDVTCPTAEETLPIELALEARQQNKYENYSTSFFIRDIIKPDPPKNLQMKPLKNSQVEVSWEYPDSWSTPHSYFSLKFFVRIQRAKEKMAETEEGCNQKGAFLVEKTSTEVQCKGGNVCVQAQDRYYNSSCSKWACVPCRVRSGGGGSGGGGSGGGGSRVIPVSGPARCLSQSRNLLKTTDDMVKTAREKLKHYSCTAEDIDHEDITRDQTSTLKTCLPLELHKNESCLATRETSSTTRGSCLPPQKTSLMMTLCLGSIYEDLKMYQTEFQAINAALQNHNHQQIILDKGMLVAIDELMQSLNHNGETLRQKPPVGEADPYRVKMKLCILLHAFSTRVVTINRVMGYLSSAGGGGSGGGGSEPRGPTIKPCPPCKCPAPNLLGGPSVFIFPPKIKDVLMISLSPIVTCVVVAVSEDDPDVQISWFVNNVEVHTAQTQTHREDYGSTLRVVSALPIQHQDWMSGKEFKCKVNNKDLPAPIERTISKPKGSVRAPQVYVLPPPEEEMTKKQVTLSCAVTDFMPEDIYVEWTNNGKTELNYKNTEPVLDSDGSYFMVSKLRVEKKNWVERNSYSCSVVHEGLHNHHTTKSFSRTPGK

SEQ ID NO: 36 - protein, 764 aa, Artificial Sequence
  mu scIL-12 mut2-mu IgG2a Fc
MWELEKDVYVVEVDWTPDAPGETVNLTCDTPEEDDITWTSDQRHGVIGSGKTLTITVKEFLDAGQYTCHKGGETLSHSHLLLHKKENGIWSTEILKNFKNKTFLKCEAPNYSGRFTCSWLVQRNMDLKFNIKSSSSSPDSRAVTCGMASLSAEKVTLDQRDYEKYSVSCQEDVTCPTAEETLPIELALEARQQNKYENYSTSFFIRDIIKPDPPKNLQMKPLKNSQVEVSWEYPDSWSTPHSYFSLKFFVRIQAAAEKMAETEEGCNQKGAFLVEKTSTEVQCKGGNVCVQAQDRYYNSSCSKWACVPCRVRSGGGGSGGGGSGGGGSRVIPVSGPARCLSQSRNLLKTTDDMVKTAREKLKHYSCTAEDIDHEDITRDQTSTLKTCLPLELHKNESCLATRETSSTTRGSCLPPQKTSLMMTLCLGSIYEDLKMYQTEFQAINAALQNHNHQQIILDKGMLVAIDELMQSLNHNGETLRQKPPVGEADPYRVKMKLCILLHAFSTRVVTINRVMGYLSSAGGGGSGGGGSEPRGPTIKPCPPCKCPAPNLLGGPSVFIFPPKIKDVLMISLSPIVTCVVVDVSEDDPDVQISWFVNNVEVHTAQTQTHREDYNSTLRVVSALPIQHQDWMSGKEFKCKVNNKDLPAPIERTISKPKGSVRAPQVYVLPPPEEEMTKKQVTLTCMVTDFMPEDIYVEWTNNGKTELNYKNTEPVLDSDGSYFMYSKLRVEKKNWVERNSYSCSVVHEGLHNHHTTKSFSRTPGK

SEQ ID NO: 37 - protein, 447 aa, Artificial Sequence
  anti-mu FAP HC mu IgG2a Fc knob
QVQLQQSGAELARPGASVNLSCKASGYTFTNNGINWLKQRTGQGLEWIGEIYPRSTNTLYNEKFKGKATLTADRSSNTAYMELRSLTSEDSAVYFCARTLTAPFAFWGQGTLVTVSAAKTTAPSVYPLAPVCGDTTGSSVTLGCLVKGYFPEPVTLTWNSGSLSSGVHTFPAVLQSDLYTLSSSVTVTSSTWPSQSITCNVAHPASSTKVDKKIEPRGPTIKPCPPCKCPAPNLLGGPSVFIFPPKIKDVLMISLSPIVTCVVVDVSEDDPDVQISWFVNNVEVHTAQTQTHREDYNSTLRVVSALPIQHQDWMSGKEFKCKVNNKDLPAPIERTISKPKGSVRAPQVYVLPPPEEEMTKKQVTLWCMVTDFMPEDIYVEWTNNGKTELNYKNTEPVLDSDGSYFMYSKLRVEKKNWVERNSYSCSVVHEGLHNHHTTKSFSRTPGK

SEQ ID NO: 38 - protein, 213 aa, Artificial Sequence
  anti-mu FAP LC
QIVLTQSPAIMSASPGEKVTMTCSASSGVNFMHWYQQKSGTSPKRWIFDTSKLASGVPARFSGSGSGTSYSLTISSMEAEDAATYYCQQWSFNPPTFGGGTKLEIKRADAAPTVSIFPPSSEQLTSGGASVVCFLNNFYPKDINVKWKIDGSERQNGVLNSWTDQDSKDSTYSMSSTLTLTKDEYERHNSYTCEATHKTSTSPIVKSFNRNEC

SEQ ID NO: 39 - protein, 447 aa, Artificial Sequence
  anti-mu FAP HC mu IgG2a Fc knob DANG
QVQLQQSGAELARPGASVNLSCKASGYTFTNNGINWLKQRTGQGLEWIGEIYPRSTNTLYNEKFKGKATLTADRSSNTAYMELRSLTSEDSAVYFCARTLTAPFAFWGQGTLVTVSAAKTTAPSVYPLAPVCGDTTGSSVTLGCLVKGYFPEPVTLTWNSGSLSSGVHTFPAVLQSDLYTLSSSVTVTSSTWPSQSITCNVAHPASSTKVDKKIEPRGPTIKPCPPCKCPAPNLLGGPSVFIFPPKIKDVLMISLSPIVTCVVVAVSEDDPDVQISWFVNNVEVHTAQTQTHREDYGSTLRVVSALPIQHQDWMSGKEFKCKVNNKDLPAPIERTISKPKGSVRAPQVYVLPPPEEEMTKKQVTLWCMVTDFMPEDIYVEWTNNGKTELNYKNTEPVLDSDGSYFMYSKLRVEKKNWVERNSYSCSVVHEGLHNHHTTKSFSRTPGK

SEQ ID NO: 40 - protein, 233 aa, Artificial Sequence
  mu IgG2a Fc knob DANG
EPRGPTIKPCPPCKCPAPNLLGGPSVFIFPPKIKDVLMISLSPIVTCVVVAVSEDDPDVQISWFVNNVEVHTAQTQTHREDYGSTLRVVSALPIQHQDWMSGKEFKCKVNNKDLPAPIERTISKPKGSVRAPQVYVLPPPEEEMTKKQVTLWCMVTDFMPEDIYVEWTNNGKTELNYKNTEPVLDSDGSYFMYSKLRVEKKNWVERNSYSCSVVHEGLHNHHTTKSFSRTPGK

SEQ ID NO: 41 - protein, 233 aa, Artificial Sequence; identical to SEQ ID NO: 40
  mu IgG2a Fc hole DANG

SEQ ID NO: 42 - protein, 451 aa, Artificial Sequence
  anti-mu CD20 (18B12) HC
QVQLQQPGAELVRPGTSVKLSCKASGYTFTSYWMHWIKQRPGQGLEWIGVIDPSDNYTKYNQKFKGKATLTVDTSSSTAYMQLSSLTSEDSAVYFCAREGYYGSSPWFAYWGQGTLVTVSSAKTTAPSVYPLAPVCGDTTGSSVTLGCLVKGYFPEPVTLTWNSGSLSSGVHTFPAVLQSDLYTLSSSVTVTSSTWPSQSITCNVAHPASSTKVDKKIEPRGPTIKPCPPCKCPAPNLLGGPSVFIFPPKIKDVLMISLSPIVTCVVVDVSEDDPDVQISWFVNNVEVHTAQTQTHREDYNSTLRVVSALPIQHQDWMSGKEFKCKVNNKDLPAPIERTISKPKGSVRAPQVYVLPPPEEEMTKKQVTLTCMVTDFMPEDIYVEWTNNGKTELNYKNTEPVLDSDGSYFMYSKLRVEKKNWVERNSYSCSVVHEGLHNHHTTKSFSRTPGK

SEQ ID NO: 43 - DNA, 1353 bp, Artificial Sequence
  anti-hu CD20 HC hu IgG1 Fc knob
caggtgcagctgcagcagccaggagcagagctggtgaagcctggagcctctgtgaagatgagctgcaaggcctccggctacaccttcacaagctataacatgcactgggtgaagcagaccccaggaaggggactggagtggatcggagccatctaccctggcaacggcgacacatcctataatcagaagtttaagggcaaggccaccctgacagccgataagagctcctctaccgcctacatgcagctgagctccctgacaagcgaggactccgccgtgtactattgcgccagaagcacctactatggcggcgattggtacttcaacgtgtggggagcaggaaccacagtgaccgtgtctgccgccagcacaaagggaccatccgtgtttccactggcaccatctagcaagtctaccagcggaggaacagccgccctgggatgtctggtgaaggactacttcccagagcccgtgaccgtgtcctggaactctggcgccctgacctccggagtgcacacatttcccgccgtgctgcagtcctctggcctgtactctctgagctccgtggtgaccgtgccttctagctccctgggcacccagacatatatctgcaacgtgaatcacaagccttccaatacaaaggtggacaagaaggtggagccaaagtcttgtgataagacccacacatgccccccttgtcctgcaccagagctgctgggaggaccaagcgtgttcctgtttccacccaagcccaaggacaccctgatgatcagcaggacccctgaggtgacatgcgtggtggtggacgtgtcccacgaggacccagaggtgaagttcaactggtacgtggatggcgtggaggtgcacaatgccaagacaaagccacgggaggagcagtacaactctacctatagagtggtgagcgtgctgacagtgctgcaccaggattggctgaacggcaaggagtataagtgcaaggtgtctaataaggccctgcccgcccctatcgagaagaccatcagcaaggccaagggccagcctagggagccacaggtgtacaccctgcctccatctcgcgacgagctgacaaagaaccaggtgagcctgtggtgtctggtgaagggcttctatccaagcgatatcgccgtggagtgggagtccaatggccagcccgagaacaattacaagaccacaccccctgtgctggacagcgatggctccttctttctgtattccaagctgaccgtggataagtctagatggcagcagggcaacgtgttttcctgttctgtgatgcacgaggccctgcacaatcactacacacagaagagcctgtccctgtctcctggcaag

SEQ ID NO: 44 - DNA, 639 bp, Artificial Sequence
  anti-hu CD20 LC
cagatcgtgctgagccagtccccagcaatcctgtctgccagccctggagagaaggtgaccatgacatgccgggccagctcctctgtgagctacatccactggttccagcagaagccaggcagctcccctaagccatggatctatgccacaagcaacctggcatccggagtgcccgtgcggttttccggctctggcagcggcacctcctactctctgacaatcagcagagtggaggcagaggacgcagcaacctactattgccagcagtggacctccaatccccctacattcggcggcggcaccaagctggagatcaagaggacagtggccgccccttccgtgttcatctttccaccctctgacgagcagctgaagtctggcaccgccagcgtggtgtgcctgctgaacaacttctacccacgcgaggccaaggtgcagtggaaggtggataacgccctgcagagcggcaattcccaggagtctgtgacagagcaggacagcaaggattccacctattctctgtctagcaccctgacactgagcaaggccgattacgagaagcacaaggtgtatgcctgcgaggtgacacaccagggcctgtcctctcccgtgaccaagtccttcaacaggggcgagtgt

SEQ ID NO: 45 - DNA, 2265 bp, Artificial Sequence
  hu scIL-12-hu IgG1 Fc hole
atctgggagctgaagaaggacgtgtacgtggtggagctggactggtatcctgatgccccaggcgagatggtggtgctgacctgcgacacacccgaggaggatggcatcacctggacactggatcagagctccgaggtgctgggcagcggcaagaccctgacaatccaggtgaaggagttcggcgacgccggccagtacacctgtcacaagggaggagaggtgctgagccactccctgctgctgctgcacaagaaggaggacggcatctggagcacagacatcctgaaggatcagaaggagccaaagaacaagaccttcctgcggtgcgaggccaagaattattccggccggttcacctgttggtggctgaccacaatctccaccgatctgacattttctgtgaagtctagcaggggctcctctgacccccagggagtgacatgcggagcagccaccctgagcgccgagcgggtgagaggcgataacaaggagtacgagtattccgtggagtgccaggaggactctgcctgtcctgcagcagaggagtccctgccaatcgaagtgatggtggatgccgtgcacaagctgaagtacgagaattatacaagctccttctttatcagggacatcatcaagcctgatccccctaagaacctgcagctgaagccactgaagaatagccgccaggtggaggtgtcctgggagtacccagacacctggtccacaccccactcttatttcagcctgaccttttgcgtgcaggtgcagggcaagtccaagagggagaagaaggaccgcgtgttcaccgataagacatctgccaccgtgatctgtcggaagaacgcctctatcagcgtgcgggcccaggatagatactattctagctcctggagcgagtgggcctccgtgccttgttctggaggaggaggcagcggcggaggaggctccggaggaggaggctctagaaatctgccagtggcaacccctgacccaggaatgttcccttgcctgcaccactctcagaacctgctgcgggccgtgagcaatatgctgcagaaggccagacagacactggagttttacccctgtaccagcgaggagatcgaccacgaggatatcacaaaggataagacctccacagtggaggcctgcctgcctctggagctgaccaagaacgagagctgtctgaacagccgggagacatctttcatcaccaacggcagctgcctggcctccagaaagacatcttttatgatggccctgtgcctgtctagcatctacgaggacctgaagatgtatcaggtggagttcaagaccatgaacgccaagctgctgatggacccaaagcggcagatctttctggatcagaatatgctggccgtgatcgacgagctgatgcaggccctgaacttcaatagcgagacagtgccccagaagtcctctctggaggagcctgacttctacaagaccaagatcaagctgtgcatcctgctgcacgccttccggatcagagccgtgaccatcgatagagtgatgagctatctgaacgcaagcggcggcggaggctctggaggaggcggcagcgacaagacccacacatgcccaccatgtccagcacctgagctgctgggaggaccatccgtgttcctgtttcctccaaagcccaaggatacactgatgatcagccgcacacctgaggtgacctgcgtggtggtggacgtgtcccacgaggaccccgaggtgaagtttaactggtacgtggacggcgtggaggtgcacaatgccaagaccaagcccagggaggagcagtacaactctacatatcgcgtggtgagcgtgctgaccgtgctgcaccaggactggctgaacggcaaggagtacaagtgcaaggtgtctaataaggccctgccagcccccatcgagaagaccatcagcaaggcaaagggacagccaagggagcctcaggtgtatacactgccccctagccgcgatgagctgaccaagaaccaggtgtccctgtcttgtgccgtgaagggcttctacccatccgacatcgccgtggagtgggagtctaatggccagcccgagaacaattataagaccacaccacccgtgctggactccgatggctctttctttctggtgagcaagctgacagtggacaagtccagatggcagcagggcaacgtgtttagctgctccgtgatgcacgaggccctgcacaatcactacacccagaagtctctgagcctgtcccctggcaag

SEQ ID NO: 46 - DNA, 2265 bp, Artificial Sequence
  hu scIL-12 mut1-hu IgG1 Fc hole
atctgggagctgaagaaggacgtgtacgtggtggagctggactggtatcctgatgccccaggcgagatggtggtgctgacctgcgacacacccgaggaggatggcatcacctggacactggatcagagctccgaggtgctgggcagcggcaagaccctgacaatccaggtgaaggagttcggcgacgccggccagtacacctgtcacaagggaggagaggtgctgagccactccctgctgctgctgcacaagaaggaggacggcatctggagcacagacatcctgaaggatcagaaggagccaaagaacaagaccttcctgcggtgcgaggccaagaattattccggccggttcacctgttggtggctgaccacaatctccaccgatctgacattttctgtgaagtctagcaggggctcctctgacccccagggagtgacatgcggagcagccaccctgagcgccgagcgggtgagaggcgataacaaggagtacgagtattccgtggagtgccaggaggactctgcctgtcctgcagcagaggagtccctgccaatcgaagtgatggtggatgccgtgcacaagctgaagtacgagaattatacaagctccttctttatcagggacatcatcaagcctgatccccctaagaacctgcagctgaagccactgaagaatagccgccaggtggaggtgtcctgggagtacccagacacctggtccacaccccactcttatttcagcctgaccttttgcgtgcaggtgcagggagcatccaagagggaggcaaaggaccgcgtgttcaccgataagacatctgccaccgtgatctgtcggaagaacgcctctatcagcgtgcgggcccaggatagatactattctagctcctggagcgagtgggcctccgtgccttgttctggaggaggaggcagcggcggaggaggctccggaggaggaggctctagaaatctgccagtggcaacccctgacccaggaatgttcccttgcctgcaccactctcagaacctgctgcgggccgtgagcaatatgctgcagaaggccagacagacactggagttttacccctgtaccagcgaggagatcgaccacgaggatatcacaaaggataagacctccacagtggaggcctgcctgcctctggagctgaccaagaacgagagctgtctgaacagccgggagacatctttcatcaccaacggcagctgcctggcctccagaaagacatcttttatgatggccctgtgcctgtctagcatctacgaggacctgaagatgtatcaggtggagttcaagaccatgaacgccaagctgctgatggacccaaagcggcagatctttctggatcagaatatgctggccgtgatcgacgagctgatgcaggccctgaacttcaatagcgagacagtgccccagaagtcctctctggaggagcctgacttctacaagaccaagatcaagctgtgcatcctgctgcacgccttccggatcagagccgtgaccatcgatagagtgatgagctatctgaacgcaagcggcggcggaggctctggaggaggcggcagcgacaagacccacacatgcccaccatgtccagcacctgagctgctgggaggaccatccgtgttcctgtttcctccaaagcccaaggatacactgatgatcagccgcacacctgaggtgacctgcgtggtggtggacgtgtcccacgaggaccccgaggtgaagtttaactggtacgtggacggcgtggaggtgcacaatgccaagaccaagcccagggaggagcagtacaactctacatatcgcgtggtgagcgtgctgaccgtgctgcaccaggactggctgaacggcaaggagtacaagtgcaaggtgtctaataaggccctgccagcccccatcgagaagaccatcagcaaggcaaagggacagccaagggagcctcaggtgtatacactgccccctagccgcgatgagctgaccaagaaccaggtgtccctgtcttgtgccgtgaagggcttctacccatccgacatcgccgtggagtgggagtctaatggccagcccgagaacaattataagaccacaccacccgtgctggactccgatggctctttctttctggtgagcaagctgacagtggacaagtccagatggcagcagggcaacgtgtttagctgctccgtgatgcacgaggccctgcacaatcactacacccagaagtctctgagcctgtcccctggcaag

SEQ ID NO: 47 - DNA, 2268 bp, Artificial Sequence
  hu scIL-12 mut2-hu IgG1 Fc hole
atctgggagctgaagaaggacgtgtacgtggtggagctggactggtatcctgatgccccaggcgagatggtggtgctgacctgcgacacacccgaggaggatggcatcacctggacactggatcagagctccgaggtgctgggcagcggcaagaccctgacaatccaggtgaaggagttcggcgacgccggccagtacacctgtcacaagggaggagaggtgctgagccactccctgctgctgctgcacaagaaggaggacggcatctggagcacagacatcctgaaggatcagaaggagccaaagaacaagaccttcctgcggtgcgaggccaagaattattccggccggttcacctgttggtggctgaccacaatctccaccgatctgacattttctgtgaagtctagcaggggctcctctgacccccagggagtgacatgcggagcagccaccctgagcgccgagcgggtgagaggcgataacaaggagtacgagtattccgtggagtgccaggaggactctgcctgtcctgcagcagaggagtccctgccaatcgaagtgatggtggatgccgtgcacaagctgaagtacgagaattatacaagctccttctttatcagggacatcatcaagcctgatccccctaagaacctgcagctgaagccactgaagaatagccgccaggtggaggtgtcctgggagtacccagacacctggtccacaccccactcttatttcagcctgaccttttgcgtgcaggtgcagggcgcctccgctagggaggccgctgaccgcgtgttcaccgataagacatctgccaccgtgatctgtcggaagaacgcctctatcagcgtgcgggcccaggatagatactattctagctcctggagcgagtgggcctccgtgccttgttctggaggaggaggcagcggcggaggaggctccggaggaggaggctctagaaatctgccagtggcaacccctgacccaggaatgttcccttgcctgcaccactctcagaacctgctgcgggccgtgagcaatatgctgcagaaggccagacagacactggagttttacccctgtaccagcgaggagatcgaccacgaggatatcacaaaggataagacctccacagtggaggcctgcctgcctctggagctgaccaagaacgagagctgtctgaacagccgggagacatctttcatcaccaacggcagctgcctggcctccagaaagacatcttttatgatggccctgtgcctgtctagcatctacgaggacctgaagatgtatcaggtggagttcaagaccatgaacgccaagctgctgatggacccaaagcggcagatctttctggatcagaatatgctggccgtgatcgacgagctgatgcaggccctgaacttcaatagcgagacagtgccccagaagtcctctctggaggagcctgacttctacaagaccaagatcaagctgtgcatcctgctgcacgccttccggatcagagccgtgaccatcgatagagtgatgagctatctgaacgcaagcggcggcggaggctctggaggaggcggcagcgacaagacccacacatgcccaccatgtccagcacctgagctgctgggaggaccatccgtgttcctgtttcctccaaagcccaaggatacactgatgatcagccgcacacctgaggtgacctgcgtggtggtggacgtgtcccacgaggaccccgaggtgaagtttaactggtacgtggacggcgtggaggtgcacaatgccaagaccaagcccagggaggagcagtacaactctacatatcgcgtggtgagcgtgctgaccgtgctgcaccaggactggctgaacggcaaggagtacaagtgcaaggtgtctaataaggccctgccagcccccatcgagaagaccatcagcaaggcaaagggacagccaagggagcctcaggtgtatacactgccccctagccgcgatgagctgaccaagaaccaggtgtccctgtcttgtgccgtgaagggcttctacccatccgacatcgccgtggagtgggagtctaatggccagcccgagaacaattataagaccacaccacccgtgctggactccgatggctctttctttctggtgagcaagctgacagtggacaagtccagatggcagcagggcaacgtgtttagctgctccgtgatgcacgaggccctgcacaatcactacacccagaagtctctgagcctgtcccctggcaagtga

SEQ ID NO: 48 - DNA, 1761 bp, Artificial Sequence
  (anti-hu CD20 VH)2-hu IgG1 Fc knob
caagtgcagctgcagcagcctggcgccgagctggtgaaaccaggagcttctgtgaagatgagctgtaaagccagcggctacaccttcacctcttataatatgcactgggtcaagcagacccctggaagaggcctggaatggatcggcgctatctaccccggcaacggcgacaccagctacaaccagaagttcaagggcaaggccacactgaccgccgacaagtccagctctacagcctacatgcagctgagcagcctgacaagcgaggacagcgccgtgtactactgcgcccggagcacctactacggcggagattggtactttaacgtgtggggcgccggcaccacagtgaccgtgtccgccggtggaggtggctcaggaggaggcggttctggcggaggaggtagtcaggtgcagctgcagcagccaggagcagagctggtgaagcctggagcctctgtgaagatgagctgcaaggcctccggctacaccttcacaagctataacatgcactgggtgaagcagaccccaggaaggggactggagtggatcggagccatctaccctggcaacggcgacacatcctataatcagaagtttaagggcaaggccaccctgacagccgataagagctcctctaccgcctacatgcagctgagctccctgacaagcgaggactccgccgtgtactattgcgccagaagcacctactatggcggcgattggtacttcaacgtgtggggagcaggaaccacagtgaccgtgtctgccgccagcacaaagggaccatccgtgtttccactggcaccatctagcaagtctaccagcggaggaacagccgccctgggatgtctggtgaaggactacttcccagagcccgtgaccgtgtcctggaactctggcgccctgacctccggagtgcacacatttcccgccgtgctgcagtcctctggcctgtactctctgagctccgtggtgaccgtgccttctagctccctgggcacccagacatatatctgcaacgtgaatcacaagccttccaatacaaaggtggacaagaaggtggagccaaagtcttgtgataagacccacacatgccccccttgtcctgcaccagagctgctgggaggaccaagcgtgttcctgtttccacccaagcccaaggacaccctgatgatcagcaggacccctgaggtgacatgcgtggtggtggacgtgtcccacgaggacccagaggtgaagttcaactggtacgtggatggcgtggaggtgcacaatgccaagacaaagccacgggaggagcagtacaactctacctatagagtggtgagcgtgctgacagtgctgcaccaggattggctgaacggcaaggagtataagtgcaaggtgtctaataaggccctgcccgcccctatcgagaagaccatcagcaaggccaagggccagcctagggagccacaggtgtacaccctgcctccatctcgcgacgagctgacaaagaaccaggtgagcctgtggtgtctggtgaagggcttctatccaagcgatatcgccgtggagtgggagtccaatggccagcccgagaacaattacaagaccacaccccctgtgctggacagcgatggctccttctttctgtattccaagctgaccgtggataagtctagatggcagcagggcaacgtgttttcctgttctgtgatgcacgaggccctgcacaatcactacacacagaagagcctgtccctgtctcctggcaag

SEQ ID NO: 49 - DNA, 1002 bp, Artificial Sequence
  (anti-hu CD20 VL)2
caaatcgtgctgagccagagccctgctatcctgtccgcctctccaggcgagaaggtgaccatgacctgtagagccagcagcagcgtgtcctacatccactggtttcagcagaaacctggctctagccctaagccttggatctacgccacaagcaacctggcctccggcgtccctgtgcggttcagcggcagcggcagcggcacctcttatagcctgaccatcagcagagtggaagccgaggacgccgctacatactactgccagcagtggacatctaacccccccaccttcggcggaggaaccaagctggaaattaagggtggaggtggctcaggaggaggcggttctggcggaggaggtagtcagatcgtgctgagccagtccccagcaatcctgtctgccagccctggagagaaggtgaccatgacatgccgggccagctcctctgtgagctacatccactggttccagcagaagccaggcagctcccctaagccatggatctatgccacaagcaacctggcatccggagtgcccgtgcggttttccggctctggcagcggcacctcctactctctgacaatcagcagagtggaggcagaggacgcagcaacctactattgccagcagtggacctccaatccccctacattcggcggcggcaccaagctggagatcaagaggacagtggccgccccttccgtgttcatctttccaccctctgacgagcagctgaagtctggcaccgccagcgtggtgtgcctgctgaacaacttctacccacgcgaggccaaggtgcagtggaaggtggataacgccctgcagagcggcaattcccaggagtctgtgacagagcaggacagcaaggattccacctattctctgtctagcaccctgacactgagcaaggccgattacgagaagcacaaggtgtatgcctgcgaggtgacacaccagggcctgtcctctcccgtgaccaagtccttcaacaggggcgagtgt

SEQ ID NO: 50 - DNA, 2139 bp, Artificial Sequence
  anti-hu CD20 HC hu IgG1 Fc knob-anti-hu CD20 scFv
caggtgcagctgcagcagccaggagcagagctggtgaagcctggagcctctgtgaagatgagctgcaaggcctccggctacaccttcacaagctataacatgcactgggtgaagcagaccccaggaaggggactggagtggatcggagccatctaccctggcaacggcgacacatcctataatcagaagtttaagggcaaggccaccctgacagccgataagagctcctctaccgcctacatgcagctgagctccctgacaagcgaggactccgccgtgtactattgcgccagaagcacctactatggcggcgattggtacttcaacgtgtggggagcaggaaccacagtgaccgtgtctgccgccagcacaaagggaccatccgtgtttccactggcaccatctagcaagtctaccagcggaggaacagccgccctgggatgtctggtgaaggactacttcccagagcccgtgaccgtgtcctggaactctggcgccctgacctccggagtgcacacatttcccgccgtgctgcagtcctctggcctgtactctctgagctccgtggtgaccgtgccttctagctccctgggcacccagacatatatctgcaacgtgaatcacaagccttccaatacaaaggtggacaagaaggtggagccaaagtcttgtgataagacccacacatgccccccttgtcctgcaccagagctgctgggaggaccaagcgtgttcctgtttccacccaagcccaaggacaccctgatgatcagcaggacccctgaggtgacatgcgtggtggtggacgtgtcccacgaggacccagaggtgaagttcaactggtacgtggatggcgtggaggtgcacaatgccaagacaaagccacgggaggagcagtacaactctacctatagagtggtgagcgtgctgacagtgctgcaccaggattggctgaacggcaaggagtataagtgcaaggtgtctaataaggccctgcccgcccctatcgagaagaccatcagcaaggccaagggccagcctagggagccacaggtgtacaccctgcctccatctcgcgacgagctgacaaagaaccaggtgagcctgtggtgtctggtgaagggcttctatccaagcgatatcgccgtggagtgggagtccaatggccagcccgagaacaattacaagaccacaccccctgtgctggacagcgatggctccttctttctgtattccaagctgaccgtggataagtctagatggcagcagggcaacgtgttttcctgttctgtgatgcacgaggccctgcacaatcactacacacagaagagcctgtccctgtctcctggcaagggtggaggtggctcaggaggaggcggttctggcggaggaggtagtcaagtgcagctgcagcagcctggcgccgagctggtgaaaccaggagcttctgtgaagatgagctgtaaagccagcggctacaccttcacctcttataatatgcactgggtcaagcagacccctggaagaggcctggaatggatcggcgctatctaccccggcaacggcgacaccagctacaaccagaagttcaagggcaaggccacactgaccgccgacaagtccagctctacagcctacatgcagctgagcagcctgacaagcgaggacagcgccgtgtactactgcgcccggagcacctactacggcggagattggtactttaacgtgtggggcgccggcaccacagtgaccgtgtccgccggcggaggaggtagcggtggtggaggatctggcggtggcggaagcggtggaggcggttcacaaatcgtgctgagccagagccctgctatcctgtccgcctctccaggcgagaaggtgaccatgacctgtagagccagcagcagcgtgtcctacatccactggtttcagcagaaacctggctctagccctaagccttggatctacgccacaagcaacctggcctccggcgtccctgtgcggttcagcggcagcggcagcggcacctcttatagcctgaccatcagcagagtggaagccgaggacgccgctacatactactgccagcagtggacatctaacccccccaccttcggcggaggaaccaagctggaaattaag

SEQ ID NO: 51 - DNA, 1425 bp, Artificial Sequence
  anti-hu CD20 LC-anti-hu CD20 scFv
cagatcgtgctgagccagtccccagcaatcctgtctgccagccctggagagaaggtgaccatgacatgccgggccagctcctctgtgagctacatccactggttccagcagaagccaggcagctcccctaagccatggatctatgccacaagcaacctggcatccggagtgcccgtgcggttttccggctctggcagcggcacctcctactctctgacaatcagcagagtggaggcagaggacgcagcaacctactattgccagcagtggacctccaatccccctacattcggcggcggcaccaagctggagatcaagaggacagtggccgccccttccgtgttcatctttccaccctctgacgagcagctgaagtctggcaccgccagcgtggtgtgcctgctgaacaacttctacccacgcgaggccaaggtgcagtggaaggtggataacgccctgcagagcggcaattcccaggagtctgtgacagagcaggacagcaaggattccacctattctctgtctagcaccctgacactgagcaaggccgattacgagaagcacaaggtgtatgcctgcgaggtgacacaccagggcctgtcctctcccgtgaccaagtccttcaacaggggcgagtgtggtggaggtggctcaggaggaggcggttctggcggaggaggtagtcaagtgcagctgcagcagcctggcgccgagctggtgaaaccaggagcttctgtgaagatgagctgtaaagccagcggctacaccttcacctcttataatatgcactgggtcaagcagacccctggaagaggcctggaatggatcggcgctatctaccccggcaacggcgacaccagctacaaccagaagttcaagggcaaggccacactgaccgccgacaagtccagctctacagcctacatgcagctgagcagcctgacaagcgaggacagcgccgtgtactactgcgcccggagcacctactacggcggagattggtactttaacgtgtggggcgccggcaccacagtgaccgtgtccgccggcggaggaggtagcggtggtggaggatctggcggtggcggaagcggtggaggcggttcacaaatcgtgctgagccagagccctgctatcctgtccgcctctccaggcgagaaggtgaccatgacctgtagagccagcagcagcgtgtcctacatccactggtttcagcagaaacctggctctagccctaagccttggatctacgccacaagcaacctggcctccggcgtccctgtgcggttcagcggcagcggcagcggcacctcttatagcctgaccatcagcagagtggaagccgaggacgccgctacatactactgccagcagtggacatctaacccccccaccttcggcggaggaaccaagctggaaattaag

SEQ ID NO: 52 - DNA, 2952 bp, Artificial Sequence
  anti-hu CD20 HC hu IgG1 Fc hole-hu scIL-12
caggtgcagctgcagcagccaggagcagagctggtgaagcctggagcctctgtgaagatgagctgcaaggcctccggctacaccttcacaagctataacatgcactgggtgaagcagaccccaggaaggggactggagtggatcggagccatctaccctggcaacggcgacacatcctataatcagaagtttaagggcaaggccaccctgacagccgataagagctcctctaccgcctacatgcagctgagctccctgacaagcgaggactccgccgtgtactattgcgccagaagcacctactatggcggcgattggtacttcaacgtgtggggagcaggaaccacagtgaccgtgtctgccgccagcacaaagggaccatccgtgtttccactggcaccatctagcaagtctaccagcggaggaacagccgccctgggatgtctggtgaaggactacttcccagagcccgtgaccgtgtcctggaactctggcgccctgacctccggagtgcacacatttcccgccgtgctgcagtcctctggcctgtactctctgagctccgtggtgaccgtgccttctagctccctgggcacccagacatatatctgcaacgtgaatcacaagccttccaatacaaaggtggacaagaaggtggagccaaagtcttgtgacaagacccacacatgcccaccatgtccagcacctgagctgctgggaggaccatccgtgttcctgtttcctccaaagcccaaggatacactgatgatcagccgcacacctgaggtgacctgcgtggtggtggacgtgtcccacgaggaccccgaggtgaagtttaactggtacgtggacggcgtggaggtgcacaatgccaagaccaagcccagggaggagcagtacaactctacatatcgcgtggtgagcgtgctgaccgtgctgcaccaggactggctgaacggcaaggagtacaagtgcaaggtgtctaataaggccctgccagcccccatcgagaagaccatcagcaaggcaaagggacagccaagggagcctcaggtgtatacactgccccctagccgcgatgagctgaccaagaaccaggtgtccctgtcttgtgccgtgaagggcttctacccatccgacatcgccgtggagtgggagtctaatggccagcccgagaacaattataagaccacaccacccgtgctggactccgatggctctttctttctggtgagcaagctgacagtggacaagtccagatggcagcagggcaacgtgtttagctgctccgtgatgcacgaggccctgcacaatcactacacccagaagtctctgagcctgtcccctggcaagggtggaggtggctcaggaggaggcggttctggcggaggaggtagtatctgggagctgaagaaggacgtgtacgtggtggagctggactggtatcctgatgccccaggcgagatggtggtgctgacctgcgacacacccgaggaggatggcatcacctggacactggatcagagctccgaggtgctgggcagcggcaagaccctgacaatccaggtgaaggagttcggcgacgccggccagtacacctgtcacaagggaggagaggtgctgagccactccctgctgctgctgcacaagaaggaggacggcatctggagcacagacatcctgaaggatcagaaggagccaaagaacaagaccttcctgcggtgcgaggccaagaattattccggccggttcacctgttggtggctgaccacaatctccaccgatctgacattttctgtgaagtctagcaggggctcctctgacccccagggagtgacatgcggagcagccaccctgagcgccgagcgggtgagaggcgataacaaggagtacgagtattccgtggagtgccaggaggactctgcctgtcctgcagcagaggagtccctgccaatcgaagtgatggtggatgccgtgcacaagctgaagtacgagaattatacaagctccttctttatcagggacatcatcaagcctgatccccctaagaacctgcagctgaagccactgaagaatagccgccaggtggaggtgtcctgggagtacccagacacctggtccacaccccactcttatttcagcctgaccttttgcgtgcaggtgcagggcaagtccaagagggagaagaaggaccgcgtgttcaccgataagacatctgccaccgtgatctgtcggaagaacgcctctatcagcgtgcgggcccaggatagatactattctagctcctggagcgagtgggcctccgtgccttgttctggaggaggaggcagcggcggaggaggctccggaggaggaggctctagaaatctgccagtggcaacccctgacccaggaatgttcccttgcctgcaccactctcagaacctgctgcgggccgtgagcaatatgctgcagaaggccagacagacactggagttttacccctgtaccagcgaggagatcgaccacgaggatatcacaaaggataagacctccacagtggaggcctgcctgcctctggagctgaccaagaacgagagctgtctgaacagccgggagacatctttcatcaccaacggcagctgcctggcctccagaaagacatcttttatgatggccctgtgcctgtctagcatctacgaggacctgaagatgtatcaggtggagttcaagaccatgaacgccaagctgctgatggacccaaagcggcagatctttctggatcagaatatgctggccgtgatcgacgagctgatgcaggccctgaacttcaatagcgagacagtgccccagaagtcctctctggaggagcctgacttctacaagaccaagatcaagctgtgcatcctgctgcacgccttccggatcagagccgtgaccatcgatagagtgatgagctatctgaacgcaagc

SEQ ID NO: 53 - DNA, 2952 bp, Artificial Sequence
  anti-hu CD20 HC hu IgG1 Fc hole-hu scIL-12 mut2
caggtgcagctgcagcagccaggagcagagctggtgaagcctggagcctctgtgaagatgagctgcaaggcctccggctacaccttcacaagctataacatgcactgggtgaagcagaccccaggaaggggactggagtggatcggagccatctaccctggcaacggcgacacatcctataatcagaagtttaagggcaaggccaccctgacagccgataagagctcctctaccgcctacatgcagctgagctccctgacaagcgaggactccgccgtgtactattgcgccagaagcacctactatggcggcgattggtacttcaacgtgtggggagcaggaaccacagtgaccgtgtctgccgccagcacaaagggaccatccgtgtttccactggcaccatctagcaagtctaccagcggaggaacagccgccctgggatgtctggtgaaggactacttcccagagcccgtgaccgtgtcctggaactctggcgccctgacctccggagtgcacacatttcccgccgtgctgcagtcctctggcctgtactctctgagctccgtggtgaccgtgccttctagctccctgggcacccagacatatatctgcaacgtgaatcacaagccttccaatacaaaggtggacaagaaggtggagccaaagtcttgtgacaagacccacacatgcccaccatgtccagcacctgagctgctgggaggaccatccgtgttcctgtttcctccaaagcccaaggatacactgatgatcagccgcacacctgaggtgacctgcgtggtggtggacgtgtcccacgaggaccccgaggtgaagtttaactggtacgtggacggcgtggaggtgcacaatgccaagaccaagcccagggaggagcagtacaactctacatatcgcgtggtgagcgtgctgaccgtgctgcaccaggactggctgaacggcaaggagtacaagtgcaaggtgtctaataaggccctgccagcccccatcgagaagaccatcagcaaggcaaagggacagccaagggagcctcaggtgtatacactgccccctagccgcgatgagctgaccaagaaccaggtgtccctgtcttgtgccgtgaagggcttctacccatccgacatcgccgtggagtgggagtctaatggccagcccgagaacaattataagaccacaccacccgtgctggactccgatggctctttctttctggtgagcaagctgacagtggacaagtccagatggcagcagggcaacgtgtttagctgctccgtgatgcacgaggccctgcacaatcactacacccagaagtctctgagcctgtcccctggcaagggtggaggtggctcaggaggaggcggttctggcggaggaggtagtatctgggagctgaagaaggacgtgtacgtggtggagctggactggtatcctgatgccccaggcgagatggtggtgctgacctgcgacacacccgaggaggatggcatcacctggacactggatcagagctccgaggtgctgggcagcggcaagaccctgacaatccaggtgaaggagttcggcgacgccggccagtacacctgtcacaagggaggagaggtgctgagccactccctgctgctgctgcacaagaaggaggacggcatctggagcacagacatcctgaaggatcagaaggagccaaagaacaagaccttcctgcggtgcgaggccaagaattattccggccggttcacctgttggtggctgaccacaatctccaccgatctgacattttctgtgaagtctagcaggggctcctctgacccccagggagtgacatgcggagcagccaccctgagcgccgagcgggtgagaggcgataacaaggagtacgagtattccgtggagtgccaggaggactctgcctgtcctgcagcagaggagtccctgccaatcgaagtgatggtggatgccgtgcacaagctgaagtacgagaattatacaagctccttctttatcagggacatcatcaagcctgatccccctaagaacctgcagctgaagccactgaagaatagccgccaggtggaggtgtcctgggagtacccagacacctggtccacaccccactcttatttcagcctgaccttttgcgtgcaggtgcagggcgcctccgctagggaggccgctgaccgcgtgttcaccgataagacatctgccaccgtgatctgtcggaagaacgcctctatcagcgtgcgggcccaggatagatactattctagctcctggagcgagtgggcctccgtgccttgttctggaggaggaggcagcggcggaggaggctccggaggaggaggctctagaaatctgccagtggcaacccctgacccaggaatgttcccttgcctgcaccactctcagaacctgctgcgggccgtgagcaatatgctgcagaaggccagacagacactggagttttacccctgtaccagcgaggagatcgaccacgaggatatcacaaaggataagacctccacagtggaggcctgcctgcctctggagctgaccaagaacgagagctgtctgaacagccgggagacatctttcatcaccaacggcagctgcctggcctccagaaagacatcttttatgatggccctgtgcctgtctagcatctacgaggacctgaagatgtatcaggtggagttcaagaccatgaacgccaagctgctgatggacccaaagcggcagatctttctggatcagaatatgctggccgtgatcgacgagctgatgcaggccctgaacttcaatagcgagacagtgccccagaagtcctctctggaggagcctgacttctacaagaccaagatcaagctgtgcatcctgctgcacgccttccggatcagagccgtgaccatcgatagagtgatgagctatctgaacgcaagc

SEQ ID NO: 54 - DNA, 1353 bp, Artificial Sequence
  anti-hu CD20 HC hu IgG1 Fc knob DANG
caggtgcagctgcagcagccaggagcagagctggtgaagcctggagcctctgtgaagatgagctgcaaggcctccggctacaccttcacaagctataacatgcactgggtgaagcagaccccaggaaggggactggagtggatcggagccatctaccctggcaacggcgacacatcctataatcagaagtttaagggcaaggccaccctgacagccgataagagctcctctaccgcctacatgcagctgagctccctgacaagcgaggactccgccgtgtactattgcgccagaagcacctactatggcggcgattggtacttcaacgtgtggggagcaggaaccacagtgaccgtgtctgccgccagcacaaagggaccatccgtgtttccactggcaccatctagcaagtctaccagcggaggaacagccgccctgggatgtctggtgaaggactacttcccagagcccgtgaccgtgtcctggaactctggcgccctgacctccggagtgcacacatttcccgccgtgctgcagtcctctggcctgtactctctgagctccgtggtgaccgtgccttctagctccctgggcacccagacatatatctgcaacgtgaatcacaagccttccaatacaaaggtggacaagaaggtggagccaaagtcttgtgataagacccacacatgccccccttgtcctgcaccagagctgctgggaggaccaagcgtgttcctgtttccacccaagcccaaggacaccctgatgatcagcaggacccctgaggtgacatgcgtggtggtggccgtgtcccacgaggacccagaggtgaagttcaactggtacgtggatggcgtggaggtgcacaatgccaagacaaagccacgggaggagcagtacggctctacctatagagtggtgagcgtgctgacagtgctgcaccaggattggctgaacggcaaggagtataagtgcaaggtgtctaataaggccctgcccgcccctatcgagaagaccatcagcaaggccaagggccagcctagggagccacaggtgtacaccctgcctccatctcgcgacgagctgacaaagaaccaggtgagcctgtggtgtctggtgaagggcttctatccaagcgatatcgccgtggagtgggagtccaatggccagcccgagaacaattacaagaccacaccccctgtgctggacagcgatggctccttctttctgtattccaagctgaccgtggataagtctagatggcagcagggcaacgtgttttcctgttctgtgatgcacgaggccctgcacaatcactacacacagaagagcctgtccctgtctcctggcaag

SEQ ID NO: 55 - DNA, 2265 bp, Artificial Sequence
  hu scIL-12-hu IgG1 Fc hole DANG
atctgggagctgaagaaggacgtgtacgtggtggagctggactggtatcctgatgccccaggcgagatggtggtgctgacctgcgacacacccgaggaggatggcatcacctggacactggatcagagctccgaggtgctgggcagcggcaagaccctgacaatccaggtgaaggagttcggcgacgccggccagtacacctgtcacaagggaggagaggtgctgagccactccctgctgctgctgcacaagaaggaggacggcatctggagcacagacatcctgaaggatcagaaggagccaaagaacaagaccttcctgcggtgcgaggccaagaattattccggccggttcacctgttggtggctgaccacaatctccaccgatctgacattttctgtgaagtctagcaggggctcctctgacccccagggagtgacatgcggagcagccaccctgagcgccgagcgggtgagaggcgataacaaggagtacgagtattccgtggagtgccaggaggactctgcctgtcctgcagcagaggagtccctgccaatcgaagtgatggtggatgccgtgcacaagctgaagtacgagaattatacaagctccttctttatcagggacatcatcaagcctgatccccctaagaacctgcagctgaagccactgaagaatagccgccaggtggaggtgtcctgggagtacccagacacctggtccacaccccactcttatttcagcctgaccttttgcgtgcaggtgcagggcaagtccaagagggagaagaaggaccgcgtgttcaccgataagacatctgccaccgtgatctgtcggaagaacgcctctatcagcgtgcgggcccaggatagatactattctagctcctggagcgagtgggcctccgtgccttgttctggaggaggaggcagcggcggaggaggctccggaggaggaggctctagaaatctgccagtggcaacccctgacccaggaatgttcccttgcctgcaccactctcagaacctgctgcgggccgtgagcaatatgctgcagaaggccagacagacactggagttttacccctgtaccagcgaggagatcgaccacgaggatatcacaaaggataagacctccacagtggaggcctgcctgcctctggagctgaccaagaacgagagctgtctgaacagccgggagacatctttcatcaccaacggcagctgcctggcctccagaaagacatcttttatgatggccctgtgcctgtctagcatctacgaggacctgaagatgtatcaggtggagttcaagaccatgaacgccaagctgctgatggacccaaagcggcagatctttctggatcagaatatgctggccgtgatcgacgagctgatgcaggccctgaacttcaatagcgagacagtgccccagaagtcctctctggaggagcctgacttctacaagaccaagatcaagctgtgcatcctgctgcacgccttccggatcagagccgtgaccatcgatagagtgatgagctatctgaacgcaagcggcggcggaggctctggaggaggcggcagcgacaagacccacacatgcccaccatgtccagcacctgagctgctgggaggaccatccgtgttcctgtttcctccaaagcccaaggatacactgatgatcagccgcacacctgaggtgacctgcgtggtggtggccgtgtcccacgaggaccccgaggtgaagtttaactggtacgtggacggcgtggaggtgcacaatgccaagaccaagcccagggaggagcagtacggctctacatatcgcgtggtgagcgtgctgaccgtgctgcaccaggactggctgaacggcaaggagtacaagtgcaaggtgtctaataaggccctgccagcccccatcgagaagaccatcagcaaggcaaagggacagccaagggagcctcaggtgtatacactgccccctagccgcgatgagctgaccaagaaccaggtgtccctgtcttgtgccgtgaagggcttctacccatccgacatcgccgtggagtgggagtctaatggccagcccgagaacaattataagaccacaccacccgtgctggactccgatggctctttctttctggtgagcaagctgacagtggacaagtccagatggcagcagggcaacgtgtttagctgctccgtgatgcacgaggccctgcacaatcactacacccagaagtctctgagcctgtcccctggcaag

SEQ ID NO: 56 - DNA, 2265 bp, Artificial Sequence
  hu scIL-12 mut1-hu IgG1 Fc hole DANG
atctgggagctgaagaaggacgtgtacgtggtggagctggactggtatcctgatgccccaggcgagatggtggtgctgacctgcgacacacccgaggaggatggcatcacctggacactggatcagagctccgaggtgctgggcagcggcaagaccctgacaatccaggtgaaggagttcggcgacgccggccagtacacctgtcacaagggaggagaggtgctgagccactccctgctgctgctgcacaagaaggaggacggcatctggagcacagacatcctgaaggatcagaaggagccaaagaacaagaccttcctgcggtgcgaggccaagaattattccggccggttcacctgttggtggctgaccacaatctccaccgatctgacattttctgtgaagtctagcaggggctcctctgacccccagggagtgacatgcggagcagccaccctgagcgccgagcgggtgagaggcgataacaaggagtacgagtattccgtggagtgccaggaggactctgcctgtcctgcagcagaggagtccctgccaatcgaagtgatggtggatgccgtgcacaagctgaagtacgagaattatacaagctccttctttatcagggacatcatcaagcctgatccccctaagaacctgcagctgaagccactgaagaatagccgccaggtggaggtgtcctgggagtacccagacacctggtccacaccccactcttatttcagcctgaccttttgcgtgcaggtgcagggagcatccaagagggaggcaaaggaccgcgtgttcaccgataagacatctgccaccgtgatctgtcggaagaacgcctctatcagcgtgcgggcccaggatagatactattctagctcctggagcgagtgggcctccgtgccttgttctggaggaggaggcagcggcggaggaggctccggaggaggaggctctagaaatctgccagtggcaacccctgacccaggaatgttcccttgcctgcaccactctcagaacctgctgcgggccgtgagcaatatgctgcagaaggccagacagacactggagttttacccctgtaccagcgaggagatcgaccacgaggatatcacaaaggataagacctccacagtggaggcctgcctgcctctggagctgaccaagaacgagagctgtctgaacagccgggagacatctttcatcaccaacggcagctgcctggcctccagaaagacatcttttatgatggccctgtgcctgtctagcatctacgaggacctgaagatgtatcaggtggagttcaagaccatgaacgccaagctgctgatggacccaaagcggcagatctttctggatcagaatatgctggccgtgatcgacgagctgatgcaggccctgaacttcaatagcgagacagtgccccagaagtcctctctggaggagcctgacttctacaagaccaagatcaagctgtgcatcctgctgcacgccttccggatcagagccgtgaccatcgatagagtgatgagctatctgaacgcaagcggcggcggaggctctggaggaggcggcagcgacaagacccacacatgcccaccatgtccagcacctgagctgctgggaggaccatccgtgttcctgtttcctccaaagcccaaggatacactgatgatcagccgcacacctgaggtgacctgcgtggtggtggccgtgtcccacgaggaccccgaggtgaagtttaactggtacgtggacggcgtggaggtgcacaatgccaagaccaagcccagggaggagcagtacggctctacatatcgcgtggtgagcgtgctgaccgtgctgcaccaggactggctgaacggcaaggagtacaagtgcaaggtgtctaataaggccctgccagcccccatcgagaagaccatcagcaaggcaaagggacagccaagggagcctcaggtgtatacactgccccctagccgcgatgagctgaccaagaaccaggtgtccctgtcttgtgccgtgaagggcttctacccatccgacatcgccgtggagtgggagtctaatggccagcccgagaacaattataagaccacaccacccgtgctggactccgatggctctttctttctggtgagcaagctgacagtggacaagtccagatggcagcagggcaacgtgtttagctgctccgtgatgcacgaggccctgcacaatcactacacccagaagtctctgagcctgtcccctggcaag

SEQ ID NO: 57 - DNA, 2265 bp, Artificial Sequence
  hu scIL-12 mut2-hu IgG1 Fc
atctgggagctgaagaaggacgtgtacgtggtggagctggactggtatcctgatgccccaggcgagatggtggtgctgacctgcgacacacccgaggaggatggcatcacctggacactggatcagagctccgaggtgctgggcagcggcaagaccctgacaatccaggtgaaggagttcggcgacgccggccagtacacctgtcacaagggaggagaggtgctgagccactccctgctgctgctgcacaagaaggaggacggcatctggagcacagacatcctgaaggatcagaaggagccaaagaacaagaccttcctgcggtgcgaggccaagaattattccggccggttcacctgttggtggctgaccacaatctccaccgatctgacattttctgtgaagtctagcaggggctcctctgacccccagggagtgacatgcggagcagccaccctgagcgccgagcgggtgagaggcgataacaaggagtacgagtattccgtggagtgccaggaggactctgcctgtcctgcagcagaggagtccctgccaatcgaagtgatggtggatgccgtgcacaagctgaagtacgagaattatacaagctccttctttatcagggacatcatcaagcctgatccccctaagaacctgcagctgaagccactgaagaatagccgccaggtggaggtgtcctgggagtacccagacacctggtccacaccccactcttatttcagcctgaccttttgcgtgcaggtgcagggcgcctccgctagggaggccgctgaccgcgtgttcaccgataagacatctgccaccgtgatctgtcggaagaacgcctctatcagcgtgcgggcccaggatagatactattctagctcctggagcgagtgggcctccgtgccttgttctggaggaggaggcagcggcggaggaggctccggaggaggaggctctagaaatctgccagtggcaacccctgacccaggaatgttcccttgcctgcaccactctcagaacctgctgcgggccgtgagcaatatgctgcagaaggccagacagacactggagttttacccctgtaccagcgaggagatcgaccacgaggatatcacaaaggataagacctccacagtggaggcctgcctgcctctggagctgaccaagaacgagagctgtctgaacagccgggagacatctttcatcaccaacggcagctgcctggcctccagaaagacatcttttatgatggccctgtgcctgtctagcatctacgaggacctgaagatgtatcaggtggagttcaagaccatgaacgccaagctgctgatggacccaaagcggcagatctttctggatcagaatatgctggccgtgatcgacgagctgatgcaggccctgaacttcaatagcgagacagtgccccagaagtcctctctggaggagcctgacttctacaagaccaagatcaagctgtgcatcctgctgcacgccttccggatcagagccgtgaccatcgatagagtgatgagctatctgaacgcaagcggcggcggaggctctggaggaggcggcagcgacaagacccacacatgcccaccatgtccagcacctgagctgctgggaggaccatccgtgttcctgtttcctccaaagcccaaggatacactgatgatcagccgcacacctgaggtgacctgcgtggtggtggacgtgtcccacgaggaccccgaggtgaagtttaactggtacgtggacggcgtggaggtgcacaatgccaagaccaagcccagggaggagcagtacaactctacatatcgcgtggtgagcgtgctgaccgtgctgcaccaggactggctgaacggcaaggagtacaagtgcaaggtgtctaataaggccctgccagcccccatcgagaagaccatcagcaaggcaaagggacagccaagggagcctcaggtgtatacactgccccctagccgcgatgagctgaccaagaaccaggtgtccctgacttgtctcgtgaagggcttctacccatccgacatcgccgtggagtgggagtctaatggccagcccgagaacaattataagaccacaccacccgtgctggactccgatggctctttctttctgtacagcaagctgacagtggacaagtccagatggcagcagggcaacgtgtttagctgctccgtgatgcacgaggccctgcacaatcactacacccagaagtctctgagcctgtcccctggcaag

SEQ ID NO: 58 - DNA, 1362 bp, Artificial Sequence
  anti-hu FAP HC hu IgG1 Fc knob
caggtgcagctggtgcagtccggagcagaggtgaagaagccaggagcctctgtgaaggtgagctgcaagacctccagatacaccttcacagagtatacaatccactgggtgcgccaggcacctggacagcggctggagtggatcggaggcatcaaccccaacaatggcatccctaactacaatcagaagtttaagggcagagtgaccatcacagtggacacctccgcctctacagcctatatggagctgagctccctgaggagcgaggataccgccgtgtactattgcgcccggagaaggatcgcctacggctatgacgagggccacgccatggattactggggccagggcaccctggtgacagtgtctagcgcctctaccaagggaccaagcgtgttcccactggcaccatcctctaagagcacctccggaggaacagccgccctgggctgtctggtgaaggactatttcccagagcccgtgacagtgtcctggaactctggcgccctgacctccggagtgcacacatttcctgccgtgctgcagagctccggcctgtacagcctgtctagcgtggtgaccgtgccatcctctagcctgggcacccagacatatatctgcaacgtgaatcacaagcctagcaatacaaaggtggacaagaaggtggagccaaagtcctgtgataagacccacacatgccccccttgtcctgcaccagagctgctgggaggaccaagcgtgttcctgtttccacccaagcccaaggacaccctgatgatctctcgcaccccagaggtgacatgcgtggtggtggacgtgagccacgaggaccccgaggtgaagtttaactggtacgtggatggcgtggaggtgcacaatgccaagaccaagccaagagaggagcagtacaactccacctatagggtggtgtctgtgctgacagtgctgcaccaggattggctgaacggcaaggagtataagtgcaaggtgtccaataaggccctgcccgcccctatcgagaagaccatctctaaggcaaagggacagcctagggagccacaggtgtacaccctgcctccatcccgggacgagctgacaaagaaccaggtgtctctgtggtgtctggtgaagggcttctatccctctgatatcgccgtggagtgggagagcaatggccagcctgagaacaattacaagaccacaccccctgtgctggacagcgatggctccttctttctgtatagcaagctgaccgtggataagtcccggtggcagcagggcaacgtgttttcttgtagcgtgatgcacgaggccctgcacaatcactacacacagaagtccctgtctctgagccctggcaag

SEQ ID NO: 59 - DNA, 660 bp, Artificial Sequence
  anti-hu FAP LC
gacatcgtgatgacccagtcccctgattctctggccgtgagcctgggagagagggcaacaatcaactgcaagagctcccagagcctgctgtactcccgcaaccagaagaattacctggcctggtatcagcagaagcccggccagccccctaagctgctgatcttctgggcatctaccagggagagcggagtgcctgacagattttctggcagcggcttcggcacagacttcaccctgacaatctctagcctgcaggccgaggacgtggccgtgtactattgccagcagtacttctcctatcctctgacctttggccagggcacaaaggtggagatcaagaggaccgtggcagcaccaagcgtgttcatctttccaccctccgacgagcagctgaagtccggcaccgcctctgtggtgtgcctgctgaacaatttctacccaagggaggccaaggtgcagtggaaggtggataacgccctgcagagcggcaattcccaggagtctgtgaccgagcaggacagcaaggattccacatattctctgtcctctaccctgacactgtctaaggccgattacgagaagcacaaggtgtatgcatgcgaggtgacccaccagggactgagctccccagtgacaaagtcctttaatcggggcgagtgt

SEQ ID NO: 60 - DNA, 1362 bp, Artificial Sequence
  anti-hu FAP HC hu IgG1 Fc knob DANG
caggtgcagctggtgcagtccggagcagaggtgaagaagccaggagcctctgtgaaggtgagctgcaagacctccagatacaccttcacagagtatacaatccactgggtgcgccaggcacctggacagcggctggagtggatcggaggcatcaaccccaacaatggcatccctaactacaatcagaagtttaagggcagagtgaccatcacagtggacacctccgcctctacagcctatatggagctgagctccctgaggagcgaggataccgccgtgtactattgcgcccggagaaggatcgcctacggctatgacgagggccacgccatggattactggggccagggcaccctggtgacagtgtctagcgcctctaccaagggaccaagcgtgttcccactggcaccatcctctaagagcacctccggaggaacagccgccctgggctgtctggtgaaggactatttcccagagcccgtgacagtgtcctggaactctggcgccctgacctccggagtgcacacatttcctgccgtgctgcagagctccggcctgtacagcctgtctagcgtggtgaccgtgccatcctctagcctgggcacccagacatatatctgcaacgtgaatcacaagcctagcaatacaaaggtggacaagaaggtggagccaaagtcctgtgataagacccacacatgccccccttgtcctgcaccagagctgctgggaggaccaagcgtgttcctgtttccacccaagcccaaggacaccctgatgatctctcgcaccccagaggtgacatgcgtggtggtggccgtgagccacgaggaccccgaggtgaagtttaactggtacgtggatggcgtggaggtgcacaatgccaagaccaagccaagagaggagcagtacggctccacctatagggtggtgtctgtgctgacagtgctgcaccaggattggctgaacggcaaggagtataagtgcaaggtgtccaataaggccctgcccgcccctatcgagaagaccatctctaaggcaaagggacagcctagggagccacaggtgtacaccctgcctccatcccgggacgagctgacaaagaaccaggtgtctctgtggtgtctggtgaagggcttctatccctctgatatcgccgtggagtgggagagcaatggccagcctgagaacaattacaagaccacaccccctgtgctggacagcgatggctccttctttctgtatagcaagctgaccgtggataagtcccggtggcagcagggcaacgtgttttcttgtagcgtgatgcacgaggccctgcacaatcactacacacagaagtccctgtctctgagccctggcaag

SEQ ID NO: 61 - DNA, 681 bp, Artificial Sequence
  hu IgG1 Fc knob DANG
gacaagacccacacatgcccaccttgtccagcaccagagctgctgggaggaccatccgtgttcctgtttccacccaagcccaaggataccctgatgatcagcaggaccccagaggtgacatgcgtggtggtggccgtgtcccacgaggaccctgaggtgaagttcaactggtacgtggatggcgtggaggtgcacaatgccaagacaaagccacgggaggagcagtacggctccacctatagagtggtgtctgtgctgacagtgctgcaccaggactggctgaacggcaaggagtataagtgcaaggtgtctaataaggccctgcctgccccaatcgagaagaccatcagcaaggcaaagggacagccaagggagcctcaggtgtacaccctgcctccatcccgcgacgagctgacaaagaaccaggtgtctctgtggtgtctggtgaagggcttctatccttctgatatcgccgtggagtgggagagcaatggccagccagagaacaattacaagaccacaccccctgtgctggactctgatggcagcttctttctgtatagcaagctgaccgtggataagtccaggtggcagcagggcaacgtgtttagctgttccgtgatgcacgaggccctgcacaatcactacacacagaagtctctgagcctgtcccctggcaag

SEQ ID NO: 62 - DNA, 681 bp, Artificial Sequence
  hu IgG1 Fc hole DANG
gacaagacccacacatgcccaccttgtccagcaccagagctgctgggaggaccatccgtgttcctgtttccacccaagcccaaggataccctgatgatcagcaggaccccagaggtgacatgcgtggtggtggccgtgtcccacgaggaccctgaggtgaagttcaactggtacgtggatggcgtggaggtgcacaatgccaagacaaagccacgggaggagcagtacggcagcacctatagagtggtgtccgtgctgacagtgctgcaccaggactggctgaacggcaaggagtacaagtgcaaggtgtctaataaggccctgcctgccccaatcgagaagaccatcagcaaggcaaagggacagccaagggagcctcaggtgtataccctgcctccaagccgcgacgagctgacaaagaaccaggtgagcctgtcctgtgccgtgaagggcttctacccttccgatatcgccgtggagtgggagtctaatggccagccagagaacaattataagaccacaccccctgtgctggactccgatggctctttctttctggtgtctaagctgaccgtggataagagcaggtggcagcagggcaacgtgttttcttgtagcgtgatgcacgaggccctgcacaatcactatacacagaagtccctgtctctgagccctggcaag

SEQ ID NO: 63 - DNA, 1353 bp, Artificial Sequence
  anti-hu CD20 (Rituximab) HC
caggtgcagctgcagcagccaggagcagagctggtgaagcctggagcctctgtgaagatgagctgcaaggcctccggctacaccttcacaagctataacatgcactgggtgaagcagaccccaggaaggggactggagtggatcggagccatctaccctggcaacggcgacacatcctataatcagaagtttaagggcaaggccaccctgacagccgataagagctcctctaccgcctacatgcagctgagctccctgacaagcgaggactccgccgtgtactattgcgccagaagcacctactatggcggcgattggtacttcaacgtgtggggagcaggaaccacagtgaccgtgtctgccgccagcacaaagggaccatccgtgtttccactggcaccatctagcaagtctaccagcggaggaacagccgccctgggatgtctggtgaaggactacttcccagagcccgtgaccgtgtcctggaactctggcgccctgacctccggagtgcacacatttcccgccgtgctgcagtcctctggcctgtactctctgagctccgtggtgaccgtgccttctagctccctgggcacccagacatatatctgcaacgtgaatcacaagccttccaatacaaaggtggacaagaaggtggagccaaagtcttgtgataagacccacacatgccccccttgtcctgcaccagagctgctgggaggaccaagcgtgttcctgtttccacccaagcccaaggacaccctgatgatcagcaggacccctgaggtgacatgcgtggtggtggacgtgtcccacgaggacccagaggtgaagttcaactggtacgtggatggcgtggaggtgcacaatgccaagacaaagccacgggaggagcagtacaactctacctatagagtggtgagcgtgctgacagtgctgcaccaggattggctgaacggcaaggagtataagtgcaaggtgtctaataaggccctgcccgcccctatcgagaagaccatcagcaaggccaagggccagcctagggagccacaggtgtacaccctgcctccatctcgcgacgagctgacaaagaaccaggtgagcctgacctgtctggtgaagggcttctatccaagcgatatcgccgtggagtgggagtccaatggccagcccgagaacaattacaagaccacaccccctgtgctggacagcgatggctccttctttctgtattccaagctgaccgtggataagtctagatggcagcagggcaacgtgttttcctgttctgtgatgcacgaggccctgcacaatcactacacacagaagagcctgtccctgtctcctggcaag

SEQ ID NO: 64 - DNA, 1353 bp, Artificial Sequence
  anti-mu CD20 HC mu IgG2a Fc knob
caggtgcagctgcagcagccaggagcagagctggtgaggccaggcacctctgtgaagctgagctgcaaggcctccggctacaccttcacatcttattggatgcactggatcaagcagaggccaggacagggactggagtggatcggcgtgatcgacccctccgataactacaccaagtacaaccagaagtttaagggcaaggccaccctgacagtggacaccagctcctctacagcctacatgcagctgagctccctgacatccgaggattctgccgtgtatttctgtgcccgggagggctactatggctctagcccatggtttgcctactggggccagggcaccctggtgacagtgtcctctgccaagaccacagcccccagcgtgtatcctctggccccagtgtgcggcgataccacaggcagctccgtgaccctgggctgtctggtgaagggctacttccctgagccagtgaccctgacatggaactctggcagcctgtctagcggagtgcacacctttccagccgtgctgcagtccgatctgtatacactgtcctctagcgtgaccgtgacatcctctacctggccctcccagtctatcacatgcaacgtggcccaccctgccagctccaccaaggtggacaagaagatcgagccccggggccctacaatcaagccatgtccaccttgcaagtgtccagcacctaatctgctgggaggacctagcgtgttcatctttccacccaagatcaaggacgtgctgatgatcagcctgtcccctatcgtgacctgcgtggtggtggacgtgagcgaggacgatccagatgtgcagatctcctggttcgtgaacaatgtggaggtgcacaccgcccagacccagacacaccgggaggactacaactccacactgagagtggtgtctgccctgcctatccagcaccaggactggatgtccggcaaggagtttaagtgcaaggtgaacaataaggatctgccagcccccatcgagcggaccatctctaagcctaagggcagcgtgagagccccacaggtgtatgtgctgcctccacccgaggaggagatgaccaagaagcaggtgacactgtggtgtatggtgaccgacttcatgcctgaggatatctacgtggagtggaccaacaatggcaagacagagctgaactataagaatacagagccagtgctggacagcgatggctcctactttatgtatagcaagctgagggtggagaagaagaactgggtggagcgcaattcttacagctgttccgtggtgcacgagggcctgcacaatcaccacaccacaaagtctttcagcagaacccccggcaag

SEQ ID NO: 65 - DNA, 639 bp, Artificial Sequence
  anti-mu CD20 LC
cagatcgtgatgagccagtcccctgccatcctgtccgccagccctggcgagaaggtgacaatgacctgcagggccagatcctccgtgtcctacatccactggtaccagcagaagcccggcagcagccctaagccctggatctacgccaccagcaacctggccagcggcgtgcctggcagattttccggctccggcagcggcaccagctacagcctgacaatcacaagggtggaggccgaggatgccgccacatactactgccagcagtggagctccaagcctcccaccttcggcggcggcaccaagctggagatcaagaggaccgacgccgcccccaccgtgtccatctttcccccttcctccgagcagctgacctccggcggcgcttccgtggtgtgtttcctgaataatttctaccctaaggatatcaacgtgaagtggaagatcgatggcagcgagaggcagaatggcgtgctgaatagctggaccgaccaggacagcaaggatagcacctacagcatgagctccacactgaccctgacaaaggacgagtacgagaggcacaattcctacacatgtgaggccacacacaagacctccacctcccctatcgtgaagtccttcaacaggaacgagtgc

SEQ ID NO: 66 - DNA, 2292 bp, Artificial Sequence
  mu scIL-12-mu IgG2a Fc hole
atgtgggagctggagaaggacgtgtacgtggtggaggtggattggacacctgacgcccccggcgagacagtgaacctgacatgcgatacccctgaggaggatgatatcacatggacctccgatcagagacacggcgtgatcggcagcggcaagaccctgacaatcaccgtgaaggagtttctggatgccggccagtacacctgtcacaagggcggcgagacactgagccactcccacctgctgctgcacaagaaggagaatggcatctggtccaccgagatcctgaagaacttcaagaacaagaccttcctgaagtgtgaggcccctaattactccggcaggtttacatgctcctggctggtgcagagaaacatggacctgaagtttaatatcaagagctcctcctccagccccgatagcagagccgtgacctgtggcatggccagcctgagcgccgagaaggtgaccctggatcagagggattacgagaagtactccgtgtcctgtcaggaggatgtgacatgtcctacagccgaggagacactgcctatcgagctggccctggaggccaggcagcagaataagtacgagaactacagcacaagctttttcatcagggacatcatcaagcccgatccccccaagaacctgcagatgaagcccctgaagaacagccaggtggaggtgtcctgggagtaccctgatagctggtccacccctcactcctacttctccctgaagttctttgtgagaatccagagaaagaaggagaagatgaaggagacagaggagggctgcaatcagaagggcgccttcctggtggagaagacatccaccgaggtgcagtgtaagggcggcaacgtgtgcgtgcaggcccaggacagatactacaattccagctgtagcaagtgggcctgtgtgccttgtagagtgagatccggcggcggcggctccggaggaggaggaagcggaggaggcggctccagagtgatccctgtgtccggccctgccagatgtctgtcccagagcagaaacctgctgaagaccacagacgacatggtgaagacagccagagagaagctgaagcactacagctgcaccgccgaggacatcgaccacgaggatatcacaagagaccagacatccaccctgaagacatgtctgcctctggagctgcacaagaatgagtcctgcctggccaccagagagacctccagcaccaccaggggcagctgcctgccccctcagaagacctccctgatgatgacactgtgcctgggcagcatctacgaggacctgaagatgtaccagaccgagttccaggccatcaatgccgccctgcagaaccacaaccaccagcagatcatcctggataagggcatgctggtggccatcgacgagctgatgcagagcctgaaccacaatggcgagaccctgaggcagaagcctcctgtgggcgaggccgatccctacagagtgaagatgaagctgtgtatcctgctgcacgccttttccacaagggtggtgaccatcaacagggtcatgggctacctgtccagcgccggcggcggcggcagcggaggaggaggctccgagccacgcggccccacaatcaagccatgccccccttgcaagtgtcctgcaccaaatctgctgggaggaccatccgtgttcatctttccacccaagatcaaggacgtgctgatgatcagcctgtccccaatcgtgacctgcgtggtcgtggacgtgagcgaggacgatcctgatgtgcagatctcctggttcgtgaacaatgtggaggtgcacaccgcccagacccagacacaccgggaggactacaactccacactgagagtggtgtctgccctgcccatccagcaccaggactggatgagcggcaaggagtttaagtgcaaggtgaacaataaggatctgcccgcccctatcgagcggacaatctctaagcctaagggcagcgtgagagccccacaggtgtatgtgctgcctccacccgaggaggagatgaccaagaagcaggtgacactgtcttgtgccgtgaccgacttcatgcctgaggatatctatgtggagtggaccaacaatggcaagacagagctgaactacaagaatacagagccagtgctggactccgatggctcttacttcatggtgagcaagctgagggtggagaagaagaactgggtggagcgcaattcttacagctgctccgtggtgcacgagggcctgcacaaccaccacaccacaaagtcttttagccggacccctggcaag

SEQ ID NO: 67 - DNA, 2292 bp, Artificial Sequence
  mu scIL-12 mut1-mu IgG2a Fc hole
atgtgggagctggagaaggacgtgtacgtggtggaggtggattggacacctgacgcccccggcgagacagtgaacctgacatgcgatacccctgaggaggatgatatcacatggacctccgatcagagacacggcgtgatcggcagcggcaagaccctgacaatcaccgtgaaggagtttctggatgccggccagtacacctgtcacaagggcggcgagacactgagccactcccacctgctgctgcacaagaaggagaatggcatctggtccaccgagatcctgaagaacttcaagaacaagaccttcctgaagtgtgaggcccctaattactccggcaggtttacatgctcctggctggtgcagagaaacatggacctgaagtttaatatcaagagctcctcctccagccccgatagcagagccgtgacctgtggcatggccagcctgagcgccgagaaggtgaccctggatcagagggattacgagaagtactccgtgtcctgtcaggaggatgtgacatgtcctacagccgaggagacactgcctatcgagctggccctggaggccaggcagcagaataagtacgagaactacagcacaagctttttcatcagggacatcatcaagcccgatccccccaagaacctgcagatgaagcccctgaagaacagccaggtggaggtgtcctgggagtaccctgatagctggtccacccctcactcctacttctccctgaagttctttgtgagaatccagagagccaaggagaagatggccgagacagaggagggctgcaatcagaagggcgccttcctggtggagaagacatccaccgaggtgcagtgtaagggcggcaacgtgtgcgtgcaggcccaggacagatactacaattccagctgtagcaagtgggcctgtgtgccttgtagagtgagatccggcggcggcggctccggaggaggaggaagcggaggaggcggctccagagtgatccctgtgtccggccctgccagatgtctgtcccagagcagaaacctgctgaagaccacagacgacatggtgaagacagccagagagaagctgaagcactacagctgcaccgccgaggacatcgaccacgaggatatcacaagagaccagacatccaccctgaagacatgtctgcctctggagctgcacaagaatgagtcctgcctggccaccagagagacctccagcaccaccaggggcagctgcctgccccctcagaagacctccctgatgatgacactgtgcctgggcagcatctacgaggacctgaagatgtaccagaccgagttccaggccatcaatgccgccctgcagaaccacaaccaccagcagatcatcctggataagggcatgctggtggccatcgacgagctgatgcagagcctgaaccacaatggcgagaccctgaggcagaagcctcctgtgggcgaggccgatccctacagagtgaagatgaagctgtgtatcctgctgcacgccttttccacaagggtggtgaccatcaacagggtcatgggctacctgtccagcgccggcggcggcggcagcggaggaggaggctccgagccacgcggccccacaatcaagccatgccccccttgcaagtgtcctgcaccaaatctgctgggaggaccatccgtgttcatctttccacccaagatcaaggacgtgctgatgatcagcctgtccccaatcgtgacctgcgtggtcgtggacgtgagcgaggacgatcctgatgtgcagatctcctggttcgtgaacaatgtggaggtgcacaccgcccagacccagacacaccgggaggactacaactccacactgagagtggtgtctgccctgcccatccagcaccaggactggatgagcggcaaggagtttaagtgcaaggtgaacaataaggatctgcccgcccctatcgagcggacaatctctaagcctaagggcagcgtgagagccccacaggtgtatgtgctgcctccacccgaggaggagatgaccaagaagcaggtgacactgtcttgtgccgtgaccgacttcatgcctgaggatatctatgtggagtggaccaacaatggcaagacagagctgaactacaagaatacagagccagtgctggactccgatggctcttacttcatggtgagcaagctgagggtggagaagaagaactgggtggagcgcaattcttacagctgctccgtggtgcacgagggcctgcacaaccaccacaccacaaagtcttttagccggacccctggcaag

SEQ ID NO: 68 - DNA, 2292 bp, Artificial Sequence
  mu scIL-12 mut2-mu IgG2a Fc hole
atgtgggagctggagaaggacgtgtacgtggtggaggtggattggacacctgacgcccccggcgagacagtgaacctgacatgcgatacccctgaggaggatgatatcacatggacctccgatcagagacacggcgtgatcggcagcggcaagaccctgacaatcaccgtgaaggagtttctggatgccggccagtacacctgtcacaagggcggcgagacactgagccactcccacctgctgctgcacaagaaggagaatggcatctggtccaccgagatcctgaagaacttcaagaacaagaccttcctgaagtgtgaggcccctaattactccggcaggtttacatgctcctggctggtgcagagaaacatggacctgaagtttaatatcaagagctcctcctccagccccgatagcagagccgtgacctgtggcatggccagcctgagcgccgagaaggtgaccctggatcagagggattacgagaagtactccgtgtcctgtcaggaggatgtgacatgtcctacagccgaggagacactgcctatcgagctggccctggaggccaggcagcagaataagtacgagaactacagcacaagctttttcatcagggacatcatcaagcccgatccccccaagaacctgcagatgaagcccctgaagaacagccaggtggaggtgtcctgggagtaccctgatagctggtccacccctcactcctacttctccctgaagttctttgtgagaatccaggccgccgctgagaagatggccgagacagaggagggctgcaatcagaagggcgccttcctggtggagaagacatccaccgaggtgcagtgtaagggcggcaacgtgtgcgtgcaggcccaggacagatactacaattccagctgtagcaagtgggcctgtgtgccttgtagagtgagatccggcggcggcggctccggaggaggaggaagcggaggaggcggctccagagtgatccctgtgtccggccctgccagatgtctgtcccagagcagaaacctgctgaagaccacagacgacatggtgaagacagccagagagaagctgaagcactacagctgcaccgccgaggacatcgaccacgaggatatcacaagagaccagacatccaccctgaagacatgtctgcctctggagctgcacaagaatgagtcctgcctggccaccagagagacctccagcaccaccaggggcagctgcctgccccctcagaagacctccctgatgatgacactgtgcctgggcagcatctacgaggacctgaagatgtaccagaccgagttccaggccatcaatgccgccctgcagaaccacaaccaccagcagatcatcctggataagggcatgctggtggccatcgacgagctgatgcagagcctgaaccacaatggcgagaccctgaggcagaagcctcctgtgggcgaggccgatccctacagagtgaagatgaagctgtgtatcctgctgcacgccttttccacaagggtggtgaccatcaacagggtcatgggctacctgtccagcgccggcggcggcggcagcggaggaggaggctccgagccacgcggccccacaatcaagccatgccccccttgcaagtgtcctgcaccaaatctgctgggaggaccatccgtgttcatctttccacccaagatcaaggacgtgctgatgatcagcctgtccccaatcgtgacctgcgtggtcgtggacgtgagcgaggacgatcctgatgtgcagatctcctggttcgtgaacaatgtggaggtgcacaccgcccagacccagacacaccgggaggactacaactccacactgagagtggtgtctgccctgcccatccagcaccaggactggatgagcggcaaggagtttaagtgcaaggtgaacaataaggatctgcccgcccctatcgagcggacaatctctaagcctaagggcagcgtgagagccccacaggtgtatgtgctgcctccacccgaggaggagatgaccaagaagcaggtgacactgtcttgtgccgtgaccgacttcatgcctgaggatatctatgtggagtggaccaacaatggcaagacagagctgaactacaagaatacagagccagtgctggactccgatggctcttacttcatggtgagcaagctgagggtggagaagaagaactgggtggagcgcaattcttacagctgctccgtggtgcacgagggcctgcacaaccaccacaccacaaagtcttttagccggacccctggcaag

SEQ ID NO: 69 - DNA, 1761 bp, Artificial Sequence
  (anti-mu CD20 VH)2-mu IgG2a Fc knob
caagtgcagctgcagcaacctggtgctgagctggtgcgccccggcacaagcgtgaagctcagctgcaaggcctccggatacaccttcactagctactggatgcactggattaaacagcggcctggccagggcctggaatggatcggcgtgatcgatcccagcgacaactacacaaagtacaaccagaagttcaagggcaaggccacactgacagtggacaccagcagctccaccgcctatatgcagctgagctccctgaccagcgaggattctgccgtgtacttctgcgccagagagggctactacggctccagcccttggttcgcctactggggccagggcaccctggtcaccgtgtcctccggcggcggcggaagcggcggcggcggcagcggaggaggcggaagccaggtgcagctgcagcagccaggagcagagctggtgaggccaggcacctctgtgaagctgagctgcaaggcctccggctacaccttcacatcttattggatgcactggatcaagcagaggccaggacagggactggagtggatcggcgtgatcgacccctccgataactacaccaagtacaaccagaagtttaagggcaaggccaccctgacagtggacaccagctcctctacagcctacatgcagctgagctccctgacatccgaggattctgccgtgtatttctgtgcccgggagggctactatggctctagcccatggtttgcctactggggccagggcaccctggtgacagtgtcctctgccaagaccacagcccccagcgtgtatcctctggccccagtgtgcggcgataccacaggcagctccgtgaccctgggctgtctggtgaagggctacttccctgagccagtgaccctgacatggaactctggcagcctgtctagcggagtgcacacctttccagccgtgctgcagtccgatctgtatacactgtcctctagcgtgaccgtgacatcctctacctggccctcccagtctatcacatgcaacgtggcccaccctgccagctccaccaaggtggacaagaagatcgagccccggggccctacaatcaagccatgtccaccttgcaagtgtccagcacctaatctgctgggaggacctagcgtgttcatctttccacccaagatcaaggacgtgctgatgatcagcctgtcccctatcgtgacctgcgtggtggtggacgtgagcgaggacgatccagatgtgcagatctcctggttcgtgaacaatgtggaggtgcacaccgcccagacccagacacaccgggaggactacaactccacactgagagtggtgtctgccctgcctatccagcaccaggactggatgtccggcaaggagtttaagtgcaaggtgaacaataaggatctgccagcccccatcgagcggaccatctctaagcctaagggcagcgtgagagccccacaggtgtatgtgctgcctccacccgaggaggagatgaccaagaagcaggtgacactgtggtgtatggtgaccgacttcatgcctgaggatatctacgtggagtggaccaacaatggcaagacagagctgaactataagaatacagagccagtgctggacagcgatggctcctactttatgtatagcaagctgagggtggagaagaagaactgggtggagcgcaattcttacagctgttccgtggtgcacgagggcctgcacaatcaccacaccacaaagtctttcagcagaacccccggcaag

SEQ ID NO: 70 - DNA, 1002 bp, Artificial Sequence
  (anti-mu CD20 VL)2
cagatcgtgatgagccagagccccgccatcctgtctgctagtcctggcgagaaggtgacaatgacctgtagagcccggagcagcgtttcttatatccactggtaccagcagaaacccggctcttctccaaagccttggatctacgccaccagcaatctggccagcggagtgccaggtagattcagcggcagcggaagcggaacctcttacagcctgaccatcaccagagtggaagccgaggacgccgctacatactactgccagcagtggagcagcaaacctcctacctttggcggcggcaccaagctggaaatcaagggcggcggaggctctggcggagggggcagcggcggcggcggcagtcagatcgtgatgtcccagtctccagcaatcctgagcgcctcccctggagagaaggtgaccatgacatgccgggccagaagctccgtgagctacatccactggtatcagcagaagccaggctctagccctaagccatggatctacgccaccagcaacctggcatccggagtgccaggccggttctctggcagcggctccggcacatcttatagcctgaccatcacaagagtggaggccgaggacgccgccacctactattgccagcagtggtcctctaagccccctacattcggcggcggcaccaagctggagatcaagaggactgatgcagcacctacagtgtccatctttccacccagctccgagcagctgacctctggaggagcaagcgtggtgtgcttcctgaacaacttctacccaaaggacatcaacgtgaagtggaagatcgatggctccgagcggcagaacggcgtgctgaacagctggacagaccaggatagcaaggactccacctattctatgtctagcaccctgacactgaccaaggatgagtacgagaggcacaatagctatacatgcgaggccacccacaagacatccacctctcccatcgtgaagtcctttaaccgcaatgagtgt

SEQ ID NO: 71 - DNA, 2139 bp, Artificial Sequence
  anti-mu CD20 HC mu IgG2a Fc knob-anti-mu CD20 scFv
caggtgcagctgcagcagccaggagcagagctggtgaggccaggcacctctgtgaagctgagctgcaaggcctccggctacaccttcacatcttattggatgcactggatcaagcagaggccaggacagggactggagtggatcggcgtgatcgacccctccgataactacaccaagtacaaccagaagtttaagggcaaggccaccctgacagtggacaccagctcctctacagcctacatgcagctgagctccctgacatccgaggattctgccgtgtatttctgtgcccgggagggctactatggctctagcccatggtttgcctactggggccagggcaccctggtgacagtgtcctctgccaagaccacagcccccagcgtgtatcctctggccccagtgtgcggcgataccacaggcagctccgtgaccctgggctgtctggtgaagggctacttccctgagccagtgaccctgacatggaactctggcagcctgtctagcggagtgcacacctttccagccgtgctgcagtccgatctgtatacactgtcctctagcgtgaccgtgacatcctctacctggccctcccagtctatcacatgcaacgtggcccaccctgccagctccaccaaggtggacaagaagatcgagccccggggccctacaatcaagccatgtccaccttgcaagtgtccagcacctaatctgctgggaggacctagcgtgttcatctttccacccaagatcaaggacgtgctgatgatcagcctgtcccctatcgtgacctgcgtggtggtggacgtgagcgaggacgatccagatgtgcagatctcctggttcgtgaacaatgtggaggtgcacaccgcccagacccagacacaccgggaggactacaactccacactgagagtggtgtctgccctgcctatccagcaccaggactggatgtccggcaaggagtttaagtgcaaggtgaacaataaggatctgccagcccccatcgagcggaccatctctaagcctaagggcagcgtgagagccccacaggtgtatgtgctgcctccacccgaggaggagatgaccaagaagcaggtgacactgtggtgtatggtgaccgacttcatgcctgaggatatctacgtggagtggaccaacaatggcaagacagagctgaactataagaatacagagccagtgctggacagcgatggctcctactttatgtatagcaagctgagggtggagaagaagaactgggtggagcgcaattcttacagctgttccgtggtgcacgagggcctgcacaatcaccacaccacaaagtctttcagcagaacccccggcaagggcggcggaggctctggcggagggggcagcggcggcggcggcagtcaagtgcagctgcagcaacctggtgctgagctggtgcgccccggcacaagcgtgaagctcagctgcaaggcctccggatacaccttcactagctactggatgcactggattaaacagcggcctggccagggcctggaatggatcggcgtgatcgatcccagcgacaactacacaaagtacaaccagaagttcaagggcaaggccacactgacagtggacaccagcagctccaccgcctatatgcagctgagctccctgaccagcgaggattctgccgtgtacttctgcgccagagagggctactacggctccagcccttggttcgcctactggggccagggcaccctggtcaccgtgtcctccggcggcggcggaagcggcggcggcggcagcggaggaggcggaagcggcggcggcggatctcagatcgtgatgagccagagccccgccatcctgtctgctagtcctggcgagaaggtgacaatgacctgtagagcccggagcagcgtttcttatatccactggtaccagcagaaacccggctcttctccaaagccttggatctacgccaccagcaatctggccagcggagtgccaggtagattcagcggcagcggaagcggaacctcttacagcctgaccatcaccagagtggaagccgaggacgccgctacatactactgccagcagtggagcagcaaacctcctacctttggcggcggcaccaagctggaaatcaag

SEQ ID NO: 72 - DNA, 1425 bp, Artificial Sequence
  anti-mu CD20 LC-anti-mu CD20 scFv
cagatcgtgatgtcccagtctccagcaatcctgagcgcctcccctggagagaaggtgaccatgacatgccgggccagaagctccgtgagctacatccactggtatcagcagaagccaggctctagccctaagccatggatctacgccaccagcaacctggcatccggagtgccaggccggttctctggcagcggctccggcacatcttatagcctgaccatcacaagagtggaggccgaggacgccgccacctactattgccagcagtggtcctctaagccccctacattcggcggcggcaccaagctggagatcaagaggactgatgcagcacctacagtgtccatctttccacccagctccgagcagctgacctctggaggagcaagcgtggtgtgcttcctgaacaacttctacccaaaggacatcaacgtgaagtggaagatcgatggctccgagcggcagaacggcgtgctgaacagctggacagaccaggatagcaaggactccacctattctatgtctagcaccctgacactgaccaaggatgagtacgagaggcacaatagctatacatgcgaggccacccacaagacatccacctctcccatcgtgaagtcctttaaccgcaatgagtgtggcggcggaggctctggcggagggggcagcggcggcggcggcagtcaagtgcagctgcagcaacctggtgctgagctggtgcgccccggcacaagcgtgaagctcagctgcaaggcctccggatacaccttcactagctactggatgcactggattaaacagcggcctggccagggcctggaatggatcggcgtgatcgatcccagcgacaactacacaaagtacaaccagaagttcaagggcaaggccacactgacagtggacaccagcagctccaccgcctatatgcagctgagctccctgaccagcgaggattctgccgtgtacttctgcgccagagagggctactacggctccagcccttggttcgcctactggggccagggcaccctggtcaccgtgtcctccggcggcggcggaagcggcggcggcggcagcggaggaggcggaagcggcggcggcggatctcagatcgtgatgagccagagccccgccatcctgtctgctagtcctggcgagaaggtgacaatgacctgtagagcccggagcagcgtttcttatatccactggtaccagcagaaacccggctcttctccaaagccttggatctacgccaccagcaatctggccagcggagtgccaggtagattcagcggcagcggaagcggaacctcttacagcctgaccatcaccagagtggaagccgaggacgccgctacatactactgccagcagtggagcagcaaacctcctacctttggcggcggcaccaagctggaaatcaag

SEQ ID NO: 73 - DNA, 2961 bp, Artificial Sequence
  anti-mu CD20 HC mu IgG2a Fc hole-mu scIL-12
caggtgcagctgcagcagccaggagcagagctggtgaggccaggcacctctgtgaagctgagctgcaaggcctccggctacaccttcacatcttattggatgcactggatcaagcagaggccaggacagggactggagtggatcggcgtgatcgacccctccgataactacaccaagtacaaccagaagtttaagggcaaggccaccctgacagtggacaccagctcctctacagcctacatgcagctgagctccctgacatccgaggattctgccgtgtatttctgtgcccgggagggctactatggctctagcccatggtttgcctactggggccagggcaccctggtgacagtgtcctctgccaagaccacagcccccagcgtgtatcctctggccccagtgtgcggcgataccacaggcagctccgtgaccctgggctgtctggtgaagggctacttccctgagccagtgaccctgacatggaactctggcagcctgtctagcggagtgcacacctttccagccgtgctgcagtccgatctgtatacactgtcctctagcgtgaccgtgacatcctctacctggccctcccagtctatcacatgcaacgtggcccaccctgccagctccaccaaggtggacaagaagatcgagccacgcggccccacaatcaagccatgccccccttgcaagtgtcctgcaccaaatctgctgggaggaccatccgtgttcatctttccacccaagatcaaggacgtgctgatgatcagcctgtccccaatcgtgacctgcgtggtcgtggacgtgagcgaggacgatcctgatgtgcagatctcctggttcgtgaacaatgtggaggtgcacaccgcccagacccagacacaccgggaggactacaactccacactgagagtggtgtctgccctgcccatccagcaccaggactggatgagcggcaaggagtttaagtgcaaggtgaacaataaggatctgcccgcccctatcgagcggacaatctctaagcctaagggcagcgtgagagccccacaggtgtatgtgctgcctccacccgaggaggagatgaccaagaagcaggtgacactgtcttgtgccgtgaccgacttcatgcctgaggatatctatgtggagtggaccaacaatggcaagacagagctgaactacaagaatacagagccagtgctggactccgatggctcttacttcatggtgagcaagctgagggtggagaagaagaactgggtggagcgcaattcttacagctgctccgtggtgcacgagggcctgcacaaccaccacaccacaaagtcttttagccggacccctggcaagggtggaggtggctcaggaggaggcggttctggcggaggaggtagtatgtgggagctggagaaggacgtgtacgtggtggaggtggattggacacctgacgcccccggcgagacagtgaacctgacatgcgatacccctgaggaggatgatatcacatggacctccgatcagagacacggcgtgatcggcagcggcaagaccctgacaatcaccgtgaaggagtttctggatgccggccagtacacctgtcacaagggcggcgagacactgagccactcccacctgctgctgcacaagaaggagaatggcatctggtccaccgagatcctgaagaacttcaagaacaagaccttcctgaagtgtgaggcccctaattactccggcaggtttacatgctcctggctggtgcagagaaacatggacctgaagtttaatatcaagagctcctcctccagccccgatagcagagccgtgacctgtggcatggccagcctgagcgccgagaaggtgaccctggatcagagggattacgagaagtactccgtgtcctgtcaggaggatgtgacatgtcctacagccgaggagacactgcctatcgagctggccctggaggccaggcagcagaataagtacgagaactacagcacaagctttttcatcagggacatcatcaagcccgatccccccaagaacctgcagatgaagcccctgaagaacagccaggtggaggtgtcctgggagtaccctgatagctggtccacccctcactcctacttctccctgaagttctttgtgagaatccagagaaagaaggagaagatgaaggagacagaggagggctgcaatcagaagggcgccttcctggtggagaagacatccaccgaggtgcagtgtaagggcggcaacgtgtgcgtgcaggcccaggacagatactacaattccagctgtagcaagtgggcctgtgtgccttgtagagtgagatccggcggcggcggctccggaggaggaggaagcggaggaggcggctccagagtgatccctgtgtccggccctgccagatgtctgtcccagagcagaaacctgctgaagaccacagacgacatggtgaagacagccagagagaagctgaagcactacagctgcaccgccgaggacatcgaccacgaggatatcacaagagaccagacatccaccctgaagacatgtctgcctctggagctgcacaagaatgagtcctgcctggccaccagagagacctccagcaccaccaggggcagctgcctgccccctcagaagacctccctgatgatgacactgtgcctgggcagcatctacgaggacctgaagatgtaccagaccgagttccaggccatcaatgccgccctgcagaaccacaaccaccagcagatcatcctggataagggcatgctggtggccatcgacgagctgatgcagagcctgaaccacaatggcgagaccctgaggcagaagcctcctgtgggcgaggccgatccctacagagtgaagatgaagctgtgtatcctgctgcacgccttttccacaagggtggtgaccatcaacagggtcatgggctacctgtccagcgcc

SEQ ID NO: 74 - DNA, 2961 bp, Artificial Sequence
  anti-mu CD20 HC mu IgG2a Fc hole-mu scIL-12 mut2
caggtgcagctgcagcagccaggagcagagctggtgaggccaggcacctctgtgaagctgagctgcaaggcctccggctacaccttcacatcttattggatgcactggatcaagcagaggccaggacagggactggagtggatcggcgtgatcgacccctccgataactacaccaagtacaaccagaagtttaagggcaaggccaccctgacagtggacaccagctcctctacagcctacatgcagctgagctccctgacatccgaggattctgccgtgtatttctgtgcccgggagggctactatggctctagcccatggtttgcctactggggccagggcaccctggtgacagtgtcctctgccaagaccacagcccccagcgtgtatcctctggccccagtgtgcggcgataccacaggcagctccgtgaccctgggctgtctggtgaagggctacttccctgagccagtgaccctgacatggaactctggcagcctgtctagcggagtgcacacctttccagccgtgctgcagtccgatctgtatacactgtcctctagcgtgaccgtgacatcctctacctggccctcccagtctatcacatgcaacgtggcccaccctgccagctccaccaaggtggacaagaagatcgagccacgcggccccacaatcaagccatgccccccttgcaagtgtcctgcaccaaatctgctgggaggaccatccgtgttcatctttccacccaagatcaaggacgtgctgatgatcagcctgtccccaatcgtgacctgcgtggtcgtggacgtgagcgaggacgatcctgatgtgcagatctcctggttcgtgaacaatgtggaggtgcacaccgcccagacccagacacaccgggaggactacaactccacactgagagtggtgtctgccctgcccatccagcaccaggactggatgagcggcaaggagtttaagtgcaaggtgaacaataaggatctgcccgcccctatcgagcggacaatctctaagcctaagggcagcgtgagagccccacaggtgtatgtgctgcctccacccgaggaggagatgaccaagaagcaggtgacactgtcttgtgccgtgaccgacttcatgcctgaggatatctatgtggagtggaccaacaatggcaagacagagctgaactacaagaatacagagccagtgctggactccgatggctcttacttcatggtgagcaagctgagggtggagaagaagaactgggtggagcgcaattcttacagctgctccgtggtgcacgagggcctgcacaaccaccacaccacaaagtcttttagccggacccctggcaagggtggaggtggctcaggaggaggcggttctggcggaggaggtagtatgtgggagctggagaaggacgtgtacgtggtggaggtggattggacacctgacgcccccggcgagacagtgaacctgacatgcgatacccctgaggaggatgatatcacatggacctccgatcagagacacggcgtgatcggcagcggcaagaccctgacaatcaccgtgaaggagtttctggatgccggccagtacacctgtcacaagggcggcgagacactgagccactcccacctgctgctgcacaagaaggagaatggcatctggtccaccgagatcctgaagaacttcaagaacaagaccttcctgaagtgtgaggcccctaattactccggcaggtttacatgctcctggctggtgcagagaaacatggacctgaagtttaatatcaagagctcctcctccagccccgatagcagagccgtgacctgtggcatggccagcctgagcgccgagaaggtgaccctggatcagagggattacgagaagtactccgtgtcctgtcaggaggatgtgacatgtcctacagccgaggagacactgcctatcgagctggccctggaggccaggcagcagaataagtacgagaactacagcacaagctttttcatcagggacatcatcaagcccgatccccccaagaacctgcagatgaagcccctgaagaacagccaggtggaggtgtcctgggagtaccctgatagctggtccacccctcactcctacttctccctgaagttctttgtgagaatccaggctgccgccgagaagatggccgagacagaggagggctgcaatcagaagggcgccttcctggtggagaagacatccaccgaggtgcagtgtaagggcggcaacgtgtgcgtgcaggcccaggacagatactacaattccagctgtagcaagtgggcctgtgtgccttgtagagtgagatccggcggcggcggctccggaggaggaggaagcggaggaggcggctccagagtgatccctgtgtccggccctgccagatgtctgtcccagagcagaaacctgctgaagaccacagacgacatggtgaagacagccagagagaagctgaagcactacagctgcaccgccgaggacatcgaccacgaggatatcacaagagaccagacatccaccctgaagacatgtctgcctctggagctgcacaagaatgagtcctgcctggccaccagagagacctccagcaccaccaggggcagctgcctgccccctcagaagacctccctgatgatgacactgtgcctgggcagcatctacgaggacctgaagatgtaccagaccgagttccaggccatcaatgccgccctgcagaaccacaaccaccagcagatcatcctggataagggcatgctggtggccatcgacgagctgatgcagagcctgaaccacaatggcgagaccctgaggcagaagcctcctgtgggcgaggccgatccctacagagtgaagatgaagctgtgtatcctgctgcacgccttttccacaagggtggtgaccatcaacagggtcatgggctacctgtccagcgcc

SEQ ID NO: 75 - DNA, 1353 bp, Artificial Sequence
  anti-mu CD20 HC mu IgG2a Fc knob DANG
caggtgcagctgcagcagccaggagcagagctggtgaggccaggcacctctgtgaagctgagctgcaaggcctccggctacaccttcacatcttattggatgcactggatcaagcagaggccaggacagggactggagtggatcggcgtgatcgacccctccgataactacaccaagtacaaccagaagtttaagggcaaggccaccctgacagtggacaccagctcctctacagcctacatgcagctgagctccctgacatccgaggattctgccgtgtatttctgtgcccgggagggctactatggctctagcccatggtttgcctactggggccagggcaccctggtgacagtgtcctctgccaagaccacagcccccagcgtgtatcctctggccccagtgtgcggcgataccacaggcagctccgtgaccctgggctgtctggtgaagggctacttccctgagccagtgaccctgacatggaactctggcagcctgtctagcggagtgcacacctttccagccgtgctgcagtccgatctgtatacactgtcctctagcgtgaccgtgacatcctctacctggccctcccagtctatcacatgcaacgtggcccaccctgccagctccaccaaggtggacaagaagatcgagccccggggccctacaatcaagccatgtccaccttgcaagtgtccagcacctaatctgctgggaggacctagcgtgttcatctttccacccaagatcaaggacgtgctgatgatcagcctgtcccctatcgtgacctgcgtggtggtggccgtgagcgaggacgatccagatgtgcagatctcctggttcgtgaacaatgtggaggtgcacaccgcccagacccagacacaccgggaggactacggctccacactgagagtggtgtctgccctgcctatccagcaccaggactggatgtccggcaaggagtttaagtgcaaggtgaacaataaggatctgccagcccccatcgagcggaccatctctaagcctaagggcagcgtgagagccccacaggtgtatgtgctgcctccacccgaggaggagatgaccaagaagcaggtgacactgtggtgtatggtgaccgacttcatgcctgaggatatctacgtggagtggaccaacaatggcaagacagagctgaactataagaatacagagccagtgctggacagcgatggctcctactttatgtatagcaagctgagggtggagaagaagaactgggtggagcgcaattcttacagctgttccgtggtgcacgagggcctgcacaatcaccacaccacaaagtctttcagcagaacccccggcaag

SEQ ID NO: 76 - DNA, 2292 bp, Artificial Sequence
  mu scIL-12-mu IgG2a Fc hole DANG
atgtgggagctggagaaggacgtgtacgtggtggaggtggattggacacctgacgcccccggcgagacagtgaacctgacatgcgatacccctgaggaggatgatatcacatggacctccgatcagagacacggcgtgatcggcagcggcaagaccctgacaatcaccgtgaaggagtttctggatgccggccagtacacctgtcacaagggcggcgagacactgagccactcccacctgctgctgcacaagaaggagaatggcatctggtccaccgagatcctgaagaacttcaagaacaagaccttcctgaagtgtgaggcccctaattactccggcaggtttacatgctcctggctggtgcagagaaacatggacctgaagtttaatatcaagagctcctcctccagccccgatagcagagccgtgacctgtggcatggccagcctgagcgccgagaaggtgaccctggatcagagggattacgagaagtactccgtgtcctgtcaggaggatgtgacatgtcctacagccgaggagacactgcctatcgagctggccctggaggccaggcagcagaataagtacgagaactacagcacaagctttttcatcagggacatcatcaagcccgatccccccaagaacctgcagatgaagcccctgaagaacagccaggtggaggtgtcctgggagtaccctgatagctggtccacccctcactcctacttctccctgaagttctttgtgagaatccagagaaagaaggagaagatgaaggagacagaggagggctgcaatcagaagggcgccttcctggtggagaagacatccaccgaggtgcagtgtaagggcggcaacgtgtgcgtgcaggcccaggacagatactacaattccagctgtagcaagtgggcctgtgtgccttgtagagtgagatccggcggcggcggctccggaggaggaggaagcggaggaggcggctccagagtgatccctgtgtccggccctgccagatgtctgtcccagagcagaaacctgctgaagaccacagacgacatggtgaagacagccagagagaagctgaagcactacagctgcaccgccgaggacatcgaccacgaggatatcacaagagaccagacatccaccctgaagacatgtctgcctctggagctgcacaagaatgagtcctgcctggccaccagagagacctccagcaccaccaggggcagctgcctgccccctcagaagacctccctgatgatgacactgtgcctgggcagcatctacgaggacctgaagatgtaccagaccgagttccaggccatcaatgccgccctgcagaaccacaaccaccagcagatcatcctggataagggcatgctggtggccatcgacgagctgatgcagagcctgaaccacaatggcgagaccctgaggcagaagcctcctgtgggcgaggccgatccctacagagtgaagatgaagctgtgtatcctgctgcacgccttttccacaagggtggtgaccatcaacagggtcatgggctacctgtccagcgccggcggcggcggcagcggaggaggaggctccgagccacgcggccccacaatcaagccatgccccccttgcaagtgtcctgcaccaaatctgctgggaggaccatccgtgttcatctttccacccaagatcaaggacgtgctgatgatcagcctgtccccaatcgtgacctgcgtggtcgtggccgtgagcgaggacgatcctgatgtgcagatctcctggttcgtgaacaatgtggaggtgcacaccgcccagacccagacacaccgggaggactacggctccacactgagagtggtgtctgccctgcccatccagcaccaggactggatgagcggcaaggagtttaagtgcaaggtgaacaataaggatctgcccgcccctatcgagcggacaatctctaagcctaagggcagcgtgagagccccacaggtgtatgtgctgcctccacccgaggaggagatgaccaagaagcaggtgacactgtcttgtgccgtgaccgacttcatgcctgaggatatctatgtggagtggaccaacaatggcaagacagagctgaactacaagaatacagagccagtgctggactccgatggctcttacttcatggtgagcaagctgagggtggagaagaagaactgggtggagcgcaattcttacagctgctccgtggtgcacgagggcctgcacaaccaccacaccacaaagtcttttagccggacccctggcaag

SEQ ID NO: 77 - DNA, 2292 bp, Artificial Sequence
  mu scIL-12 mut1-mu IgG2a Fc hole DANG
atgtgggagctggagaaggacgtgtacgtggtggaggtggattggacacctgacgcccccggcgagacagtgaacctgacatgcgatacccctgaggaggatgatatcacatggacctccgatcagagacacggcgtgatcggcagcggcaagaccctgacaatcaccgtgaaggagtttctggatgccggccagtacacctgtcacaagggcggcgagacactgagccactcccacctgctgctgcacaagaaggagaatggcatctggtccaccgagatcctgaagaacttcaagaacaagaccttcctgaagtgtgaggcccctaattactccggcaggtttacatgctcctggctggtgcagagaaacatggacctgaagtttaatatcaagagctcctcctccagccccgatagcagagccgtgacctgtggcatggccagcctgagcgccgagaaggtgaccctggatcagagggattacgagaagtactccgtgtcctgtcaggaggatgtgacatgtcctacagccgaggagacactgcctatcgagctggccctggaggccaggcagcagaataagtacgagaactacagcacaagctttttcatcagggacatcatcaagcccgatccccccaagaacctgcagatgaagcccctgaagaacagccaggtggaggtgtcctgggagtaccctgatagctggtccacccctcactcctacttctccctgaagttctttgtgagaatccagagagccaaggagaagatggccgagacagaggagggctgcaatcagaagggcgccttcctggtggagaagacatccaccgaggtgcagtgtaagggcggcaacgtgtgcgtgcaggcccaggacagatactacaattccagctgtagcaagtgggcctgtgtgccttgtagagtgagatccggcggcggcggctccggaggaggaggaagcggaggaggcggctccagagtgatccctgtgtccggccctgccagatgtctgtcccagagcagaaacctgctgaagaccacagacgacatggtgaagacagccagagagaagctgaagcactacagctgcaccgccgaggacatcgaccacgaggatatcacaagagaccagacatccaccctgaagacatgtctgcctctggagctgcacaagaatgagtcctgcctggccaccagagagacctccagcaccaccaggggcagctgcctgccccctcagaagacctccctgatgatgacactgtgcctgggcagcatctacgaggacctgaagatgtaccagaccgagttccaggccatcaatgccgccctgcagaaccacaaccaccagcagatcatcctggataagggcatgctggtggccatcgacgagctgatgcagagcctgaaccacaatggcgagaccctgaggcagaagcctcctgtgggcgaggccgatccctacagagtgaagatgaagctgtgtatcctgctgcacgccttttccacaagggtggtgaccatcaacagggtcatgggctacctgtccagcgccggcggcggcggcagcggaggaggaggctccgagccacgcggccccacaatcaagccatgccccccttgcaagtgtcctgcaccaaatctgctgggaggaccatccgtgttcatctttccacccaagatcaaggacgtgctgatgatcagcctgtccccaatcgtgacctgcgtggtcgtggccgtgagcgaggacgatcctgatgtgcagatctcctggttcgtgaacaatgtggaggtgcacaccgcccagacccagacacaccgggaggactacggctccacactgagagtggtgtctgccctgcccatccagcaccaggactggatgagcggcaaggagtttaagtgcaaggtgaacaataaggatctgcccgcccctatcgagcggacaatctctaagcctaagggcagcgtgagagccccacaggtgtatgtgctgcctccacccgaggaggagatgaccaagaagcaggtgacactgtcttgtgccgtgaccgacttcatgcctgaggatatctatgtggagtggaccaacaatggcaagacagagctgaactacaagaatacagagccagtgctggactccgatggctcttacttcatggtgagcaagctgagggtggagaagaagaactgggtggagcgcaattcttacagctgctccgtggtgcacgagggcctgcacaaccaccacaccacaaagtcttttagccggacccctggcaag

SEQ ID NO: 78 - DNA, 2292 bp, Artificial Sequence
  mu scIL-12 mut2-mu IgG2a Fc
atgtgggagctggagaaggacgtgtacgtggtggaggtggattggacacctgacgcccccggcgagacagtgaacctgacatgcgatacccctgaggaggatgatatcacatggacctccgatcagagacacggcgtgatcggcagcggcaagaccctgacaatcaccgtgaaggagtttctggatgccggccagtacacctgtcacaagggcggcgagacactgagccactcccacctgctgctgcacaagaaggagaatggcatctggtccaccgagatcctgaagaacttcaagaacaagaccttcctgaagtgtgaggcccctaattactccggcaggtttacatgctcctggctggtgcagagaaacatggacctgaagtttaatatcaagagctcctcctccagccccgatagcagagccgtgacctgtggcatggccagcctgagcgccgagaaggtgaccctggatcagagggattacgagaagtactccgtgtcctgtcaggaggatgtgacatgtcctacagccgaggagacactgcctatcgagctggccctggaggccaggcagcagaataagtacgagaactacagcacaagctttttcatcagggacatcatcaagcccgatccccccaagaacctgcagatgaagcccctgaagaacagccaggtggaggtgtcctgggagtaccctgatagctggtccacccctcactcctacttctccctgaagttctttgtgagaatccaggccgcggctgagaagatggccgagacagaggagggctgcaatcagaagggcgccttcctggtggagaagacatccaccgaggtgcagtgtaagggcggcaacgtgtgcgtgcaggcccaggacagatactacaattccagctgtagcaagtgggcctgtgtgccttgtagagtgagatccggcggcggcggctccggaggaggaggaagcggaggaggcggctccagagtgatccctgtgtccggccctgccagatgtctgtcccagagcagaaacctgctgaagaccacagacgacatggtgaagacagccagagagaagctgaagcactacagctgcaccgccgaggacatcgaccacgaggatatcacaagagaccagacatccaccctgaagacatgtctgcctctggagctgcacaagaatgagtcctgcctggccaccagagagacctccagcaccaccaggggcagctgcctgccccctcagaagacctccctgatgatgacactgtgcctgggcagcatctacgaggacctgaagatgtaccagaccgagttccaggccatcaatgccgccctgcagaaccacaaccaccagcagatcatcctggataagggcatgctggtggccatcgacgagctgatgcagagcctgaaccacaatggcgagaccctgaggcagaagcctcctgtgggcgaggccgatccctacagagtgaagatgaagctgtgtatcctgctgcacgccttttccacaagggtggtgaccatcaacagggtcatgggctacctgtccagcgccggcggcggcggcagcggaggaggaggctccgagccacgcggccccacaatcaagccatgccccccttgcaagtgtcctgcaccaaatctgctgggaggaccatccgtgttcatctttccacccaagatcaaggacgtgctgatgatcagcctgtccccaatcgtgacctgcgtggtcgtggacgtgagcgaggacgatcctgatgtgcagatctcctggttcgtgaacaatgtggaggtgcacaccgcccagacccagacacaccgggaggactacaactccacactgagagtggtgtctgccctgcccatccagcaccaggactggatgagcggcaaggagtttaagtgcaaggtgaacaataaggatctgcccgcccctatcgagcggacaatctctaagcctaagggcagcgtgagagccccacaggtgtatgtgctgcctccacccgaggaggagatgaccaagaagcaggtgacactgacttgtatggtgaccgacttcatgcctgaggatatctatgtggagtggaccaacaatggcaagacagagctgaactacaagaatacagagccagtgctggactccgatggctcttacttcatgtacagcaagctgagggtggagaagaagaactgggtggagcgcaattcttacagctgctccgtggtgcacgagggcctgcacaaccaccacaccacaaagtcttttagccggacccctggcaag

SEQ ID NO: 79 - DNA, 1344 bp, Artificial Sequence
  anti-mu FAP HC mu IgG2a Fc knob
caggtgcagctgcagcagtccggagcagagctggcaaggcctggagcctctgtgaacctgagctgcaaggcctccggctacaccttcacaaacaatggcatcaattggctgaagcagaggaccggacagggactggagtggatcggcgagatctacccaagatctaccaacacactgtataatgagaagttcaagggcaaggccaccctgacagcagaccggagctccaacaccgcctacatggagctgagaagcctgacatccgaggattctgccgtgtatttttgtgcacgcaccctgacagcacccttcgccttttggggacagggcaccctggtgacagtgagcgccgcaaagaccacagcaccaagcgtgtatccactggcacccgtgtgcggcgataccacaggctctagcgtgaccctgggctgtctggtgaagggctacttccctgagccagtgaccctgacatggaacagcggctctctgtcctctggcgtgcacacctttcctgccgtgctgcagtccgatctgtatacactgagctcctctgtgaccgtgacaagctccacctggcccagccagtccatcacatgcaacgtggcccaccctgcctctagcaccaaggtggacaagaagatcgagccacggggccccacaatcaagccatgtccaccttgcaagtgtccagcacctaatctgctgggaggacctagcgtgttcatctttccacccaagatcaaggacgtgctgatgatctctctgagccctatcgtgacctgcgtggtggtggacgtgtctgaggacgatccagatgtgcagatcagctggttcgtgaacaatgtggaggtgcacaccgcccagacccagacacaccgggaggactacaactccacactgagagtggtgtctgccctgcccatccagcaccaggactggatgtccggcaaggagtttaagtgcaaggtgaacaataaggatctgccagcccccatcgagaggaccatctctaagcctaagggcagcgtgcgcgcaccacaggtgtatgtgctgcctccacccgaggaggagatgaccaagaagcaggtgacactgtggtgtatggtgaccgacttcatgccagaggatatctacgtggagtggaccaacaatggcaagacagagctgaactataagaatacagagcccgtgctggacagcgatggctcctactttatgtatagcaagctgagggtggagaagaagaactgggtggagcgcaattcctactcttgtagcgtggtgcacgagggcctgcacaaccaccacaccacaaagtccttttctagaacccccggcaagtga

SEQ ID NO: 80 - DNA, 639 bp, Artificial Sequence
  anti-mu FAP LC
cagatcgtgctgacacagtcccctgccatcatgtctgccagcccaggcgagaaggtgaccatgacatgctctgccagctccggcgtgaacttcatgcactggtaccagcagaagtctggcacaagccccaagcggtggatcttcgacacctccaagctggcctctggcgtgcctgccagattttccggctctggcagcggcacatcctattctctgaccatctctagcatggaggccgaggacgccgccacctactattgccagcagtggagcttcaatccccctacatttggcggcggcaccaagctggagatcaagagggcagatgcagcaccaacagtgtccatctttccaccctcctctgagcagctgaccagcggaggagcatccgtggtgtgcttcctgaacaacttctaccccaaggacatcaacgtgaagtggaagatcgatggctctgagaggcagaacggcgtgctgaatagctggacagaccaggattccaaggactctacctatagcatgagctccaccctgacactgaccaaggatgagtacgagaggcacaatagctatacatgcgaggccacccacaagacaagcacctcccctatcgtgaagtccttcaaccgcaatgagtgt

SEQ ID NO: 81 - DNA, 1341 bp, Artificial Sequence
  anti-mu FAP HC mu IgG2a Fc knob DANG
caggtgcagctgcagcagtccggagcagagctggcaaggcctggagcctctgtgaacctgagctgcaaggcctccggctacaccttcacaaacaatggcatcaattggctgaagcagaggaccggacagggactggagtggatcggcgagatctacccaagatctaccaacacactgtataatgagaagttcaagggcaaggccaccctgacagcagaccggagctccaacaccgcctacatggagctgagaagcctgacatccgaggattctgccgtgtatttttgtgcacgcaccctgacagcacccttcgccttttggggacagggcaccctggtgacagtgagcgccgccaagaccacagcaccaagcgtgtatccactggcacccgtgtgcggcgataccacaggctctagcgtgaccctgggctgtctggtgaagggctacttccctgagccagtgaccctgacatggaacagcggctctctgtcctctggcgtgcacacctttcctgccgtgctgcagtccgatctgtatacactgagctcctctgtgaccgtgacaagctccacctggcccagccagtccatcacatgcaacgtggcccaccctgcctctagcaccaaggtggacaagaagatcgagccacggggccccacaatcaagccatgtccaccttgcaagtgtccagcacctaatctgctgggaggacctagcgtgttcatctttccacccaagatcaaggacgtgctgatgatctctctgagccctatcgtgacctgcgtggtggtggccgtgtctgaggacgatccagatgtgcagatcagctggttcgtgaacaatgtggaggtgcacaccgcccagacccagacacaccgggaggactacggctccacactgagagtggtgtctgccctgcccatccagcaccaggactggatgtccggcaaggagtttaagtgcaaggtgaacaataaggatctgccagcccccatcgagaggaccatctctaagcctaagggcagcgtgcgcgcaccacaggtgtatgtgctgcctccacccgaggaggagatgaccaagaagcaggtgacactgtggtgtatggtgaccgacttcatgccagaggatatctacgtggagtggaccaacaatggcaagacagagctgaactataagaatacagagcccgtgctggacagcgatggctcctactttatgtatagcaagctgagggtggagaagaagaactgggtggagcgcaattcctactcttgtagcgtggtgcacgagggcctgcacaaccaccacaccacaaagtccttttctagaacccccggcaag

SEQ ID NO: 82 - DNA, 699 bp, Artificial Sequence
  mu IgG2a Fc knob DANG
gagccaaggggccccaccatcaagccatgccccccttgcaagtgtcctgcaccaaacctgctgggaggaccaagcgtgttcatctttccacccaagatcaaggacgtgctgatgatcagcctgtcccccatcgtgacatgcgtggtggtggccgtgtccgaggacgatcctgatgtgcagatctcttggttcgtgaacaatgtggaggtgcacaccgcccagacccagacacaccgggaggactacggctctacactgagagtggtgagcgccctgcccatccagcaccaggactggatgtccggcaaggagtttaagtgcaaggtgaacaataaggatctgcccgcccctatcgagcggaccatcagcaagcctaagggctccgtgagagccccacaggtgtatgtgctgcctccacccgaggaggagatgaccaagaagcaggtgacactgtggtgtatggtgaccgacttcatgcctgaggatatctacgtggagtggaccaacaatggcaagacagagctgaactataagaatacagagccagtgctggactccgatggctcttactttatgtattctaagctgagggtggagaagaagaactgggtggagcgcaattcttacagctgctccgtggtgcacgagggcctgcacaatcaccacaccacaaagtctttcagcagaacccctggcaag

SEQ ID NO: 83 - DNA, 699 bp, Artificial Sequence
  mu IgG2a Fc hole DANG
gagccaaggggccccaccatcaagccatgccccccttgcaagtgtcctgcaccaaacctgctgggaggaccaagcgtgttcatctttccacccaagatcaaggacgtgctgatgatcagcctgtcccccatcgtgacatgcgtggtggtggccgtgtccgaggacgatcctgatgtgcagatctcttggttcgtgaacaatgtggaggtgcacaccgcccagacccagacacaccgggaggactatggctctacactgagagtggtgagcgccctgcccatccagcaccaggactggatgagcggcaaggagtttaagtgcaaggtgaacaataaggatctgcccgcccctatcgagcggaccatcagcaagcctaagggctccgtgagagccccacaggtgtacgtgctgcctccacccgaggaggagatgaccaagaagcaggtgacactgagctgtgccgtgaccgacttcatgcctgaggatatctacgtggagtggaccaacaatggcaagacagagctgaactataagaatacagagccagtgctggactccgatggctcttactttatggtgtccaagctgagggtggagaagaagaactgggtggagcgcaattcttatagctgctccgtggtgcacgagggcctgcacaatcaccacaccacaaagtctttcagcagaacccctggcaag

SEQ ID NO: 84 - DNA, 1353 bp, Artificial Sequence
  anti-mu CD20 (18B12) HC
caggtgcagctgcagcagccaggagcagagctggtgaggccaggcacctctgtgaagctgagctgcaaggcctccggctacaccttcacatcttattggatgcactggatcaagcagaggccaggacagggactggagtggatcggcgtgatcgacccctccgataactacaccaagtacaaccagaagtttaagggcaaggccaccctgacagtggacaccagctcctctacagcctacatgcagctgagctccctgacatccgaggattctgccgtgtatttctgtgcccgggagggctactatggctctagcccatggtttgcctactggggccagggcaccctggtgacagtgtcctctgccaagaccacagcccccagcgtgtatcctctggccccagtgtgcggcgataccacaggcagctccgtgaccctgggctgtctggtgaagggctacttccctgagccagtgaccctgacatggaactctggcagcctgtctagcggagtgcacacctttccagccgtgctgcagtccgatctgtatacactgtcctctagcgtgaccgtgacatcctctacctggccctcccagtctatcacatgcaacgtggcccaccctgccagctccaccaaggtggacaagaagatcgagccccggggccctacaatcaagccatgtccaccttgcaagtgtccagcacctaatctgctgggaggacctagcgtgttcatctttccacccaagatcaaggacgtgctgatgatcagcctgtcccctatcgtgacctgcgtggtggtggacgtgagcgaggacgatccagatgtgcagatctcctggttcgtgaacaatgtggaggtgcacaccgcccagacccagacacaccgggaggactacaactccacactgagagtggtgtctgccctgcctatccagcaccaggactggatgtccggcaaggagtttaagtgcaaggtgaacaataaggatctgccagcccccatcgagcggaccatctctaagcctaagggcagcgtgagagccccacaggtgtatgtgctgcctccacccgaggaggagatgaccaagaagcaggtgacactgacctgtatggtgaccgacttcatgcctgaggatatctacgtggagtggaccaacaatggcaagacagagctgaactataagaatacagagccagtgctggacagcgatggctcctactttatgtatagcaagctgagggtggagaagaagaactgggtggagcgcaattcttacagctgttccgtggtgcacgagggcctgcacaatcaccacaccacaaagtctttcagcagaacccccggcaag

SEQ ID NO: 85 - protein, 219 aa, Artificial Sequence
  anti-hu CD20 HC
QVQLQQPGAELVKPGASVKMSCKASGYTFTSYNMHWVKQTPGRGLEWIGAIYPGNGDTSYNQKFKGKATLTADKSSSTAYMQLSSLTSEDSAVYYCARSTYYGGDWYFNVWGAGTTVTVSAASTKGPSVFPLAPSSKSTSGGTAALGCLVKDYFPEPVTVSWNSGALTSGVHTFPAVLQSSGLYSLSSVVTVPSSSLGTQTYICNVNHKPSNTKVDKKV

SEQ ID NO: 86 - protein, 217 aa, Artificial Sequence
  mu IgG2a Fc DANG
APNLLGGPSVFIFPPKIKDVLMISLSPIVTCVVVAVSEDDPDVQISWFVNNVEVHTAQTQTHREDYGSTLRVVSALPIQHQDWMSGKEFKCKVNNKDLPAPIERTISKPKGSVRAPQVYVLPPPEEEMTKKQVTLTCMVTDFMPEDIYVEWTNNGKTELNYKNTEPVLDSDGSYFMYSKLRVEKKNWVERNSYSCSVVHEGLHNHHTTKSFSRTPGK

SEQ ID NO: 87 - protein, 209 aa, Artificial Sequence
  hu IgG1 Fc DANG
SVFLFPPKPKDTLMISRTPEVTCVVVAVSHEDPEVKFNWYVDGVEVHNAKTKPREEQYGSTYRVVSVLTVLHQDWLNGKEYKCKVSNKALPAPIEKTISKAKGQPREPQVYTLPPSRDELTKNQVSLTCLVKGFYPSDIAVEWESNGQPENNYKTTPPVLDSDGSFFLYSKLTVDKSRWQQGNVFSCSVMHEALHNHYTQKSLSLSPGK

SEQ ID NO: 88 - protein, 247 aa, Artificial Sequence
  anti-hu CD20 scFv
QVQLQQPGAELVKPGASVKMSCKASGYTFTSYNMHWVKQTPGRGLEWIGAIYPGNGDTSYNQKFKGKATLTADKSSSTAYMQLSSLTSEDSAVYYCARSTYYGGDWYFNVWGAGTTVTVSAGGGGSGGGGSGGGGSGGGGSQIVLSQSPAILSASPGEKVTMTCRASSSVSYIHWFQQKPGSSPKPWIYATSNLASGVPVRFSGSGSGTSYSLTISRVEAEDAATYYCQQWTSNPPTFGGGTKLEIK

SEQ ID NO: 89 - protein, 247 aa, Artificial Sequence
  anti-mu CD20 scFv
QVQLQQPGAELVRPGTSVKLSCKASGYTFTSYWMHWIKQRPGQGLEWIGVIDPSDNYTKYNQKFKGKATLTVDTSSSTAYMQLSSLTSEDSAVYFCAREGYYGSSPWFAYWGQGTLVTVSSGGGGSGGGGSGGGGSGGGGSQIVMSQSPAILSASPGEKVTMTCRARSSVSYIHWYQQKPGSSPKPWIYATSNLASGVPGRFSGSGSGTSYSLTITRVEAEDAATYYCQQWSSKPPTFGGGTKLEIK

SEQ ID NO: 90 - protein, 218 aa, Artificial Sequence
  anti-mu CD20 HC
QVQLQQPGAELVRPGTSVKLSCKASGYTFTSYWMHWIKQRPGQGLEWIGVIDPSDNYTKYNQKFKGKATLTVDTSSSTAYMQLSSLTSEDSAVYFCAREGYYGSSPWFAYWGQGTLVTVSSAKTTAPSVYPLAPVCGDTTGSSVTLGCLVKGYFPEPVTLTWNSGSLSSGVHTFPAVLQSDLYTLSSSVTVTSSTWPSQSITCNVAHPASSTKVDKKI

SEQ ID NO: 91 - protein, 10 aa, Artificial Sequence
  linker 1
GGGGSGGGGS

SEQ ID NO: 92 - protein, 15 aa, Artificial Sequence
  linker 2
GGGGSGGGGSGGGGS

SEQ ID NO: 93 - protein, 20 aa, Artificial Sequence
  linker 3
GGGGSGGGGSGGGGSGGGGS

SEQ ID NO: 94 - protein, 23 aa, Artificial Sequence
  hu IgG1 Hinge
EPKSCDKTHTCPPCPAPELLGGP

SEQ ID NO: 95 - protein, 14 aa, Artificial Sequence
  hu IgG1 Hinge-core 1
EPKSCDKTHTCPPC

SEQ ID NO: 96 - protein, 9 aa, Artificial Sequence
  hu IgG1 Hinge-core 2
DKTHTCPPC

SEQ ID NO: 97 - protein, 11 aa, Artificial Sequence
  hu IgG1 Hinge-core 3
CDKTHTCPPCP

SEQ ID NO: 98 - protein, 5 aa, Artificial Sequence
  hu IgG1 Hinge-core 4
CPPCP

SEQ ID NO: 99 - protein, 4 aa, Artificial Sequence
  hu IgG1 Hinge-core 5
CPPC

SEQ ID NO: 100 - protein, 28 aa, Artificial Sequence
  hu IgG1 Hinge Linker
GGGGSGGGGSDKTHTCPPCPAPELLGGP

SEQ ID NO: 101 - protein, 16 aa, Artificial Sequence
  mu IgG2a Hinge
EPRGPTIKPCPPCKCP

SEQ ID NO: 102 - protein, 26 aa, Artificial Sequence
  mu IgG2a Hinge Linker
GGGGSGGGGSEPRGPTIKPCPPCKCP

SEQ ID NO: 103 - protein, 227 aa, Artificial Sequence [sequence omitted]

SEQ ID NO: 104 - protein, 227 aa, Artificial Sequence
  hu IgG1 Fc hole
DKTHTCPPCPAPELLGGPSVFLFPPKPKDTLMISRTPEVTCVVVDVSHEDPEVKFNWYVDGVEVHNAKTKPREEQYNSTYRVVSVLTVLHQDWLNGKEYKCKVSNKALPAPIEKTISKAKGQPREPQVYTLPPSRDELTKNQVSLSCAVKGFYPSDIAVEWESNGQPENNYKTTPPVLDSDGSFFLVSKLTVDKSRWQQGNVFSCSVMHEALHNHYTQKSLSLSPGK

SEQ ID NO: 105 - protein, 233 aa, Artificial Sequence
  mu IgG2a Fc knob
EPRGPTIKPCPPCKCPAPNLLGGPSVFIFPPKIKDVLMISLSPIVTCVVVDVSEDDPDVQISWFVNNVEVHTAQTQTHREDYNSTLRVVSALPIQHQDWMSGKEFKCKVNNKDLPAPIERTISKPKGSVRAPQVYVLPPPEEEMTKKQVTLWCMVTDFMPEDIYVEWTNNGKTELNYKNTEPVLDSDGSYFMYSKLRVEKKNWVERNSYSCSVVHEGLHNHHTTKSFSRTPGK

SEQ ID NO: 106 - protein, 233 aa, Artificial Sequence
  mu IgG2a Fc hole
EPRGPTIKPCPPCKCPAPNLLGGPSVFIFPPKIKDVLMISLSPIVTCVVVDVSEDDPDVQISWFVNNVEVHTAQTQTHREDYNSTLRVVSALPIQHQDWMSGKEFKCKVNNKDLPAPIERTISKPKGSVRAPQVYVLPPPEEEMTKKQVTLSCAVTDFMPEDIYVEWTNNGKTELNYKNTEPVLDSDGSYFMVSKLRVEKKNWVERNSYSCSVVHEGLHNHHTTKSFSRTPGK

SEQ ID NO: 107 - protein, 5 aa, Artificial Sequence
  anti-hu CD20 HCDR1
SYNMH

SEQ ID NO: 108 - protein, 17 aa, Artificial Sequence
  anti-hu CD20 HCDR2
AIYPGNGDTSYNQKFKG

SEQ ID NO: 109 - protein, 12 aa, Artificial Sequence
  anti-hu CD20 HCDR3
STYYGGDWYFNV

SEQ ID NO: 110 - protein, 10 aa, Artificial Sequence
  anti-hu CD20 LCDR1
RASSSVSYIH

SEQ ID NO: 111 - protein, 7 aa, Artificial Sequence
  anti-hu CD20 LCDR2
ATSNLAS

SEQ ID NO: 112 - protein, 9 aa, Artificial Sequence
  anti-hu CD20 LCDR3
QQWTSNPPT

SEQ ID NO: 113 - protein, 121 aa, Artificial Sequence [sequence omitted]

SEQ ID NO: 114 - protein, 106 aa, Artificial Sequence [sequence omitted]

SEQ ID NO: 115 - protein, 5 aa, Artificial Sequence
  anti-mu CD20 HCDR1
SYWMH

SEQ ID NO: 116 - protein, 17 aa, Artificial Sequence
  anti-mu CD20 HCDR2
VIDPSDNYTKYNQKFKG

SEQ ID NO: 117 - protein, 12 aa, Artificial Sequence
  anti-mu CD20 HCDR3
EGYYGSSPWFAY

SEQ ID NO: 118 - protein, 10 aa, Artificial Sequence
  anti-mu CD20 LCDR1
RARSSVSYIH

SEQ ID NO: 119 - protein, 7 aa, Artificial Sequence
  anti-mu CD20 LCDR2
ATSNLAS

SEQ ID NO: 120 - protein, 9 aa, Artificial Sequence
  anti-mu CD20 LCDR3
QQWSSKPPT

SEQ ID NO: 121 - protein, 121 aa, Artificial Sequence
  anti-mu CD20 HCVR
QVQLQQPGAELVRPGTSVKLSCKASGYTFTSYWMHWIKQRPGQGLEWIGVIDPSDNYTKYNQKFKGKATLTVDTSSSTAYMQLSSLTSEDSAVYFCAREGYYGSSPWFAYWGQGTLVTVSS

SEQ ID NO: 122 - protein, 106 aa, Artificial Sequence
  anti-mu CD20 LCVR
QIVMSQSPAILSASPGEKVTMTCRARSSVSYIHWYQQKPGSSPKPWIYATSNLASGVPGRFSGSGSGTSYSLTITRVEAEDAATYYCQQWSSKPPTFGGGTKLEIK

SEQ ID NO: 123 - protein, 518 aa, Artificial Sequence
  hu scIL-12
IWELKKDVYVVELDWYPDAPGEMVVLTCDTPEEDGITWTLDQSSEVLGSGKTLTIQVKEFGDAGQYTCHKGGEVLSHSLLLLHKKEDGIWSTDILKDQKEPKNKTFLRCEAKNYSGRFTCWWLTTISTDLTFSVKSSRGSSDPQGVTCGAATLSAERVRGDNKEYEYSVECQEDSACPAAEESLPIEVMVDAVHKLKYENYTSSFFIRDIIKPDPPKNLQLKPLKNSRQVEVSWEYPDTWSTPHSYFSLTFCVQVQGKSKREKKDRVFTDKTSATVICRKNASISVRAQDRYYSSSWSEWASVPCSGGGGSGGGGSGGGGSRNLPVATPDPGMFPCLHHSQNLLRAVSNMLQKARQTLEFYPCTSEEIDHEDITKDKTSTVEACLPLELTKNESCLNSRETSFITNGSCLASRKTSFMMALCLSSIYEDLKMYQVEFKTMNAKLLMDPKRQIFLDQNMLAVIDELMQALNFNSETVPQKSSLEEPDFYKTKIKLCILLHAFRIRAVTIDRVMSYLNAS

SEQ ID NO: 124 - protein, 306 aa, Artificial Sequence
  hu scIL-12 p40
IWELKKDVYVVELDWYPDAPGEMVVLTCDTPEEDGITWTLDQSSEVLGSGKTLTIQVKEFGDAGQYTCHKGGEVLSHSLLLLHKKEDGIWSTDILKDQKEPKNKTFLRCEAKNYSGRFTCWWLTTISTDLTFSVKSSRGSSDPQGVTCGAATLSAERVRGDNKEYEYSVECQEDSACPAAEESLPIEVMVDAVHKLKYENYTSSFFIRDIIKPDPPKNLQLKPLKNSRQVEVSWEYPDTWSTPHSYFSLTFCVQVQGKSKREKKDRVFTDKTSATVICRKNASISVRAQDRYYSSSWSEWASVPCS

SEQ ID NO: 125 - protein, 197 aa, Artificial Sequence
  hu scIL-12 p35
RNLPVATPDPGMFPCLHHSQNLLRAVSNMLQKARQTLEFYPCTSEEIDHEDITKDKTSTVEACLPLELTKNESCLNSRETSFITNGSCLASRKTSFMMALCLSSIYEDLKMYQVEFKTMNAKLLMDPKRQIFLDQNMLAVIDELMQALNFNSETVPQKSSLEEPDFYKTKIKLCILLHAFRIRAVTIDRVMSYLNAS

SEQ ID NO: 126 - protein, 518 aa, Artificial Sequence
  hu scIL-12 mut1
IWELKKDVYVVELDWYPDAPGEMVVLTCDTPEEDGITWTLDQSSEVLGSGKTLTIQVKEFGDAGQYTCHKGGEVLSHSLLLLHKKEDGIWSTDILKDQKEPKNKTFLRCEAKNYSGRFTCWWLTTISTDLTFSVKSSRGSSDPQGVTCGAATLSAERVRGDNKEYEYSVECQEDSACPAAEESLPIEVMVDAVHKLKYENYTSSFFIRDIIKPDPPKNLQLKPLKNSRQVEVSWEYPDTWSTPHSYFSLTFCVQVQGASKREAKDRVFTDKTSATVICRKNASISVRAQDRYYSSSWSEWASVPCSGGGGSGGGGSGGGGSRNLPVATPDPGMFPCLHHSQNLLRAVSNMLQKARQTLEFYPCTSEEIDHEDITKDKTSTVEACLPLELTKNESCLNSRETSFITNGSCLASRKTSFMMALCLSSIYEDLKMYQVEFKTMNAKLLMDPKRQIFLDQNMLAVIDELMQALNFNSETVPQKSSLEEPDFYKTKIKLCILLHAFRIRAVTIDRVMSYLNAS

SEQ ID NO: 127 - protein, 306 aa, Artificial Sequence
  hu scIL-12 mut1 p40
IWELKKDVYVVELDWYPDAPGEMVVLTCDTPEEDGITWTLDQSSEVLGSGKTLTIQVKEFGDAGQYTCHKGGEVLSHSLLLLHKKEDGIWSTDILKDQKEPKNKTFLRCEAKNYSGRFTCWWLTTISTDLTFSVKSSRGSSDPQGVTCGAATLSAERVRGDNKEYEYSVECQEDSACPAAEESLPIEVMVDAVHKLKYENYTSSFFIRDIIKPDPPKNLQLKPLKNSRQVEVSWEYPDTWSTPHSYFSLTFCVQVQGASKREAKDRVFTDKTSATVICRKNASISVRAQDRYYSSSWSEWASVPCS

SEQ ID NO: 128 - protein, 518 aa, Artificial Sequence
  hu scIL-12 mut2
IWELKKDVYVVELDWYPDAPGEMVVLTCDTPEEDGITWTLDQSSEVLGSGKTLTIQVKEFGDAGQYTCHKGGEVLSHSLLLLHKKEDGIWSTDILKDQKEPKNKTFLRCEAKNYSGRFTCWWLTTISTDLTFSVKSSRGSSDPQGVTCGAATLSAERVRGDNKEYEYSVECQEDSACPAAEESLPIEVMVDAVHKLKYENYTSSFFIRDIIKPDPPKNLQLKPLKNSRQVEVSWEYPDTWSTPHSYFSLTFCVQVQGASAREAADRVFTDKTSATVICRKNASISVRAQDRYYSSSWSEWASVPCSGGGGSGGGGSGGGGSRNLPVATPDPGMFPCLHHSQNLLRAVSNMLQKARQTLEFYPCTSEEIDHEDITKDKTSTVEACLPLELTKNESCLNSRETSFITNGSCLASRKTSFMMALCLSSIYEDLKMYQVEFKTMNAKLLMDPKRQIFLDQNMLAVIDELMQALNFNSETVPQKSSLEEPDFYKTKIKLCILLHAFRIRAVTIDRVMSYLNAS

SEQ ID NO: 129 - protein, 306 aa, Artificial Sequence
  hu scIL-12 mut2 p40
IWELKKDVYVVELDWYPDAPGEMVVLTCDTPEEDGITWTLDQSSEVLGSGKTLTIQVKEFGDAGQYTCHKGGEVLSHSLLLLHKKEDGIWSTDILKDQKEPKNKTFLRCEAKNYSGRFTCWWLTTISTDLTFSVKSSRGSSDPQGVTCGAATLSAERVRGDNKEYEYSVECQEDSACPAAEESLPIEVMVDAVHKLKYENYTSSFFIRDIIKPDPPKNLQLKPLKNSRQVEVSWEYPDTWSTPHSYFSLTFCVQVQGASAREAADRVFTDKTSATVICRKNASISVRAQDRYYSSSWSEWASVPCS

SEQ ID NO: 130 - protein, 521 aa, Artificial Sequence
  mu scIL-12
MWELEKDVYVVEVDWTPDAPGETVNLTCDTPEEDDITWTSDQRHGVIGSGKTLTITVKEFLDAGQYTCHKGGETLSHSHLLLHKKENGIWSTEILKNFKNKTFLKCEAPNYSGRFTCSWLVQRNMDLKFNIKSSSSSPDSRAVTCGMASLSAEKVTLDQRDYEKYSVSCQEDVTCPTAEETLPIELALEARQQNKYENYSTSFFIRDIIKPDPPKNLQMKPLKNSQVEVSWEYPDSWSTPHSYFSLKFFVRIQRKKEKMKETEEGCNQKGAFLVEKTSTEVQCKGGNVCVQAQDRYYNSSCSKWACVPCRVRSGGGGSGGGGSGGGGSRVIPVSGPARCLSQSRNLLKTTDDMVKTAREKLKHYSCTAEDIDHEDITRDQTSTLKTCLPLELHKNESCLATRETSSTTRGSCLPPQKTSLMMTLCLGSIYEDLKMYQTEFQAINAALQNHNHQQIILDKGMLVAIDELMQSLNHNGETLRQKPPVGEADPYRVKMKLCILLHAFSTRVVTINRVMGYLSSA

SEQ ID NO: 131 - protein, 313 aa, Artificial Sequence
  mu scIL-12 p40
MWELEKDVYVVEVDWTPDAPGETVNLTCDTPEEDDITWTSDQRHGVIGSGKTLTITVKEFLDAGQYTCHKGGETLSHSHLLLHKKENGIWSTEILKNFKNKTFLKCEAPNYSGRFTCSWLVQRNMDLKFNIKSSSSSPDSRAVTCGMASLSAEKVTLDQRDYEKYSVSCQEDVTCPTAEETLPIELALEARQQNKYENYSTSFFIRDIIKPDPPKNLQMKPLKNSQVEVSWEYPDSWSTPHSYFSLKFFVRIQRKKEKMKETEEGCNQKGAFLVEKTSTEVQCKGGNVCVQAQDRYYNSSCSKWACVPCRVRS

SEQ ID NO: 132 - protein, 193 aa, Artificial Sequence
  mu scIL-12 p35
RVIPVSGPARCLSQSRNLLKTTDDMVKTAREKLKHYSCTAEDIDHEDITRDQTSTLKTCLPLELHKNESCLATRETSSTTRGSCLPPQKTSLMMTLCLGSIYEDLKMYQTEFQAINAALQNHNHQQIILDKGMLVAIDELMQSLNHNGETLRQKPPVGEADPYRVKMKLCILLHAFSTRVVTINRVMGYLSSA

SEQ ID NO: 133 - protein, 521 aa, Artificial Sequence
  mu scIL-12 mut1
MWELEKDVYVVEVDWTPDAPGETVNLTCDTPEEDDITWTSDQRHGVIGSGKTLTITVKEFLDAGQYTCHKGGETLSHSHLLLHKKENGIWSTEILKNFKNKTFLKCEAPNYSGRFTCSWLVQRNMDLKFNIKSSSSSPDSRAVTCGMASLSAEKVTLDQRDYEKYSVSCQEDVTCPTAEETLPIELALEARQQNKYENYSTSFFIRDIIKPDPPKNLQMKPLKNSQVEVSWEYPDSWSTPHSYFSLKFFVRIQRAKEKMAETEEGCNQKGAFLVEKTSTEVQCKGGNVCVQAQDRYYNSSCSKWACVPCRVRSGGGGSGGGGSGGGGSRVIPVSGPARCLSQSRNLLKTTDDMVKTAREKLKHYSCTAEDIDHEDITRDQTSTLKTCLPLELHKNESCLATRETSSTTRGSCLPPQKTSLMMTLCLGSIYEDLKMYQTEFQAINAALQNHNHQQIILDKGMLVAIDELMQSLNHNGETLRQKPPVGEADPYRVKMKLCILLHAFSTRVVTINRVMGYLSSA

SEQ ID NO: 134 - protein, 313 aa, Artificial Sequence
  mu scIL-12 mut1 p40
MWELEKDVYVVEVDWTPDAPGETVNLTCDTPEEDDITWTSDQRHGVIGSGKTLTITVKEFLDAGQYTCHKGGETLSHSHLLLHKKENGIWSTEILKNFKNKTFLKCEAPNYSGRFTCSWLVQRNMDLKFNIKSSSSSPDSRAVTCGMASLSAEKVTLDQRDYEKYSVSCQEDVTCPTAEETLPIELALEARQQNKYENYSTSFFIRDIIKPDPPKNLQMKPLKNSQVEVSWEYPDSWSTPHSYFSLKFFVRIQRAKEKMAETEEGCNQKGAFLVEKTSTEVQCKGGNVCVQAQDRYYNSSCSKWACVPCRVRS

SEQ ID NO: 135 - protein, 521 aa, Artificial Sequence
  mu scIL-12 mut2
MWELEKDVYVVEVDWTPDAPGETVNLTCDTPEEDDITWTSDQRHGVIGSGKTLTITVKEFLDAGQYTCHKGGETLSHSHLLLHKKENGIWSTEILKNFKNKTFLKCEAPNYSGRFTCSWLVQRNMDLKFNIKSSSSSPDSRAVTCGMASLSAEKVTLDQRDYEKYSVSCQEDVTCPTAEETLPIELALEARQQNKYENYSTSFFIRDIIKPDPPKNLQMKPLKNSQVEVSWEYPDSWSTPHSYFSLKFFVRIQAAAEKMAETEEGCNQKGAFLVEKTSTEVQCKGGNVCVQAQDRYYNSSCSKWACVPCRVRSGGGGSGGGGSGGGGSRVIPVSGPARCLSQSRNLLKTTDDMVKTAREKLKHYSCTAEDIDHEDITRDQTSTLKTCLPLELHKNESCLATRETSSTTRGSCLPPQKTSLMMTLCLGSIYEDLKMYQTEFQAINAALQNHNHQQIILDKGMLVAIDELMQSLNHNGETLRQKPPVGEADPYRVKMKLCILLHAFSTRVVTINRVMGYLSSA

SEQ ID NO: 136 - protein, 313 aa, Artificial Sequence
  mu scIL-12 mut2 p40
MWELEKDVYVVEVDWTPDAPGETVNLTCDTPEEDDITWTSDQRHGVIGSGKTLTITVKEFLDAGQYTCHKGGETLSHSHLLLHKKENGIWSTEILKNFKNKTFLKCEAPNYSGRFTCSWLVQRNMDLKFNIKSSSSSPDSRAVTCGMASLSAEKVTLDQRDYEKYSVSCQEDVTCPTAEETLPIELALEARQQNKYENYSTSFFIRDIIKPDPPKNLQMKPLKNSQVEVSWEYPDSWSTPHSYFSLKFFVRIQAAAEKMAETEEGCNQKGAFLVEKTSTEVQCKGGNVCVQAQDRYYNSSCSKWACVPCRVRS

SEQ ID NO: 137 - protein, 328 aa, Artificial Sequence
  hu IL-12 p40 wt_AAD56386
MCHQQLVISWFSLVFLASPLVAIWELKKDVYVVELDWYPDAPGEMVVLTCDTPEEDGITWTLDQSSEVLGSGKTLTIQVKEFGDAGQYTCHKGGEVLSHSLLLLHKKEDGIWSTDILKDQKEPKNKTFLRCEAKNYSGRFTCWWLTTISTDLTFSVKSSRGSSDPQGVTCGAATLSAERVRGDNKEYEYSVECQEDSACPAAEESLPIEVMVDAVHKLKYENYTSSFFIRDIIKPDPPKNLQLKPLKNSRQVEVSWEYPDTWSTPHSYFSLTFCVQVQGKSKREKKDRVFTDKTSATVICRKNASISVRAQDRYYSSSWSEWASVPCS

SEQ ID NO: 138 - protein, 219 aa, Artificial Sequence
  hu IL-12 p35 wt_AAK84425
MCPARSLLLVATLVLLDHLSLARNLPVATPDPGMFPCLHHSQNLLRAVSNMLQKARQTLEFYPCTSEEIDHEDITKDKTSTVEACLPLELTKNESCLNSRETSFITNGSCLASRKTSFMMALCLSSIYEDLKMYQVEFKTMNAKLLMDPKRQIFLDQNMLAVIDELMQALNFNSETVPQKSSLEEPDFYKTKIKLCILLHAFRIRAVTIDRVMSYLNAS

SEQ ID NO: 139 - protein, 335 aa, Artificial Sequence
  mu IL-12 p40 wt_AAA39296
MCPQKLTISWFAIVLLVSPLMAMWELEKDVYVVEVDWTPDAPGETVNLTCDTPEEDDITWTSDQRHGVIGSGKTLTITVKEFLDAGQYTCHKGGETLSHSHLLLHKKENGIWSTEILKNFKNKTFLKCEAPNYSGRFTCSWLVQRNMDLKFNIKSSSSSPDSRAVTCGMASLSAEKVTLDQRDYEKYSVSCQEDVTCPTAEETLPIELALEARQQNKYENYSTSFFIRDIIKPDPPKNLQMKPLKNSQVEVSWEYPDSWSTPHSYFSLKFFVRIQRKKEKMKETEEGCNQKGAFLVEKTSTEVQCKGGNVCVQAQDRYYNSSCSKWACVPCRVRS

SEQ ID NO: 140 - protein, 215 aa, Artificial Sequence
  mu IL-12 p35 wt_AAK39292
MCQSRYLLFLATLALLNHLSLARVIPVSGPARCLSQSRNLLKTTDDMVKTAREKLKHYSCTAEDIDHEDITRDQTSTLKTCLPLELHKNESCLATRETSSTTRGSCLPPQKTSLMMTLCLGSIYEDLKMYQTEFQAINAALQNHNHQQIILDKGMLVAIDELMQSLNHNGETLRQKPPVGEADPYRVKMKLCILLHAFSTRVVTINRVMGYLSSA

SEQ ID NO: 141 - protein, 252 aa, Artificial Sequence
  hu IL-12 p40_X1
IWELKKDVYVVELDWYPDAPGEMVVLTCDTPEEDGITWTLDQSSEVLGSGKTLTIQVKEFGDAGQYTCHKGGEVLSHSLLLLHKKEDGIWSTDILKDQKEPKNKTFLRCEAKNYSGRFTCWWLTTISTDLTFSVKSSRGSSDPQGVTCGAATLSAERVRGDNKEYEYSVECQEDSACPAAEESLPIEVMVDAVHKLKYENYTSSFFIRDIIKPDPPKNLQLKPLKNSRQVEVSWEYPDTWSTPHSYFSLTFC

SEQ ID NO: 142 - protein, 42 aa, Artificial Sequence
  hu IL-12 p40_X2
DRVFTDKTSATVICRKNASISVRAQDRYYSSSWSEWASVPCS

SEQ ID NO: 143 - protein, 10 aa, Artificial Sequence
  Ocrelizumab HCDR1
GYTFTSYNMH

SEQ ID NO: 144 - protein, 17 aa, Artificial Sequence
  Ocrelizumab HCDR2
AIYPGNGDTSYNQKFKG

SEQ ID NO: 145 - protein, 13 aa, Artificial Sequence
  Ocrelizumab HCDR3
VVYYSNSYWYFDV

SEQ ID NO: 146 - protein, 10 aa, Artificial Sequence
  Ocrelizumab LCDR1
RASSSVSYMH

SEQ ID NO: 147 - protein, 7 aa, Artificial Sequence
  Ocrelizumab LCDR2
APSNLAS

SEQ ID NO: 148 - protein, 9 aa, Artificial Sequence
  Ocrelizumab LCDR3
QQWSFNPPT

SEQ ID NO: 149 - protein, 5 aa, Artificial Sequence
  RG-7159 HCDR1
YSWIN

SEQ ID NO: 150 - protein, 17 aa, Artificial Sequence
  RG-7159 HCDR2
RIFPGDGDTDYNGKFKG

SEQ ID NO: 151 - protein, 10 aa, Artificial Sequence
  RG-7159 HCDR3
NVFDGYWLVY

SEQ ID NO: 152 - protein, 16 aa, Artificial Sequence
  RG-7159 LCDR1
RSSKSLLHSNGITYLY

SEQ ID NO: 153 - protein, 7 aa, Artificial Sequence
  RG-7159 LCDR2
QMSNLVS

SEQ ID NO: 154 - protein, 9 aa, Artificial Sequence
  RG-7159 LCDR3
AQNLELPYT

SEQ ID NO: 155 - protein, 6 aa, Artificial Sequence
  Ofatumumab HCDR1
NDYAMH

SEQ ID NO: 156 - protein, 17 aa, Artificial Sequence
  Ofatumumab HCDR2
TISWNSGSIGYADSVKG

SEQ ID NO: 157 - protein, 13 aa, Artificial Sequence
  Ofatumumab HCDR3
DIQYGNYYYGMDV

SEQ ID NO: 158 - protein, 11 aa, Artificial Sequence
  Ofatumumab LCDR1
RASQSVSSYLA

SEQ ID NO: 159 - protein, 7 aa, Artificial Sequence
  Ofatumumab LCDR2
DASNRAT

SEQ ID NO: 160 - protein, 9 aa, Artificial Sequence
  Ofatumumab LCDR3
QQRSNWPIT

SEQ ID NO: 161 - protein, 5 aa, Artificial Sequence
  2B8 HCDR1
SYNMH

SEQ ID NO: 162 - protein, 17 aa, Artificial Sequence
  2B8 HCDR2
AIYPGNGDTSYNQKFKG

SEQ ID NO: 163 - protein, 12 aa, Artificial Sequence
  2B8 HCDR3
STYYGGDWYFNV

SEQ ID NO: 164 - protein, 10 aa, Artificial Sequence
  2B8 LCDR1
RASSSVSYIH

SEQ ID NO: 165 - protein, 7 aa, Artificial Sequence
  2B8 LCDR2
ATSNLAS

SEQ ID NO: 166 - protein, 9 aa, Artificial Sequence
  2B8 LCDR3
QQWTSNPPT

SEQ ID NO: 167 - protein, 5 aa, Artificial Sequence
  Tositumomab HCDR1
SYNMH

SEQ ID NO: 168 - protein, 17 aa, Artificial Sequence
  Tositumomab HCDR2
AIYPGNGDTSYNQKFKG

SEQ ID NO: 169 - protein, 13 aa, Artificial Sequence
  Tositumomab HCDR3
VVYYSNSYWYFDV

SEQ ID NO: 170 - protein, 10 aa, Artificial Sequence
  Tositumomab LCDR1
RASSSVSYMH

SEQ ID NO: 171 - protein, 7 aa, Artificial Sequence
  Tositumomab LCDR2
APSNLAS

SEQ ID NO: 172 - protein, 9 aa, Artificial Sequence
  Tositumomab LCDR3
QQWSFNPPT

SEQ ID NO: 173 - protein, 8 aa, Artificial Sequence
  Ublituximab HCDR1
GYTFTSYN

SEQ ID NO: 174 - protein, 8 aa, Artificial Sequence
  Ublituximab HCDR2
IYPGNGDT

SEQ ID NO: 175 - protein, 11 aa, Artificial Sequence
  Ublituximab HCDR3
ARYDYNYAMDY

SEQ ID NO: 176 - protein, 5 aa, Artificial Sequence
  Ublituximab LCDR1
SSVSY

SEQ ID NO: 177 - protein, 3 aa, Artificial Sequence
  Ublituximab LCDR2
ATS

SEQ ID NO: 178 - protein, 9 aa, Artificial Sequence
  Ublituximab LCDR3
QQWTFNPPT

SEQ ID NO: 179 - protein, 8 aa, Artificial Sequence
  Epcortitamab, 7D8 HCDR1
GFTFHDYA

SEQ ID NO: 180 - protein, 8 aa, Artificial Sequence
  Epcortitamab, 7D8 HCDR2
ISWNSGTI

SEQ ID NO: 181 - protein, 15 aa, Artificial Sequence
  Epcortitamab, 7D8 HCDR3
AKDIQYGNYYYGMDV

SEQ ID NO: 182 - protein, 6 aa, Artificial Sequence
  Epcortitamab, 7D8 LCDR1
QSVSSY

SEQ ID NO: 183 - protein, 3 aa, Artificial Sequence
  Epcortitamab, 7D8 LCDR2
DAS

SEQ ID NO: 184 - protein, 9 aa, Artificial Sequence
  Epcortitamab, 7D8 LCDR3
QQRSNWPIT

SEQ ID NO: 185 - protein, 5 aa, Artificial Sequence
  Divozilimab HCDR1
SYNMH

SEQ ID NO: 186 - protein, 17 aa, Artificial Sequence
  Divozilimab HCDR2
AIYPGNGDTSYNQKFKG

SEQ ID NO: 187 - protein, 12 aa, Artificial Sequence
  Divozilimab HCDR3
STYYGGDWYFNV

SEQ ID NO: 188 - protein, 10 aa, Artificial Sequence
  Divozilimab LCDR1
RASSSVSYIH

SEQ ID NO: 189 - protein, 7 aa, Artificial Sequence
  Divozilimab LCDR2
ATSNLAS

SEQ ID NO: 190 - protein, 9 aa, Artificial Sequence
  Divozilimab LCDR3
QQWTSNPPT

SEQ ID NO: 191 - protein, 8 aa, Artificial Sequence
  Odronextabmab HCDR1
GFTFNDYA

SEQ ID NO: 192 - protein, 8 aa, Artificial Sequence
  Odronextabmab HCDR2
ISWNSDSI

SEQ ID NO: 193 - protein, 20 aa, Artificial Sequence
  Odronextabmab HCDR3
AKDNHYGSGSYYYYQYGMDV

SEQ ID NO: 194 - protein, 6 aa, Artificial Sequence
  Odronextabmab LCDR1
QSVSSN

SEQ ID NO: 195 - protein, 3 aa, Artificial Sequence
  Odronextabmab LCDR2
GAS

SEQ ID NO: 196 - protein, 9 aa, Artificial Sequence
  Odronextabmab LCDR3
QHYINWPLT

SEQ ID NO: 197 - protein, 5 aa, Artificial Sequence
  Veltuzumab HCDR1
SYNMH

SEQ ID NO: 198 - protein, 17 aa, Artificial Sequence
  Veltuzumab HCDR2
AIYPGNGDTSYNQKFKG

SEQ ID NO: 199 - protein, 12 aa, Artificial Sequence
  Veltuzumab HCDR3-1
STYYGGDWYFDV

SEQ ID NO: 200 - protein, 13 aa, Artificial Sequence
  Veltuzumab HCDR3-2
VVYYSNSYWYFDV

SEQ ID NO: 201 - protein, 10 aa, Artificial Sequence
  Veltuzumab LCDR1
RASSSVSYIH

SEQ ID NO: 202 - protein, 7 aa, Artificial Sequence
  Veltuzumab LCDR2
ATSNLAS

SEQ ID NO: 203 - protein, 9 aa, Artificial Sequence
  Veltuzumab LCDR3
QQWTSNPPT

SEQ ID NO: 204 - protein, 5 aa, Artificial Sequence
  MB-CART2019.1 HCDR1
SYNMH

SEQ ID NO: 205 - protein, 17 aa, Artificial Sequence
  MB-CART2019.1 HCDR2
AIYPGNGDTSYNQKFKG

SEQ ID NO: 206 - protein, 13 aa, Artificial Sequence
  MB-CART2019.1 HCDR3
SNYYGSSYWFFDV

SEQ ID NO: 207 - protein, 10 aa, Artificial Sequence
  MB-CART2019.1 LCDR1
RASSSVNYMD

SEQ ID NO: 208 - protein, 7 aa, Artificial Sequence
  MB-CART2019.1 LCDR2
ATSNLAS

SEQ ID NO: 209 - protein, 9 aa, Artificial Sequence
  MB-CART2019.1 LCDR3
QQWSFNPPT

SEQ ID NO: 210 - protein, 10 aa, Artificial Sequence
  Ocaratuzumab HCDR1
GRTFTSYNMH

SEQ ID NO: 211 - protein, 16 aa, Artificial Sequence
  Ocaratuzumab HCDR2
AIYPLTGDTSYNQKSK

SEQ ID NO: 212 - protein, 12 aa, Artificial Sequence
  Ocaratuzumab HCDR3
STYVGGDWQFDV

SEQ ID NO: 213 - protein, 10 aa, Artificial Sequence
  Ocaratuzumab LCDR1
RASSSVPYIH

SEQ ID NO: 214 - protein, 7 aa, Artificial Sequence
  Ocaratuzumab LCDR2
ATSALAS

SEQ ID NO: 215 - protein, 9 aa, Artificial Sequence
  Ocaratuzumab LCDR3
QQWLSNPPT

SEQ ID NO: 216 - protein, 8 aa, Artificial Sequence
  ADI-001 HCDR1
GFTFYDYA

SEQ ID NO: 217 - protein, 8 aa, Artificial Sequence
  ADI-001 HCDR2
ISWNSGYI

SEQ ID NO: 218 - protein, 15 aa, Artificial Sequence
  ADI-001 HCDR3
AKDNSYGKFYYGLDV

SEQ ID NO: 219 - protein, 6 aa, Artificial Sequence
  ADI-001 LCDR1
QSVSSN

SEQ ID NO: 220 - protein, 3 aa, Artificial Sequence
  ADI-001 LCDR2
GAS

SEQ ID NO: 221 - protein, 9 aa, Artificial Sequence
  ADI-001 LCDR3
QQYNNWPIT

SEQ ID NO: 222 - protein, 7 aa, Artificial Sequence
  Pamotamab HCDR1
YTFTSYN

SEQ ID NO: 223 - protein, 6 aa, Artificial Sequence
  Pamotamab HCDR2
YPGNGD

SEQ ID NO: 224 - protein, 12 aa, Artificial Sequence
  Pamotamab HCDR3
STYYGGDWYFNV

SEQ ID NO: 225 - protein, 6 aa, Artificial Sequence
  Pamotamab LCDR1
SSSVSY

SEQ ID NO: 226 - protein, 7 aa, Artificial Sequence
  Pamotamab LCDR2
ATSNLAS

SEQ ID NO: 227 - protein, 7 aa, Artificial Sequence
  Pamotamab LCDR3
WTSNPPT

SEQ ID NO: 228 - protein, 5 aa, Artificial Sequence
  DNL-1 HCDR1
SYNMH

SEQ ID NO: 229 - protein, 17 aa, Artificial Sequence
  DNL-1 HCDR2
AIYPGNGDTSYNQKFKG

SEQ ID NO: 230 - protein, 12 aa, Artificial Sequence
  DNL-1 HCDR3
STYYGGDWYFDV

SEQ ID NO: 231 - protein, 10 aa, Artificial Sequence
  DNL-1 LCDR1
RASSSVSYIH

SEQ ID NO: 232 - protein, 7 aa, Artificial Sequence
  DNL-1 LCDR2
ATSNLAS

SEQ ID NO: 233 - protein, 9 aa, Artificial Sequence
  DNL-1 LCDR3
QQWTSNPPT

SEQ ID NO: 234 - protein, 10 aa, Artificial Sequence
  mAb-1.5.3 HCDR1
GYSFTSYWIG

SEQ ID NO: 235 - protein, 17 aa, Artificial Sequence
  mAb-1.5.3 HCDR2
IIYPGDSDTRYSPSFQG

SEQ ID NO: 236 - protein, 13 aa, Artificial Sequence
  mAb-1.5.3 HCDR3
HPSYGSGSPNFDY

SEQ ID NO: 237 - protein, 16 aa, Artificial Sequence
  mAb-1.5.3 LCDR1
RSSQSLVYSDGNTYLS

SEQ ID NO: 238 - protein, 7 aa, Artificial Sequence
  mAb-1.5.3 LCDR2
KISNRFS

SEQ ID NO: 239 - protein, 9 aa, Artificial Sequence
  mAb-1.5.3 LCDR3
VQATQFPLT

SEQ ID NO: 240 - protein, 122 aa, Artificial Sequence [sequence omitted]

SEQ ID NO: 241 - protein, 107 aa, Artificial Sequence
  VL of Ocrelizumab
DIQMTQSPSSLSASVGDRVTITCRASSSVSYMHWYQQKPGKAPKPLIYAPSNLASGVPSRFSGSGSGTDFTLTISSLQPEDFATYYCQQWSFNPPTFGQGTKVEIKR

SEQ ID NO: 242 - protein, 119 aa, Artificial Sequence
  VH of RG-7159
QVQLVQSGAEVKKPGSSVKVSCKASGYAFSYSWINWVRQAPGQGLEWMGRIFPGDGDTDYNGKFKGRVTITADKSTSTAYMELSSLRSEDTAVYYCARNVFDGYWLVYWGQGTLVTVSS

SEQ ID NO: 243 - protein, 112 aa, Artificial Sequence
  VL of RG-7159
DIVMTQTPLSLPVTPGEPASISCRSSKSLLHSNGITYLYWYLQKPGQSPQLLIYQMSNLVSGVPDRFSGSGSGTDFTLKISRVEAEDVGVYYCAQNLELPYTFGGGTKVEIK

SEQ ID NO: 244 - protein, 122 aa, Artificial Sequence
  VH of Ofatumumab
EVQLVESGGGLVQPGRSLRLSCAASGFTFNDYAMHWVRQAPGKGLEWVSTISWNSGSIGYADSVKGRFTISRDNAKKSLYLQMNSLRAEDTALYYCAKDIQYGNYYYGMDVWGQGTTVTVSS

SEQ ID NO: 245 - protein, 107 aa, Artificial Sequence
  VL of Ofatumumab
EIVLTQSPATLSLSPGERATLSCRASQSVSSYLAWYQQKPGQAPRLLIYDASNRATGIPARFSGSGSGTDFTLTISSLEPEDFAVYYCQQRSNWPITFGQGTRLEIK

SEQ ID NO: 246 - protein, 121 aa, Artificial Sequence [sequence omitted]

SEQ ID NO: 247 - protein, 106 aa, Artificial Sequence [sequence omitted]

SEQ ID NO: 248 - protein, 122 aa, Artificial Sequence
  VH of Tositumomab
QAYLQQSGAELVRPGASVKMSCKASGYTFTSYNMHWVKQTPRQGLEWIGAIYPGNGDTSYNQKFKGKATLTVDKSSSTAYMQLSSLTSEDSAVYFCARVVYYSNSYWYFDVWGTGTTVTVSG

SEQ ID NO: 249 - protein, 106 aa, Artificial Sequence [sequence omitted]

SEQ ID NO: 250 - protein, 118 aa, Artificial Sequence
  VH of Ublituximab
QAYLQQSGAELVRPGASVKMSCKASGYTFTSYNMHWVKQTPRQGLEWIGGIYPGNGDTSYNQKFKGKATLTVGKSSSTAYMQLSSLTSEDSAVYFCARYDYNYAMDYWGQGTSVTVSS

SEQ ID NO: 251 - protein, 106 aa, Artificial Sequence
  VL of Ublituximab
QIVLSQSPAILSASPGEKVTMTCRASSSVSYMHWYQQKPGSSPKPWIYATSNLASGVPARFSGSGSGTSYSFTISRVEAEDAATYYCQQWTFNPPTFGGGTRLEIK

SEQ ID NO: 252 - protein, 122 aa, Artificial Sequence
  VH of Epcortitamab
EVQLVESGGGLVQPDRSLRLSCAASGFTFHDYAMHWVRQAPGKGLEWVSTISWNSGTIGYADSVKGRFTISRDNAKNSLYLQMNSLRAEDTALYYCAKDIQYGNYYYGMDVWGQGTTVTVSS

SEQ ID NO: 253 - protein, 107 aa, Artificial Sequence; identical to SEQ ID NO: 245
  VL of Epcortitamab

SEQ ID NO: 254 - protein, 121 aa, Artificial Sequence
  VH of Divozilimab
EVQLVQPGAEVVKPGASVKVSCKASGYTFTSYNMHWVRQAPGRGLEWMGAIYPGNGDTSYNQKFKGRVTMTRDKSTSTVYMELSSLRSEDTAVYYCARSTYYGGDWYFNVWGQGTLVTVSS

SEQ ID NO: 255 - protein, 106 aa, Artificial Sequence
  VL of Divozilimab
QIVLSQSPAILSASPGERVTLTCRASSSVSYIHWFQQKPGKAPKPLIYATSNLASGVPSRFSGSGSGTDFSLTISRVEPEDFAVYYCQQWTSNPPTFGGGTKVEIK

SEQ ID NO: 256 - protein, 127 aa, Artificial Sequence
  VH of Odronextabmab
EVQLVESGGGLVQPGRSLRLSCVASGFTFNDYAMHWVRQAPGKGLEWVSVISWNSDSIGYADSVKGRFTISRDNAKNSLYLQMHSLRAEDTALYYCAKDNHYGSGSYYYYQYGMDVWGQGTTVTVSS

SEQ ID NO: 257 - protein, 108 aa, Artificial Sequence
  VL of Odronextabmab
EIVMTQSPATLSVSPGERATLSCRASQSVSSNLAWYQQKPGQAPRLLIYGASTRATGIPARFSGSGSGTEFTLTISSLQSEDFAVYYCQHYINWPLTFGGGTKVEIKR

SEQ ID NO: 258 - protein, 121 aa, Artificial Sequence
  VH of Veltuzumab
QVQLQQSGAEVKKPGSSVKVSCKASGYTFTSYNMHWVKQAPGQGLEWIGAIYPGNGDTSYNQKFKGKATLTADESTNTAYMELSSLRSEDTAFYYCARSTYYGGDWYFDVWGQGTTVTVSS

SEQ ID NO: 259 - protein, 107 aa, Artificial Sequence
  VL of Veltuzumab
DIQLTQSPSSLSASVGDRVTMTCRASSSVSYIHWFQQKPGKAPKPWIYATSNLASGVPVRFSGSGSGTDYTFTISSLQPEDIATYYCQQWTSNPPTFGGGTKLEIKR

SEQ ID NO: 260 - protein, 122 aa, Artificial Sequence
  VH of MB-CART2019.1
EVQLQQSGAELVKPGASVKMSCKASGYTFTSYNMHWVKQTPGQGLEWIGAIYPGNGDTSYNQKFKGKATLTADKSSSTAYMQLSSLTSEDSADYYCARSNYYGSSYWFFDVWGAGTTVTVSS

SEQ ID NO: 261 - protein, 106 aa, Artificial Sequence
  VL of MB-CART2019.1
DIVLTQSPAILSASPGEKVTMTCRASSSVNYMDWYQKKPGSSPKPWIYATSNLASGVPARFSGSGSGTSYSLTISRVEAEDAATYYCQQWSFNPPTFGGGTKLEIK

SEQ ID NO: 262 - protein, 121 aa, Artificial Sequence
  VH of Ocaratuzumab
EVQLVQSGAEVKKPGESLKISCKGSGRTFTSYNMHWVRQMPGKGLEWMGAIYPLTGDTSYNQKSKLQVTISADKSISTAYLQWSSLKASDTAMYYCARSTYVGGDWQFDVWGKGTTVTVSS

SEQ ID NO: 263 - protein, 106 aa, Artificial Sequence
  VL of Ocaratuzumab
EIVLTQSPGTLSLSPGERATLSCRASSSVPYIHWYQQKPGQAPRLLIYATSALASGIPDRFSGSGSGTDFTLTISRLEPEDFAVYYCQQWLSNPPTFGQGTKLEIK

SEQ ID NO: 264 - protein, 122 aa, Artificial Sequence
  VH of ADI-001
EVQLVESGGGLVQPGRSLRLSCAASGFTFYDYAMHWVRQAPGKGLEWVSGISWNSGYIGYADSVKGRFTISRDNAKNSLYLQMNSLRAEDTALYYCAKDNSYGKFYYGLDVWGQGTTVTVSS

SEQ ID NO: 265 - protein, 107 aa, Artificial Sequence
  VL of ADI-001
EIVMTQSPATLSVSPGERTTLSCRASQSVSSNLAWYLQKPGQAPRLLIYGASTRATGIPARFSGSGSGTEFILTISSLQSEDFAVYYCQQYNNWPITFGQGTRLEIK

SEQ ID NO: 266 - protein, 121 aa, Artificial Sequence
  VH of Pamotamab
QVQLVQSGAEVKKPGASVKVSCKASGYTFTSYNMHWVRQAPGQGLEWMGAIYPGNGDTSYNQKFQGRVTITADKSISTAYMELSSLRSEDTAVYYCARSTYYGGDWYFNVWGAGTLVTVSS

SEQ ID NO: 267 - protein, 106 aa, Artificial Sequence
  VL of Pamotamab
QIVLTQSPSSLSASVGDRVTITCRASSSVSYIHWFQQKPGKSPKPLIYATSNLASGVPVRFSGSGSGTDYTLTISSLQPEDFATYYCQQWTSNPPTFGGGTKVEIK

SEQ ID NO: 268 - protein, 121 aa, Artificial Sequence; identical to SEQ ID NO: 258
  VH of DNL-1

SEQ ID NO: 269 - protein, 106 aa, Artificial Sequence
  VL of DNL-1
DIQLTQSPSSLSASVGDRVTMTCRASSSVSYIHWFQQKPGKAPKPWIYATSNLASGVPVRFSGSGSGTDYTFTISSLQPEDIATYYCQQWTSNPPTFGGGTKLEIK

SEQ ID NO: 270 - protein, 122 aa, Artificial Sequence
  VH of mAb-1.5.3
EVQLVQSGAEVKKPGESLKISCKGSGYSFTSYWIGWVRQMPGKGLEWMGIIYPGDSDTRYSPSFQGQVTISADKSITTAYLQWSSLKASDTAMYYCARHPSYGSGSPNFDYWGQGTLVTVSS

SEQ ID NO: 271 - protein, 112 aa, Artificial Sequence
  VL of mAb-1.5.3
DIVMTQTPLSSPVTLGQPASISCRSSQSLVYSDGNTYLSWLQQRPGQPPRLLIYKISNRFSGVPDRFSGSGAGTDFTLKISRVEAEDVGVYYCVQATQFPLTFGGGTKVEIK

SEQ ID NO: 272 - protein, 1016 aa, Artificial Sequence
  hu scIL-12-hu IgG1 Fc hole-anti-hu CD20 scFv
IWELKKDVYVVELDWYPDAPGEMVVLTCDTPEEDGITWTLDQSSEVLGSGKTLTIQVKEFGDAGQYTCHKGGEVLSHSLLLLHKKEDGIWSTDILKDQKEPKNKTFLRCEAKNYSGRFTCWWLTTISTDLTFSVKSSRGSSDPQGVTCGAATLSAERVRGDNKEYEYSVECQEDSACPAAEESLPIEVMVDAVHKLKYENYTSSFFIRDIIKPDPPKNLQLKPLKNSRQVEVSWEYPDTWSTPHSYFSLTFCVQVQGKSKREKKDRVFTDKTSATVICRKNASISVRAQDRYYSSSWSEWASVPCSGGGGSGGGGSGGGGSRNLPVATPDPGMFPCLHHSQNLLRAVSNMLQKARQTLEFYPCTSEEIDHEDITKDKTSTVEACLPLELTKNESCLNSRETSFITNGSCLASRKTSFMMALCLSSIYEDLKMYQVEFKTMNAKLLMDPKRQIFLDQNMLAVIDELMQALNFNSETVPQKSSLEEPDFYKTKIKLCILLHAFRIRAVTIDRVMSYLNASGGGGSGGGGSDKTHTCPPCPAPELLGGPSVFLFPPKPKDTLMISRTPEVTCVVVDVSHEDPEVKFNWYVDGVEVHNAKTKPREEQYNSTYRVVSVLTVLHQDWLNGKEYKCKVSNKALPAPIEKTISKAKGQPREPQVYTLPPSRDELTKNQVSLSCAVKGFYPSDIAVEWESNGQPENNYKTTPPVLDSDGSFFLVSKLTVDKSRWQQGNVFSCSVMHEALHNHYTQKSLSLSPGGGGGSGGGGSGGGGSQVQLQQPGAELVKPGASVKMSCKASGYTFTSYNMHWVKQTPGRGLEWIGAIYPGNGDTSYNQKFKGKATLTADKSSSTAYMQLSSLTSEDSAVYYCARSTYYGGDWYFNVWGAGTTVTVSAGGGGSGGGGSGGGGSGGGGSQIVLSQSPAILSASPGEKVTMTCRASSSVSYIHWFQQKPGSSPKPWIYATSNLASGVPVRFSGSGSGTSYSLTISRVEAEDAATYYCQQWTSNPPTFGGGTKLEIK

SEQ ID NO: 273 - protein, 1016 aa, Artificial Sequence
  hu scIL-12 mut2-hu IgG1 Fc hole-anti-hu CD20 scFv
IWELKKDVYVVELDWYPDAPGEMVVLTCDTPEEDGITWTLDQSSEVLGSGKTLTIQVKEFGDAGQYTCHKGGEVLSHSLLLLHKKEDGIWSTDILKDQKEPKNKTFLRCEAKNYSGRFTCWWLTTISTDLTFSVKSSRGSSDPQGVTCGAATLSAERVRGDNKEYEYSVECQEDSACPAAEESLPIEVMVDAVHKLKYENYTSSFFIRDIIKPDPPKNLQLKPLKNSRQVEVSWEYPDTWSTPHSYFSLTFCVQVQGASAREAADRVFTDKTSATVICRKNASISVRAQDRYYSSSWSEWASVPCSGGGGSGGGGSGGGGSRNLPVATPDPGMFPCLHHSQNLLRAVSNMLQKARQTLEFYPCTSEEIDHEDITKDKTSTVEACLPLELTKNESCLNSRETSFITNGSCLASRKTSFMMALCLSSIYEDLKMYQVEFKTMNAKLLMDPKRQIFLDQNMLAVIDELMQALNFNSETVPQKSSLEEPDFYKTKIKLCILLHAFRIRAVTIDRVMSYLNASGGGGSGGGGSDKTHTCPPCPAPELLGGPSVFLFPPKPKDTLMISRTPEVTCVVVDVSHEDPEVKFNWYVDGVEVHNAKTKPREEQYNSTYRVVSVLTVLHQDWLNGKEYKCKVSNKALPAPIEKTISKAKGQPREPQVYTLPPSRDELTKNQVSLSCAVKGFYPSDIAVEWESNGQPENNYKTTPPVLDSDGSFFLVSKLTVDKSRWQQGNVFSCSVMHEALHNHYTQKSLSLSPGGGGGSGGGGSGGGGSQVQLQQPGAELVKPGASVKMSCKASGYTFTSYNMHWVKQTPGRGLEWIGAIYPGNGDTSYNQKFKGKATLTADKSSSTAYMQLSSLTSEDSAVYYCARSTYYGGDWYFNVWGAGTTVTVSAGGGGSGGGGSGGGGSGGGGSQIVLSQSPAILSASPGEKVTMTCRASSSVSYIHWFQQKPGSSPKPWIYATSNLASGVPVRFSGSGSGTSYSLTISRVEAEDAATYYCQQWTSNPPTFGGGTKLEIK

SEQ ID NO: 274 - protein, 983 aa, Artificial Sequence
  anti-hu CD20 HC hu IgG1 Fc-hu scIL-12
QVQLQQPGAELVKPGASVKMSCKASGYTFTSYNMHWVKQTPGRGLEWIGAIYPGNGDTSYNQKFKGKATLTADKSSSTAYMQLSSLTSEDSAVYYCARSTYYGGDWYFNVWGAGTTVTVSAASTKGPSVFPLAPSSKSTSGGTAALGCLVKDYFPEPVTVSWNSGALTSGVHTFPAVLQSSGLYSLSSVVTVPSSSLGTQTYICNVNHKPSNTKVDKKVEPKSCDKTHTCPPCPAPELLGGPSVFLFPPKPKDTLMISRTPEVTCVVVDVSHEDPEVKFNWYVDGVEVHNAKTKPREEQYNSTYRVVSVLTVLHQDWLNGKEYKCKVSNKALPAPIEKTISKAKGQPREPQVYTLPPSRDELTKNQVSLTCLVKGFYPSDIAVEWESNGQPENNYKTTPPVLDSDGSFFLYSKLTVDKSRWQQGNVFSCSVMHEALHNHYTQKSLSLSPGGGGGSGGGGSGGGGSIWELKKDVYVVELDWYPDAPGEMVVLTCDTPEEDGITWTLDQSSEVLGSGKTLTIQVKEFGDAGQYTCHKGGEVLSHSLLLLHKKEDGIWSTDILKDQKEPKNKTFLRCEAKNYSGRFTCWWLTTISTDLTFSVKSSRGSSDPQGVTCGAATLSAERVRGDNKEYEYSVECQEDSACPAAEESLPIEVMVDAVHKLKYENYTSSFFIRDIIKPDPPKNLQLKPLKNSRQVEVSWEYPDTWSTPHSYFSLTFCVQVQGKSKREKKDRVFTDKTSATVICRKNASISVRAQDRYYSSSWSEWASVPCSGGGGSGGGGSGGGGSRNLPVATPDPGMFPCLHHSQNLLRAVSNMLQKARQTLEFYPCTSEEIDHEDITKDKTSTVEACLPLELTKNESCLNSRETSFITNGSCLASRKTSFMMALCLSSIYEDLKMYQVEFKTMNAKLLMDPKRQIFLDQNMLAVIDELMQALNFNSETVPQKSSLEEPDFYKTKIKLCILLHAFRIRAVTIDRVMSYLNAS

SEQ ID NO: 275 - protein, 983 aa, Artificial Sequence
  anti-hu CD20 HC hu IgG1 Fc-hu scIL-12 mut2
QVQLQQPGAELVKPGASVKMSCKASGYTFTSYNMHWVKQTPGRGLEWIGAIYPGNGDTSYNQKFKGKATLTADKSSSTAYMQLSSLTSEDSAVYYCARSTYYGGDWYFNVWGAGTTVTVSAASTKGPSVFPLAPSSKSTSGGTAALGCLVKDYFPEPVTVSWNSGALTSGVHTFPAVLQSSGLYSLSSVVTVPSSSLGTQTYICNVNHKPSNTKVDKKVEPKSCDKTHTCPPCPAPELLGGPSVFLFPPKPKDTLMISRTPEVTCVVVDVSHEDPEVKFNWYVDGVEVHNAKTKPREEQYNSTYRVVSVLTVLHQDWLNGKEYKCKVSNKALPAPIEKTISKAKGQPREPQVYTLPPSRDELTKNQVSLTCLVKGFYPSDIAVEWESNGQPENNYKTTPPVLDSDGSFFLYSKLTVDKSRWQQGNVFSCSVMHEALHNHYTQKSLSLSPGGGGGSGGGGSGGGGSIWELKKDVYVVELDWYPDAPGEMVVLTCDTPEEDGITWTLDQSSEVLGSGKTLTIQVKEFGDAGQYTCHKGGEVLSHSLLLLHKKEDGIWSTDILKDQKEPKNKTFLRCEAKNYSGRFTCWWLTTISTDLTFSVKSSRGSSDPQGVTCGAATLSAERVRGDNKEYEYSVECQEDSACPAAEESLPIEVMVDAVHKLKYENYTSSFFIRDIIKPDPPKNLQLKPLKNSRQVEVSWEYPDTWSTPHSYFSLTFCVQVQGASAREAADRVFTDKTSATVICRKNASISVRAQDRYYSSSWSEWASVPCSGGGGSGGGGSGGGGSRNLPVATPDPGMFPCLHHSQNLLRAVSNMLQKARQTLEFYPCTSEEIDHEDITKDKTSTVEACLPLELTKNESCLNSRETSFITNGSCLASRKTSFMMALCLSSIYEDLKMYQVEFKTMNAKLLMDPKRQIFLDQNMLAVIDELMQALNFNSETVPQKSSLEEPDFYKTKIKLCILLHAFRIRAVTIDRVMSYLNAS

SEQ ID NO: 276 - protein, 1016 aa, Artificial Sequence
  hu scIL-12-hu IgG1 Fc-anti-hu CD20 scFv
IWELKKDVYVVELDWYPDAPGEMVVLTCDTPEEDGITWTLDQSSEVLGSGKTLTIQVKEFGDAGQYTCHKGGEVLSHSLLLLHKKEDGIWSTDILKDQKEPKNKTFLRCEAKNYSGRFTCWWLTTISTDLTFSVKSSRGSSDPQGVTCGAATLSAERVRGDNKEYEYSVECQEDSACPAAEESLPIEVMVDAVHKLKYENYTSSFFIRDIIKPDPPKNLQLKPLKNSRQVEVSWEYPDTWSTPHSYFSLTFCVQVQGKSKREKKDRVFTDKTSATVICRKNASISVRAQDRYYSSSWSEWASVPCSGGGGSGGGGSGGGGSRNLPVATPDPGMFPCLHHSQNLLRAVSNMLQKARQTLEFYPCTSEEIDHEDITKDKTSTVEACLPLELTKNESCLNSRETSFITNGSCLASRKTSFMMALCLSSIYEDLKMYQVEFKTMNAKLLMDPKRQIFLDQNMLAVIDELMQALNFNSETVPQKSSLEEPDFYKTKIKLCILLHAFRIRAVTIDRVMSYLNASGGGGSGGGGSDKTHTCPPCPAPELLGGPSVFLFPPKPKDTLMISRTPEVTCVVVDVSHEDPEVKFNWYVDGVEVHNAKTKPREEQYNSTYRVVSVLTVLHQDWLNGKEYKCKVSNKALPAPIEKTISKAKGQPREPQVYTLPPSRDELTKNQVSLTCLVKGFYPSDIAVEWESNGQPENNYKTTPPVLDSDGSFFLYSKLTVDKSRWQQGNVFSCSVMHEALHNHYTQKSLSLSPGGGGGSGGGGSGGGGSQVQLQQPGAELVKPGASVKMSCKASGYTFTSYNMHWVKQTPGRGLEWIGAIYPGNGDTSYNQKFKGKATLTADKSSSTAYMQLSSLTSEDSAVYYCARSTYYGGDWYFNVWGAGTTVTVSAGGGGSGGGGSGGGGSGGGGSQIVLSQSPAILSASPGEKVTMTCRASSSVSYIHWFQQKPGSSPKPWIYATSNLASGVPVRFSGSGSGTSYSLTISRVEAEDAATYYCQQWTSNPPTFGGGTKLEIK

SEQ ID NO: 277 - protein, 1016 aa, Artificial Sequence
  hu scIL-12 mut2-hu IgG1 Fc-anti-hu CD20 scFv
IWELKKDVYVVELDWYPDAPGEMVVLTCDTPEEDGITWTLDQSSEVLGSGKTLTIQVKEFGDAGQYTCHKGGEVLSHSLLLLHKKEDGIWSTDILKDQKEPKNKTFLRCEAKNYSGRFTCWWLTTISTDLTFSVKSSRGSSDPQGVTCGAATLSAERVRGDNKEYEYSVECQEDSACPAAEESLPIEVMVDAVHKLKYENYTSSFFIRDIIKPDPPKNLQLKPLKNSRQVEVSWEYPDTWSTPHSYFSLTFCVQVQGASAREAADRVFTDKTSATVICRKNASISVRAQDRYYSSSWSEWASVPCSGGGGSGGGGSGGGGSRNLPVATPDPGMFPCLHHSQNLLRAVSNMLQKARQTLEFYPCTSEEIDHEDITKDKTSTVEACLPLELTKNESCLNSRETSFITNGSCLASRKTSFMMALCLSSIYEDLKMYQVEFKTMNAKLLMDPKRQIFLDQNMLAVIDELMQALNFNSETVPQKSSLEEPDFYKTKIKLCILLHAFRIRAVTIDRVMSYLNASGGGGSGGGGSDKTHTCPPCPAPELLGGPSVFLFPPKPKDTLMISRTPEVTCVVVDVSHEDPEVKFNWYVDGVEVHNAKTKPREEQYNSTYRVVSVLTVLHQDWLNGKEYKCKVSNKALPAPIEKTISKAKGQPREPQVYTLPPSRDELTKNQVSLTCLVKGFYPSDIAVEWESNGQPENNYKTTPPVLDSDGSFFLYSKLTVDKSRWQQGNVFSCSVMHEALHNHYTQKSLSLSPGGGGGSGGGGSGGGGSQVQLQQPGAELVKPGASVKMSCKASGYTFTSYNMHWVKQTPGRGLEWIGAIYPGNGDTSYNQKFKGKATLTADKSSSTAYMQLSSLTSEDSAVYYCARSTYYGGDWYFNVWGAGTTVTVSAGGGGSGGGGSGGGGSGGGGSQIVLSQSPAILSASPGEKVTMTCRASSSVSYIHWFQQKPGSSPKPWIYATSNLASGVPVRFSGSGSGTSYSLTISRVEAEDAATYYCQQWTSNPPTFGGGTKLEIK

SEQ ID NO: 278 - protein, 1025 aa, Artificial Sequence
  mu scIL-12-mu IgG2a Fc hole-anti-mu CD20 scFv
MWELEKDVYVVEVDWTPDAPGETVNLTCDTPEEDDITWTSDQRHGVIGSGKTLTITVKEFLDAGQYTCHKGGETLSHSHLLLHKKENGIWSTEILKNFKNKTFLKCEAPNYSGRFTCSWLVQRNMDLKFNIKSSSSSPDSRAVTCGMASLSAEKVTLDQRDYEKYSVSCQEDVTCPTAEETLPIELALEARQQNKYENYSTSFFIRDIIKPDPPKNLQMKPLKNSQVEVSWEYPDSWSTPHSYFSLKFFVRIQRKKEKMKETEEGCNQKGAFLVEKTSTEVQCKGGNVCVQAQDRYYNSSCSKWACVPCRVRSGGGGSGGGGSGGGGSRVIPVSGPARCLSQSRNLLKTTDDMVKTAREKLKHYSCTAEDIDHEDITRDQTSTLKTCLPLELHKNESCLATRETSSTTRGSCLPPQKTSLMMTLCLGSIYEDLKMYQTEFQAINAALQNHNHQQIILDKGMLVAIDELMQSLNHNGETLRQKPPVGEADPYRVKMKLCILLHAFSTRVVTINRVMGYLSSAGGGGSGGGGSEPRGPTIKPCPPCKCPAPNLLGGPSVFIFPPKIKDVLMISLSPIVTCVVVDVSEDDPDVQISWFVNNVEVHTAQTQTHREDYNSTLRVVSALPIQHQDWMSGKEFKCKVNNKDLPAPIERTISKPKGSVRAPQVYVLPPPEEEMTKKQVTLSCAVTDFMPEDIYVEWTNNGKTELNYKNTEPVLDSDGSYFMVSKLRVEKKNWVERNSYSCSVVHEGLHNHHTTKSFSRTPGGGGGSGGGGSGGGGSQVQLQQPGAELVRPGTSVKLSCKASGYTFTSYWMHWIKQRPGQGLEWIGVIDPSDNYTKYNQKFKGKATLTVDTSSSTAYMQLSSLTSEDSAVYFCAREGYYGSSPWFAYWGQGTLVTVSSGGGGSGGGGSGGGGSGGGGSQIVMSQSPAILSASPGEKVTMTCRARSSVSYIHWYQQKPGSSPKPWIYATSNLASGVPGRFSGSGSGTSYSLTITRVEAEDAATYYCQQWSSKPPTFGGGTKLEIK

SEQ ID NO: 279 - protein, 1025 aa, Artificial Sequence
  mu scIL-12 mut2-mu IgG2a Fc hole-anti-mu CD20 scFv
MWELEKDVYVVEVDWTPDAPGETVNLTCDTPEEDDITWTSDQRHGVIGSGKTLTITVKEFLDAGQYTCHKGGETLSHSHLLLHKKENGIWSTEILKNFKNKTFLKCEAPNYSGRFTCSWLVQRNMDLKFNIKSSSSSPDSRAVTCGMASLSAEKVTLDQRDYEKYSVSCQEDVTCPTAEETLPIELALEARQQNKYENYSTSFFIRDIIKPDPPKNLQMKPLKNSQVEVSWEYPDSWSTPHSYFSLKFFVRIQAAAEKMAETEEGCNQKGAFLVEKTSTEVQCKGGNVCVQAQDRYYNSSCSKWACVPCRVRSGGGGSGGGGSGGGGSRVIPVSGPARCLSQSRNLLKTTDDMVKTAREKLKHYSCTAEDIDHEDITRDQTSTLKTCLPLELHKNESCLATRETSSTTRGSCLPPQKTSLMMTLCLGSIYEDLKMYQTEFQAINAALQNHNHQQIILDKGMLVAIDELMQSLNHNGETLRQKPPVGEADPYRVKMKLCILLHAFSTRVVTINRVMGYLSSAGGGGSGGGGSEPRGPTIKPCPPCKCPAPNLLGGPSVFIFPPKIKDVLMISLSPIVTCVVVDVSEDDPDVQISWFVNNVEVHTAQTQTHREDYNSTLRVVSALPIQHQDWMSGKEFKCKVNNKDLPAPIERTISKPKGSVRAPQVYVLPPPEEEMTKKQVTLSCAVTDFMPEDIYVEWTNNGKTELNYKNTEPVLDSDGSYFMVSKLRVEKKNWVERNSYSCSVVHEGLHNHHTTKSFSRTPGGGGGSGGGGSGGGGSQVQLQQPGAELVRPGTSVKLSCKASGYTFTSYWMHWIKQRPGQGLEWIGVIDPSDNYTKYNQKFKGKATLTVDTSSSTAYMQLSSLTSEDSAVYFCAREGYYGSSPWFAYWGQGTLVTVSSGGGGSGGGGSGGGGSGGGGSQIVMSQSPAILSASPGEKVTMTCRARSSVSYIHWYQQKPGSSPKPWIYATSNLASGVPGRFSGSGSGTSYSLTITRVEAEDAATYYCQQWSSKPPTFGGGTKLEIK

SEQ ID NO: 280 - protein, 986 aa, Artificial Sequence
  anti-mu CD20 HC mu IgG2a Fc-mu scIL-12
QVQLQQPGAELVRPGTSVKLSCKASGYTFTSYWMHWIKQRPGQGLEWIGVIDPSDNYTKYNQKFKGKATLTVDTSSSTAYMQLSSLTSEDSAVYFCAREGYYGSSPWFAYWGQGTLVTVSSAKTTAPSVYPLAPVCGDTTGSSVTLGCLVKGYFPEPVTLTWNSGSLSSGVHTFPAVLQSDLYTLSSSVTVTSSTWPSQSITCNVAHPASSTKVDKKIEPRGPTIKPCPPCKCPAPNLLGGPSVFIFPPKIKDVLMISLSPIVTCVVVDVSEDDPDVQISWFVNNVEVHTAQTQTHREDYNSTLRVVSALPIQHQDWMSGKEFKCKVNNKDLPAPIERTISKPKGSVRAPQVYVLPPPEEEMTKKQVTLTCMVTDFMPEDIYVEWTNNGKTELNYKNTEPVLDSDGSYFMYSKLRVEKKNWVERNSYSCSVVHEGLHNHHTTKSFSRTPGGGGGSGGGGSGGGGSMWELEKDVYVVEVDWTPDAPGETVNLTCDTPEEDDITWTSDQRHGVIGSGKTLTITVKEFLDAGQYTCHKGGETLSHSHLLLHKKENGIWSTEILKNFKNKTFLKCEAPNYSGRFTCSWLVQRNMDLKFNIKSSSSSPDSRAVTCGMASLSAEKVTLDQRDYEKYSVSCQEDVTCPTAEETLPIELALEARQQNKYENYSTSFFIRDIIKPDPPKNLQMKPLKNSQVEVSWEYPDSWSTPHSYFSLKFFVRIQRKKEKMKETEEGCNQKGAFLVEKTSTEVQCKGGNVCVQAQDRYYNSSCSKWACVPCRVRSGGGGSGGGGSGGGGSRVIPVSGPARCLSQSRNLLKTTDDMVKTAREKLKHYSCTAEDIDHEDITRDQTSTLKTCLPLELHKNESCLATRETSSTTRGSCLPPQKTSLMMTLCLGSIYEDLKMYQTEFQAINAALQNHNHQQIILDKGMLVAIDELMQSLNHNGETLRQKPPVGEADPYRVKMKLCILLHAFSTRVVTINRVMGYLSSA

SEQ ID NO: 281 - protein, 986 aa, Artificial Sequence
  anti-mu CD20 HC mu IgG2a Fc-mu scIL-12 mut2
QVQLQQPGAELVRPGTSVKLSCKASGYTFTSYWMHWIKQRPGQGLEWIGVIDPSDNYTKYNQKFKGKATLTVDTSSSTAYMQLSSLTSEDSAVYFCAREGYYGSSPWFAYWGQGTLVTVSSAKTTAPSVYPLAPVCGDTTGSSVTLGCLVKGYFPEPVTLTWNSGSLSSGVHTFPAVLQSDLYTLSSSVTVTSSTWPSQSITCNVAHPASSTKVDKKIEPRGPTIKPCPPCKCPAPNLLGGPSVFIFPPKIKDVLMISLSPIVTCVVVDVSEDDPDVQISWFVNNVEVHTAQTQTHREDYNSTLRVVSALPIQHQDWMSGKEFKCKVNNKDLPAPIERTISKPKGSVRAPQVYVLPPPEEEMTKKQVTLTCMVTDFMPEDIYVEWTNNGKTELNYKNTEPVLDSDGSYFMYSKLRVEKKNWVERNSYSCSVVHEGLHNHHTTKSFSRTPGGGGGSGGGGSGGGGSMWELEKDVYVVEVDWTPDAPGETVNLTCDTPEEDDITWTSDQRHGVIGSGKTLTITVKEFLDAGQYTCHKGGETLSHSHLLLHKKENGIWSTEILKNFKNKTFLKCEAPNYSGRFTCSWLVQRNMDLKFNIKSSSSSPDSRAVTCGMASLSAEKVTLDQRDYEKYSVSCQEDVTCPTAEETLPIELALEARQQNKYENYSTSFFIRDIIKPDPPKNLQMKPLKNSQVEVSWEYPDSWSTPHSYFSLKFFVRIQAAAEKMAETEEGCNQKGAFLVEKTSTEVQCKGGNVCVQAQDRYYNSSCSKWACVPCRVRSGGGGSGGGGSGGGGSRVIPVSGPARCLSQSRNLLKTTDDMVKTAREKLKHYSCTAEDIDHEDITRDQTSTLKTCLPLELHKNESCLATRETSSTTRGSCLPPQKTSLMMTLCLGSIYEDLKMYQTEFQAINAALQNHNHQQIILDKGMLVAIDELMQSLNHNGETLRQKPPVGEADPYRVKMKLCILLHAFSTRVVTINRVMGYLSSA

SEQ ID NO: 282 - protein, 1025 aa, Artificial Sequence
  mu scIL-12-mu IgG2a Fc-anti-mu CD20 scFv
MWELEKDVYVVEVDWTPDAPGETVNLTCDTPEEDDITWTSDQRHGVIGSGKTLTITVKEFLDAGQYTCHKGGETLSHSHLLLHKKENGIWSTEILKNFKNKTFLKCEAPNYSGRFTCSWLVQRNMDLKFNIKSSSSSPDSRAVTCGMASLSAEKVTLDQRDYEKYSVSCQEDVTCPTAEETLPIELALEARQQNKYENYSTSFFIRDIIKPDPPKNLQMKPLKNSQVEVSWEYPDSWSTPHSYFSLKFFVRIQRKKEKMKETEEGCNQKGAFLVEKTSTEVQCKGGNVCVQAQDRYYNSSCSKWACVPCRVRSGGGGSGGGGSGGGGSRVIPVSGPARCLSQSRNLLKTTDDMVKTAREKLKHYSCTAEDIDHEDITRDQTSTLKTCLPLELHKNESCLATRETSSTTRGSCLPPQKTSLMMTLCLGSIYEDLKMYQTEFQAINAALQNHNHQQIILDKGMLVAIDELMQSLNHNGETLRQKPPVGEADPYRVKMKLCILLHAFSTRVVTINRVMGYLSSAGGGGSGGGGSEPRGPTIKPCPPCKCPAPNLLGGPSVFIFPPKIKDVLMISLSPIVTCVVVDVSEDDPDVQISWFVNNVEVHTAQTQTHREDYNSTLRVVSALPIQHQDWMSGKEFKCKVNNKDLPAPIERTISKPKGSVRAPQVYVLPPPEEEMTKKQVTLTCMVTDFMPEDIYVEWTNNGKTELNYKNTEPVLDSDGSYFMYSKLRVEKKNWVERNSYSCSVVHEGLHNHHTTKSFSRTPGGGGGSGGGGSGGGGSQVQLQQPGAELVRPGTSVKLSCKASGYTFTSYWMHWIKQRPGQGLEWIGVIDPSDNYTKYNQKFKGKATLTVDTSSSTAYMQLSSLTSEDSAVYFCAREGYYGSSPWFAYWGQGTLVTVSSGGGGSGGGGSGGGGSGGGGSQIVMSQSPAILSASPGEKVTMTCRARSSVSYIHWYQQKPGSSPKPWIYATSNLASGVPGRFSGSGSGTSYSLTITRVEAEDAATYYCQQWSSKPPTFGGGTKLEIK

SEQ ID NO: 283 - protein, 1025 aa, Artificial Sequence
  mu scIL-12 mut2-mu IgG2a Fc-anti-mu CD20 scFv
MWELEKDVYVVEVDWTPDAPGETVNLTCDTPEEDDITWTSDQRHGVIGSGKTLTITVKEFLDAGQYTCHKGGETLSHSHLLLHKKENGIWSTEILKNFKNKTFLKCEAPNYSGRFTCSWLVQRNMDLKFNIKSSSSSPDSRAVTCGMASLSAEKVTLDQRDYEKYSVSCQEDVTCPTAEETLPIELALEARQQNKYENYSTSFFIRDIIKPDPPKNLQMKPLKNSQVEVSWEYPDSWSTPHSYFSLKFFVRIQAAAEKMAETEEGCNQKGAFLVEKTSTEVQCKGGNVCVQAQDRYYNSSCSKWACVPCRVRSGGGGSGGGGSGGGGSRVIPVSGPARCLSQSRNLLKTTDDMVKTAREKLKHYSCTAEDIDHEDITRDQTSTLKTCLPLELHKNESCLATRETSSTTRGSCLPPQKTSLMMTLCLGSIYEDLKMYQTEFQAINAALQNHNHQQIILDKGMLVAIDELMQSLNHNGETLRQKPPVGEADPYRVKMKLCILLHAFSTRVVTINRVMGYLSSAGGGGSGGGGSEPRGPTIKPCPPCKCPAPNLLGGPSVFIFPPKIKDVLMISLSPIVTCVVVDVSEDDPDVQISWFVNNVEVHTAQTQTHREDYNSTLRVVSALPIQHQDWMSGKEFKCKVNNKDLPAPIERTISKPKGSVRAPQVYVLPPPEEEMTKKQVTLTCMVTDFMPEDIYVEWTNNGKTELNYKNTEPVLDSDGSYFMYSKLRVEKKNWVERNSYSCSVVHEGLHNHHTTKSFSRTPGGGGGSGGGGSGGGGSQVQLQQPGAELVRPGTSVKLSCKASGYTFTSYWMHWIKQRPGQGLEWIGVIDPSDNYTKYNQKFKGKATLTVDTSSSTAYMQLSSLTSEDSAVYFCAREGYYGSSPWFAYWGQGTLVTVSSGGGGSGGGGSGGGGSGGGGSQIVMSQSPAILSASPGEKVTMTCRARSSVSYIHWYQQKPGSSPKPWIYATSNLASGVPGRFSGSGSGTSYSLTITRVEAEDAATYYCQQWSSKPPTFGGGTKLEIK

SEQ ID NO: 284 - protein, 227 aa, Artificial Sequence
  hu IgG1 Fc
DKTHTCPPCPAPELLGGPSVFLFPPKPKDTLMISRTPEVTCVVVDVSHEDPEVKFNWYVDGVEVHNAKTKPREEQYNSTYRVVSVLTVLHQDWLNGKEYKCKVSNKALPAPIEKTISKAKGQPREPQVYTLPPSRDELTKNQVSLTCLVKGFYPSDIAVEWESNGQPENNYKTTPPVLDSDGSFFLYSKLTVDKSRWQQGNVFSCSVMHEALHNHYTQKSLSLSPGK

SEQ ID NO: 285 - protein, 233 aa, Artificial Sequence
  mu IgG2a Fc
EPRGPTIKPCPPCKCPAPNLLGGPSVFIFPPKIKDVLMISLSPIVTCVVVDVSEDDPDVQISWFVNNVEVHTAQTQTHREDYNSTLRVVSALPIQHQDWMSGKEFKCKVNNKDLPAPIERTISKPKGSVRAPQVYVLPPPEEEMTKKQVTLTCMVTDFMPEDIYVEWTNNGKTELNYKNTEPVLDSDGSYFMYSKLRVEKKNWVERNSYSCSVVHEGLHNHHTTKSFSRTPGK